European Patent Application EP 4 659 753 A1, published December 10, 2025. Title: THERAPEUTIC AND NON-THERAPEUTIC USES OF TAILOCINS OF PSEUDOMONAS SPECIES AGAINST E. COLI AND NEW TAILOCINS OF PSEUDOMONAS FLUORESCENS. Applicant: GREENPHAGE. Application EP. The sequence listing filed with the application follows.

SEQUENCE LISTING (55 sequences)

SEQ ID NO: 1 - DNA, 17544 bp, Pseudomonas fluorescens Ps36
  source 1..17544: mol_type = genomic DNA
atgcaaaaacgcaacgtatcctccgtcttaagagcgctgctcgatcagtacgggatctcccccacggagctccaccgtcgcaccggcgtgcctcaatccactctctcgcggattctcagcgggaagatcgtcgatccttcggataaacacatctcgaagattgccgagtacttcgccgtgagtaccgatcagttgcgcgggcgcgcggatgttgcgccggtcgccggcggcgggcgcgaggagttgcattccgaactcaaggacataagcctgtgggacgatgacacgcccgtcgatgacgacgaggtgtcggtgcccttccttcgcgaggttgaattggctgctggatcaggaagattcgtcatcgaagagagcgaacgctctagcttgcgcttcggcaagcgcagcctgcgccataacggcgtgcagttcgaccaggccaaatgcgtgaccgtacggggcaacagcatgttgccggtgctgcgtgacggcgccaccgtcggtgtgaacgcgggcaagtgcgggatcggcgacatcatcgatggcgacctttacgcgatcaaccacaacggtcagttgcgggtgaaacagctctatcgcctgcccaccggtatccgcctgcgcagcttcaatcgcgacgagcatccggacgaggactacagcttccaggacatgcaggaagagcagatcgtcatcctcggtcacgtcttctggtggggcatgtacgcccggtaacgatccctctctcagataaaacccgcccacggcgggttttttttcgcctgtagaaaaccggacaacccttgattggcggggcttccatgcatccgcgcatttctcatgcataaataaatgcatttacgcattgactggatatgcatacatgcatattcttgccaccaagccgctcgacaaagcggctggcaacaacagctctttagttccacaagaacaggcagcgatgaaccggcctcaacggttcagagggttggcaactgacccgggtgtgcagcgtaaagcaccagaagcagttatccggcgggcagggaccgcggtcggaaaaacaatttgaacggactcgtaccgcgccagtagcgccgaaaagtcagcttccttcacgtacacaggattgaaggaaggcgaaggagcgcattactgaaaagcccggcgagatgccgggctttttggaatgcctgtcctgggcgccagcatcgaaatccattgtgcccgcaagtgcgggtgggcaatgcacatcgataaaccatctaacagacaactgaaaaaaggaaaaaacatgcgccgatatggacgtgttgatcaggatcgaattgtcgagttttttgaaaccgacggtgacatcacgcaaatgtttcacccaagcattatctgggcagaagtgaccgatcaccccgaagtgcaactgggctgggtcgccaccaaaaccgacggtgtctggacctttgccgcctatgtgccgccaccgccgaccgagcaggaactcatcgccaaggcgcagctgaacaaatggcaactgttgaacgtggccgccaactggctgctgctcaactccctgcagttcaaggtcgacaccggtgtggccacccctgacgaacaggctctgttgctggctcacaagatgtactccatcgctgtcagcgacatcgacaaacaatcgggttacccggcaaacattgtctggccggtggctccgtactgacagtgtttgaaagacagcactgacgactatcaaatcaaaggaagcaagaatgaatcgctacatactgatgaccacggcctattcctacaaccttgtcctcgacgtggtggataccgacgggccgatgcctgaggtgccggcagatgagccctattcgagttggcaagactataccggtaacactactgcagagccgggtatgaaaatggtatggaacgggctaccgagttttgttccgacaaccgcaactgagcgggaggccatgaatcagggacgcatccaaacgcggcttcaggaggcccagagctggttgatgttcaatcccgtgcaatacaaatcggacctggggactgcctctccagccgaggaggccgcattgcttgcctacaagcagtacttcgtggcggtcgccgaagtgaaaaatcaaaccacctttccgaagctcaactggccggtcgcaccgttctgatccagcgagcttcaaactcgacatcgagaacgcattactgaaaagcccggccaccgcgccgggctttttggaatgcctgcctcgagagaaaacgattgaacccgacacacaccactcatccatcacaccaggaggcgtgacatgacaaccgagcaacaagcgttggcggacatgccgatctggctggtcatcctgcttgccgtggcgggcggggtctccggcgaaatgtggcgcgccgacaaggacggcgcccgcggctggccactgctgcggcggctggccctgcgctccggcgcctgcatgatctgcggcgtctcggcgatcatgctgctgtacgccgccggcatgtcgatctgggccgccggcgcttttggctgcctgaccgcaatggccggcgccgacgtggccatcggtctgtatgaacgctgggccgccaagcgcatcggcgtctgcgaagttccgcccgccaatacgaataaggagcaatgaaaaaatacagcggtatttgaaaaggagttcatttcatgttgagcgattttcgttgtggaaaatgcaatcggttactcgcaaaagtagatccacttcatcaagtgcaaatcaaatgccctagatgcaggacgttgaattacgcgaaaacgggatgctttaaaaaatcgcctgtgagcgaaccagggcagcagtgactgctaataataaataatcgacttataggtgatatatatggctacattgccgcgttacccctttacaaccgacggcagttcgattctgttgccgctgcatgaaatgtctgctggacaatatcttcagtcgccagacaagcgttttaaattgattgttcaacccgatggcaatctggcgatttacgaaggagcaaatacagtttgggtggcgattgccggccaaccctatacaagctccgggaagcagatagacaactcaaaaatttacttttatctgatgtattacgcgttcctcaatgatccaacgcgtggccgtatgtggggcactgctaacagcacacctctcaattctgatatctgggcggcttacaatcgtgcctatctatctctgcagaatgatggaaaccttgtagtggtcgactcgatccccgtctggtcaagcaactctgccattcctatcagtccatctgtggagtccgtatatattccggcaggtacaacgcttgaggttgaccgtcggtatgttgtgggagggacgactctggtcttccagtcggatggaaatctggtggtttcaaacggaccacttggagtcctgtgggcgagctggacccagaacaaaggtgccactcgtgcagtcatgcaggaagatggaaattttgtgatctatggacaaaacaatacaccgctctggtttaccggaactgccggtcagccaggtgcaatggcgaaagttcaggcaaatggcagtttctctattgtcagtgaaaagccggtttgggctcgatttggtttcacgccaactattttgccaaaacgcgtattccagtgggacaacggaccatggaaaccgctaatcgaaattcctttgtggcgttttaaagattaattattttgaaatttgcctcccgcttggggggcattttcataatgcttccatccgatgttttatgcgtgcttcacgaagtttcaatttgaatttatcgttgtttagctgaaacccgatatttcgcctcgctgcatgttctgcggcgggactgcgcgtggacattcaaaaaggaggtcatgcatgcctgtaccgatccgacagccttcgcagctgttcacggcaatggcgacagccttgcgcaataacgccgacctgaacgtgcaggtcggtaatcacgatgacttcaccgcacccggcgacaaggcctgggtgctgatcgacatcgaacgcaatgcaccgggagagcgcgcggccaatgggcgcattgcccacgcattgacgctgtcccttcaggttattccggccatatccgccaccgcgtttgccgcgtgtgacctgattgccgccctgaaaaacctgatcaccgacaaccgctggggcctgcccggcgatcagtgcgatctgccgatgaatctcgacggtttgccgtcgctggcgattcgcgccgatcagcccaacaaggcctggaccctgacattcaaccagaccctctacctgggcccgaccttgatcgacgacccgctcggcacaccgaaattcgcccgcacctgggaagtcagcgacatcgacgaccccgaccaatacacctcgctggaggcctgaccgatgttcgacgcgttactgcgcatgcaactgggcccgatcattgagcgtcttgccgagatggaagcggagatcgaagacctgcaccgacgcgccgaaagcttttgccgcatcggcatttgtcaggaagtcgatgcggcgagcaatacctgcaaggtcagtcacggaggattgctcaccccggccatcaagttcttcaacccgagcgccggcgcgcagagcgagtcgcggattcccagcgtgggtgaacagtgtctgctgctcaactacggcagcggagagagtggcgcacaaagcgtggcgttgtttggcttgaacagtgaccgctttccacccgttgcgaccgtccccacgctgacgcgacgggtgcatgtcgatggcagtgaaagcggctacgacgacgccacgcacaccctgcactggcaaaacggtccggcagcgttcagcggttctcgtgaagcgcttgaactgagcatcggcccggcgcgactggcgatgacagcgcaagcgatcaacctgcaactgggcgccaccggcctgaccatcgacgcctcgggcgtgcacttcagcggcccgttggtggatcaccagggtcgcgtcatcagcccctgaatcaagagcctcccatgatcggaatcgatagagacaccggggccacggtcgacgattggctgcaattcgtgcagcgcgcgacacgagccctgaccacgccgctgggcacccggcaaaaaaggcccctttatggttcgttgatccccacgctgctggggcaaaacctcggcgatgacgttctgcttctggcccagagccacgccgcgcaggcgttctacaacccgcagaacggcatcggcgatttccagcccggcgtgatcgtcgccacccgacagggcgccggcctgctgctgcgtttcgccggcacctggaaaaaccgccaacagactttcgaggtcgtgacatgagcatgttgatccctggtcagaaccaactggccgaaccttcactgatcaaggtcgaggccttcgaggatctgctcgccgagttcaagaccttcgtccttgaatacgtcggtacccgttcgccggacagtgcggcaaaactcaagatcagcctggaaaacgaaagcgaactgctgacgatggcgctcgaagcgttttgcgttcgcctgcaaacccacgaacgcaaatacaacgcccgcatcaagcagatgctggcgtggtgggcgaccggcagcaaccttgatgcgcggctggctgacatgggcctggagcgacagttgctcgacccgggcgacccggcggcatttccgccggtgccggcgatttacgaaagcgacgatgacgcccggttgcgctactacctggcgccccatgcgccggcggcaggctcgcggatgcagtaccgccgcgaggtgttcaccctcggcgagcggccgtcggtgaaagtcgaatccaccgatgccggtgtcgtcgacgtcacctacacctttgccccggacggactcgccgcacaggtcaaggatggcaatggccgtcgcaccgcacccggtgaagtgcaggtgacagtgctgtcccgcgacgccgacggcacaccgtccgctgcattgctggatggcgtgcgccaacacttcgcccggcccgatgtctgcccggaaaccgacaaggtcacggtcaagggcgccgagattcagcgctacaagattcgcgtcgtggcgaagatcaattccggcccggattcgggcctgaccaaagttgctgccgagcaacatctgcaagcctacgccgacagttgccatcgcctggaaggccgggtcgccccgagctggatcgactacacgctgcacagcgccggcgccgtgcaactggagattcttgaaccgctgacaccgattgtgtgcagcgcgtttcaagcgccttactgcacggcggtcgaagtcgaggtgcagaccctatgacggaccagacaccgcgtccgaccctgctgccggccaacagctcggcactggaacgggcgctcgatatcggcttcggcaccttgcttgaccgcatcgtgccgccgtttcccgaattgatgaacccgagcgaaacaccggtcgcgttcctgccgtatctcgcagcggatcgcggtgtggccgaatggagcaccgacgcaccggaggcggaaaagcgcctgactgtcgaactggcctggcccaccgcgcgtcaggccggcactcgcaaggcactggaaaacgccgccaaggggttgcaactgaggccggaaattcgcgcctggtacgagcagacaccgccgggcgcgccttacagcttttccgtgcgggccttcaccgaacaaccctacagcgaagaaatcgacgcccgtctcgaccgacgcctggccgatgccaagagcgaacgggacgtgctgtcggtgtcggtcggcctcagcgcattcggcaaccacgtcatcggtgccgcgacgttctgcggtgagctgaccacggtttacccggtgttcctcgaagggctcgagacatccggcgagtccttcaaggccactggtctctacaccgtcgaaacatccactatttatcctcagggggcctgaatggctgactattacaccctgctcaccaacgcagggattgcctacgaaaccgcctgcaaggcagcgggcgtgccgatcaagctgacgcagatttctgtcggcgatggcggtggcgcggtctacaacccggccgcgaccgccactgcgctgaaacgcgaagtctggcgtggaccgcttaacgcgctgtttcaggacgagaaaaatccgagctggctgctcgccgaagtcaccatcccgccagacgtcggcggctggtatgtgcgcgaagccgggctatggaccgacaccggcattctctacgccatcgtcaaatacccggagtcgttcaaaccggtgctggccacgtccggctcgggcaaagagttctacatccgctcgattttcgaaaccagcaatgcttcgctagtgacgctgctgatcgacgacactgtggtcaaggccactcgtgcctgggtcatgagctacctcgccgaagaactcggcaaacttgatggcaaacaatcggtgcgcgtcgccgccaccgccagcgtggtgttgaacggtgcgcagcagatcgacggtgtggcggtgattgccggcgaccgcgtgttgctgccgaatcagactctggccaaggacaacggtctgtggatcgtggccaacggtgactgggttcgggcaaccgatgccaacgtcagcgccaaggtcacaccgggcctgacggtgatggtggaagagggcacgctcaacggcgattcgctgtggcacctgaccaccaacgcgccgatcaccctcggcaccactgcgctgacattcaagatgctcgcggggcgcaccgggattgctgccggcacttacaaaagtctgagcgtcgacgagtatggccgcgcaacagccggctcgaatcccgacacgctggccggcttcggcatcaaggactcctacaccaaggccgaagtcgaagcactgatcgccaaggcctcggcgttgccggtgggttcgattgttgccttccctgtcgatacaccgccgccgggttttctggagctggacaacagcgtcaaaagcagcgcgacttaccctgacttgagcgcctatctgggcggcaagttcaacaagggggatgagggtgtcgggaatttccggttgcctgaggcgcgtggggagtttttgcgcggttgggatcatgggcggggggtggatgcgggccgagagcttggtactgcgcagaccgaagcgttcaaggcacacaaccatcgatattttgatagcgtcgcagcaaccatggatccagcaggtggttggcagagtgggaccgttaacggtacccaggccggtgtttccccaggtgcatttatatcggttaccaatactggtgatgccggtcagatgctgaatgcacataccaccgtcaacaccggaggtactgaaacccgcccccgtaacatcgccgtcatgtggtgcatcaaggcctggaacgccccgatcaatcagggaaatatcgacgtagcggcactggtcaaggaagtctcccgtttgggatctgccgttccggtgggtgctgtcatggcgttcccgacggggatcgtgccgcccggttttcttgagctggatggcagtgtgcaaaacattgcgacttacccggatctggcggcttacctgggaacaacattcaacaagggcgatgaaggagttggtaactttcggttgccggaatctcgtggtgagttcctgcgtggctgggatcatggtcgtggtgtggatagcgggcgaaattttggcacgtatcagactgacgatttcaaggcgcacaatcatccgccggcaaataatcgtccgggcttcatgactaatgagtttccaacggttcaggcatatcacgcagccacttcggggggacctcaatcctactcgggtgaagggcaacagattgctacgacgggtaaccggggaggcacggaaacccgccctcgcaacctcgccgtcatgtggtgcatcaaggcctggaacgcgccgatcaatcagggaagcatcgatgtagctgcactggccaaggaagtctcgcagctgaaatcgtctgttccggtaggtgctgttctgtcgtttccaacgggtgtcgttcctgccggctatctggaactggatggcagtgtgcagagcattgcgacctatccggatctggcggcgtatctcggtacgacgttcaacaagggcgatgaaggtgccgggaatttccgcttgccggaatctcgcggtgaattcctgcgcggctgggatcatgggcgaggtattgatatcggtcgtagtgtcggcagttatcagtcgggtacgaaaactcagggcgatgacggcacggcgccggctgttcaaggtatcggcaactccaatctgattgatgctgatcctgctcctggcttcagtggcgatatttactacacctccaccaatgtcgtcgtgcagaacttttccaactcgttctggaaaacggttcgcccacgcaacctcgcggtcatgtggtgcatcaaggcctggaacgcaccggtcaatcagggaagcattgatgtcgcagcattggctgcagatgccaggtcggctcgactcaacggtgcagaagtcggcgccgcgcgtaatctgagagtgtcgctacccgctgctgcatcggttgcaacgcttacggccgaccaattgattgtcgagcaaccaggcgttggccagtacaagctatcgaacgtcaatctctctataaatctagccaccattggtgcgggcggaatggacttcggcgttgcaccagcaaacggcagtgttggcatttacgttatttacaaccctgagttgaaggttgcaaagctgctgggcgtcaacgcgacatcgacttctgttccggaaatttacactggcaccaacatgcccgtcggttatagcgccagtgcgctggtcagtgtgtggcaaaccgatgccaatcgattgatgaatgccggcattcaacatcagcgttcaatttccatcattcagacgatggtgctggaaaacggattatcgatgtcgtcgacaccgatctcgctggcctctgtcgttccgaagaatgcgaaaagtgtcggtggttacattcattacattggaagcgctgatttcccgggtggtggctctctggggctttcgccggatgtcaccgaagtggggctgaaagcatgcggcatcggtggaatcgtcgggttgggtgttctcagcccgttttcggatctggtcatgacgactccacagaccatctattaccgcctttatgcgtcggtttcccgagcaaacgatgtccacatctcccaatacactttctaaggagtcctctatgttgagagcctactcaaattcagggacggcctttcgttgtgtcgccccggactggccgctatctgacggtgaagtactgtttgaccatgaacccaccgtccaggaactggaggacgcatttgggttcgcgaacggcgagctggttgtaaagcgccaatgggaacagattgcagaagaacgattccgtagagagggttcgggcatcgtggtcgcgggtgtcgctatcgatacgtcccgtgacagtcagtcactgatcgccggtatggcagtttctgcgatgctcgatcctgagtaccactgtagctacaaggctatcgaaggatttatcgatattacctctcagcagatcctgcaaattgcgcaggctgtgcgttctcatgttcaggcttgcttcgatcgggaaaaaacgttgtacgaatctgctcaagcaggcacgtatagcagagaaatgctgaccgaaggatggccagattcctcgcctgaaacaccaccgaaaaaccttcaataaccccctgcaatccagggcgtttacttgctaaccaacacccgccagcccctccccacgaggggctttcccgtttatggagaaacgaaaaatggcaacccgccaaacctacaccgtgctcgttccattccccaccggcggtgggcactggtcgagcgtcggccaggaactcgatctgctcgacgtcgaggccagtgccctgcacagcgccggtcgactggagctgaaaacacctaccaccaaggccgtgaaggccgctgccaagaaggctgactgaatatggctgaggttctgaacttcgagcacaacggcattaccgtcaatgccaccgaatcccccgaggccatgggtggcctgggtgacaacgtcatcggtctggtcggcactgcgccgaaagccgatccgctgattccgcgcaacgcaccgtttcgcatcaacagcttcaccacccacgcgctgctcgatccgaccggcgcggaagagggcactctgtaccatgccgtttaccagatcctcaaagtggtcaaggtgccggtgtacgtggtgatcgtcgaggcgggcgcgaccccggccgacaccgtcaacgcagtgatcggcggcatcgagccagccaccggccgcaaactcggtctggcggcactgggcagcgtcccggaagacctgaccatcatcggcgcgccaggcttcaccggcaccaaagcggtggccagcgagttcgcctcgttcggcaagcgcatcaaggcccgtgtggtactggacggcaaggacgcttcggtcgccgaccaggtgacctacagccaggaactgggcggcgccgacctcggtttcgaccgttgcctggtggtgcacaacatgcccgccgtgtactcgaaagcggcgaagaaaaacgtcttcctcgcgccatccagtctggcgattgccgcgctggccaaggtcaagcaatgggaaagcccgggcaatcaggtgacctacgccgaagacgtgtcccgggtcgttgagtacaacatcctcgacacctccaccgaaggcgatctgctcaaccgctacggcgtcagctattacgcccgcaccgtgctgggcggcttctcgctgctgggcaaccgctcgatcaccggcaagttcatcagctacgtcggtctggaagacgccatcagccgcaagctggtgaaggccggccagaaggccatggccaagaacctgaccaagtcgttcatggatcaggaagtcaaacgcatcaacgactggctgcagaccctggtcgccgacgaaaccattcccggcggcagcgtctacctgcacccggaactcaacagcgtcgagaagtacaagaacggcacctggtacgtggtcatcgactacggccgctacgcgccgaacgaacacatggtttatcaactcaacgcccgcgatgaaatcatcgagcagttcctggaggacgttctctaatgtttaccaaccgtaatcgccaggccatcgcggccaccctgcaaggcctgccgctgtcggcgaccgtggaggaattcactccgccgaagatcgaattcgatgtagaagaaatgcgtggcggccgcttcatcgttgaagaaatggtcaagggcggcaaagcgctcaacgccaagttgaccctgcaaggcatgggcgccgaggtcatgcttgcactgggtgtgaagctgggcgacgacatcctgctgaacgtgcgtgaagccggtcaggaccaggacggtaacacctggttcacctaccacacggtcggcggcaagctgaaatccctggaggaaaccgcggtgaagatgggtgaaaaacccaagaccaacctggagctctcctgccgtacttacaaccgtctggaaaatggcgtgccggtgatcgacatcgacgtgcgcacccagaagttcgtactcaacggcgtcgacatcctcggtgatgcccgtcgtgcggtgctgatgccgtaagcctttcggcgcatcaagcacaccctgtgggcgcttatgcccacagggatcttcaagaacacccaaggaattcctttcatgtcgtggatgccacccaagcatgacctgttgtcgccgatcaccggtgacgacggctcgcagatcgaatcgatccagctcaagcccctgttctacgccgcccagaaagaagcgctggaacgcgccggcgatgacgaagacgatcagttcttcgaactggcgctgctggccaccgggttgtcggtcaaggaactcgaccagctcaaacgtccggactacgtgagcatcgcgcagtacgtacacgagatgtcgacccgtccggcgtcgtactttctcgaccaggtcgaagacgcggaaaagtccgacgatcccgaccaggtgcaactgctgcaaccgctcgccgtcaccggccgcaccgtgacctcgctgagcctggaaatgccggcgctgcgggccaccaaagtgatgaagaaactgaaaacggccaaggaacgcgccgagttcatcaccgcccattgcaccggcctgatgatccccgatctggccctgatgagcgtcccggactggacgcaattgcaggtgcgcatcgacgattttttaaaccagccggcggccttctttcagagcgcgacatcgaagtaatcctcgatatcgtgccgctcatttacccggtaagtgaggcggaaattctggagtgggacgccgaaaaggcgttgcgccgctacgacatagcgatcactcgccttggcgtgaaacaggagtagagcggcatggcacagagcaaatttgcgctcacatacgccaatgagagtggcaacgcagcagccgggttaaagctgcccgatggccttggcaaaccactgcaggacttgaacctgacaatggcgctggcgagcgcggatatccgcttgctgacccaggagcagatcaagcttcgagagctgttggccaatcagcaatcgctgttcaaggtgagtgctgcatccccggctgcaagcgccgaaccaaagtcaaaactcaaggccgagatcgagcagcgtccacctccaaagctcatgcaaccagccatggccaacgagacggcgcttgtcgaactcaatcagttgctcaaactgagcaatgatcagcttcaagcgcactcgcagagcactctggaactcgccagcgagaaacagatatccgccagtggtgcgaccaacgcggatctgttgcaagtgcagcttgccggagccagatccggcattgccgatggtgccaaaggtgaccagcgggcgaacgcactgaagtggttctcccatgatgccgcaatcaacgcatcggcattcaggatggacgtcaaggcggctggcgaaatgctcgccgcatggcgctcctcgctgaagctggatcagtatcaaagccaggatcttgcggatgcaacgacctacctcggcaatagtggtctggatgccaaggccgcggacatcggttcggtggtgcaacgttccggtgagagtgcgattgccgccggattgactcccgaacaggtcgctgcattggcggcggcgcttctcaatagtggtgcggacaaggagggcgccagcgccgcgctgaaaggcatcacctcgatgctggccaaaggcggtgcggtatcgactgagcagcgaacagccttgactcagttagggcttgatcctcaatcgctgtctgagggtatgaagaaggatgcgcctgctgtcatcaactcggttcttgctgcacttaacaagcagcctgtgcaagagcgggcggcactgacgaagacgctgttcggcgaaaacgacaccagagttctcgaactgctgaagaagccggacgatgtaaaaaacgccttctcgctggtagccgacaagcacaagtacgcaacaacggagcttggcgcgggtgaaggcgctgcggcgaagtccgcagaggcgttcggcaatacttcgcagggtcgctggaatgcgctggacgcaagtctgacccggttgaccacatcattcggcacggcgcttgcgcccctggctgacggtgccgccgtcgtgctcaccgccctggtcaacggtgttagcgcagcggcggaaacgttcccggcactcacggcaggactggctctgctcgccgtggcagccatgccgttcgtggggggggcgttgaagtccggcgtggcctcggtgctcgacgtggtttccacgaaactattgcgcctggcatcgacgcgactgccgccggatattgccgatgtgataggcggtgatgacaacgatgacgacggtcgaaaacgcagaaagaaggggcgcggatcgcgccgacgccccccttctgctgcacggtcgtccggcaccgcttccataacccgcaagagcagtcgcttgagtggtgtgacggccagaatcgcacccatgttcgacgatgcgctcacccgattcagaatggttggcgatgttgtcaaaagcgccatgccgagccggctgagcggggctggcgcgaaagtcatgtcgttggcagagggcttgggagccaggctcatgccctcggttgtcaaggcattgcctgtcatcaaggttggcgcgcctctggccattgctcatgctgcctatacagggttgaaaggttggcgcgaaggtgacgacaaagcggtaaagggcgcggccggcgaactggccggaacggcgattggcgctacgatcggtacgttcattgcgcccggcatcggaacctttattggtggcacgctgggtggaatagccgggtccattctgggtcaaaaactggcgacgccacctgaagacaaattggcaccgccggcacaggtcgccaaagacgtatccattgcgcaaacgcaaatgcaagcgtcaaacccgcaatacacttacgcaccttcagttcatgtcagcggcagcgaactggttagttccgagaaagtcggcacgatgctttcgcaggtgctggagtcgcacttcaattctcaatttgtcccgggtgtggctaccaatgccctcgccacccgccgtgacgcagccctgaccgatggagtcgcctgatgaaacaacaaatggcactgggcagtttcatcttcggactgtcccgggattttgcgtacagcacgctgtcgcgaaaatccgagggtggctggaccgagctgcagatcctcaacagcaaacccagatcccatcagacaggacagaagcctgaaaccctgaccatctccggaacctcgatgtacgccgtggcgatggagcggctcgatgagctgcgtgcgctgcaagcgttgagagtaccgctgccgttgattgacggcatcggtcgtaactggggtttgtggcggattaacagcatcgacgaaaaccagagcgaggtcatcgatgacggaaccgcgatggtgatcaagtgggtcatcggattgtcggagttcaacaatgcgtaaggtacgaagcgtggccggcgattcggtgaatctgttgctgtaccgcgaaaccggtcgcagcgatgacagcgccgaagaagccctgtggacactcaatccgaccctggccgagcacggtccgattctgtcggccggtgtctgggtgacactgccggaactcgatagcaaaccggccgcgatcaaaccggttctggcctgggattaaggaggcagcatggcacagggatttacgccggcgatcgaaatctacggcgccaacaaggacctgctgaaccagcgcctgatcagttgggaacacatcgatgctgccgggatggagtccgatcaactgacgctggtgctcgacctggaaggccttgaaggcttgccaaccctgggcggaatcatcggcctgcgggtggggtatctggagaccgggctggtcgaaaaaggccagttccgggtgactcgattgacaccgacgctgttcccgctgcgtctgacgctggtcgcgaccgccgcacctttcagcggcaaggacgaaaccggattcaaggaacgacgcacggccagtcatggccccacgacgcttggcgggctgtttcgcaaactggtcgagccgcacggtttctcgccgcgcgtcgatcccgaactggcgctgatcaggattgctcatgtcgaccagtcaaatgaaaccgacatgggcttcatcacgcgactggcgaagaagtacgacgcggtggccaaaccgttcaacgacctctacgtactggcgaaaccggcgcagctcaaaaatctgtcgggtcaggtgataccgaatgtgaggctgtcggtgacccacaacaatcggccgggcgaacacgccttcatcagcgctacgctggaagagaccgcccgcacccagaatgaaggttgcaaagtctgctgttgggacgccaatgccggcaaacaggtggaggtgaaaaccggctcggcgccctacaaggtcgttcgtcagaaacaggccagtgtggaagaagccaaagccatcggcgaagccgaagtgcgcaagatgctgcgcgagaaatacaagctgaaggtcacctgcccgggcgatccgctgctggttgccgagggcctgctggtgctcgatgacacctggccggacttcatgcgcggtcgctggtcgatcgagaaggtgacagccagcggcaagcccgaagaaagctatcgctgcctgatcgaagcaaacggccgggatcccgaggcaaaagccaaggactgatcccccgatctcaccaccacactcctcac

SEQ ID NO: 2 - DNA, 17469 bp, Pseudomonas fluorescens Ps36
  source 1..17469: mol_type = genomic DNA
ggtggtcactcccaaaacctggaacgctccccatgaagatctccccgatcctcacgcagctgcgtgcgcaatgcccaagccttgccggccatatcgcgacaggtgtcgacctggcgctgctgcaaggcaacccgaatctgccgaccccgtcggctcatgttttaccgctggccgatctggccagcgccagcaccgcacagaattccgccagtcagccgatccgcgaccgcttcgaaatcatcctggcacttgatgccacggacgccacaaaagcgctggatctgttgcacgacctgcgcgccgaagtgtggcgtgcgctggtggggttcaagcccggttccgactacagcgccatcgtttatgacggcggcgaaacggtctcgatcaacagcagccgcgcgttctaccggctgcgcttttttgccgagttccagctgggccgcaatctgccaagtcagcctgcggagagttggcacgaacgtgaactggacggtttgtcgtcctttaccggggtcaccgtgcgggtcgatgcgatcgacccggccgaccccaacctgaaacacccgggccctgacgggcgcgtggaaatgactttctctggagacgtaaccccatgagcaaccgcatcaccgtagtgccggccactggccgtgccgtgccggacccggaagcaggcgacctgctgccactggaaggccgtgaagtgctggacagcgcctggtggcgccggcgtctggccgacggcgatatcaccctcaaaaccgcaacagctaaacaaaagggagccaaataatggcgatcggattcagcaacattcctgcggacattcgtgtaccgctgttctatgccgaaatggacaactcggccgccaatagcgcgtcctcgtccatgcgccgcctgatcgtggcacaggtcaacgacaacatcgccccgagcgaagtcggcaaactggtgctggtctccagcgtggcactggccaaaagcattggcggccagggctcgatgctcgcctcgatgtacgagaccttccgcaaggccgacccgatcggtgagatctggtgcctgccgctgcacaacgctaccggcgccatcgccaaaggcgtgctgaccctgaccggcaccgcgactcaggctggcgtgctcaacctgtatgtcggcggtgtccgtgtgcaggccaccgtggtcaacggtgccacggctgcccaggcggccaccgccctggcacagaaaatcaacgccaccgccgatctgccggtgagcgctgtggccgctgaaggcgtggtcaccctgaatgccaaatggaccggcgagagcggcaacgacatcagcctgcaattcaatcgcctgggcaagagcaacggcgaagaaaccccggccggcctgaccactgccgtcaccgccatgaccggcggcgtcggtgtaccggatcaagtggcggccgttgccgcactgggtgatgaaccgttcgaattcatcgcgctgccatggtccgatctggcgaccctcaacacctggcaagcggtgatggacgacagcaccggtcgctggtcctgggccaagcaactgttcggtcacgtctacagcgccaagcgcggcaccgtcggcactctggtggcggccggtcaggcgcgcaacgaccagcacatgaccattcaggcgctggagcctggcgttccgcaaccggtgtgggtacaagccgctgcactggctgcacgtacttcggtgttcatctccgccgacgccagccgtccgacccagagcggcagcctgccaggcgtcgatccggcgccggccagcgagcgcttcaccctgaccgagcgtcagtcgctgctcaactacggcatcgccaccgcgtactacgaaggcggctacgtgcgcatccagcgctcgatcaccacctatcagaagaacgcttacggccaggccgacaactcgtacctggacagcgaaaccatgcaccagtcggcgttcatcgtgcgtcgtctgcaaagcgtgatcaccagcaaatacggtcgccacaaactggcctccgacggcacccgtttcggcgccggtcagccgatcgttaccccggcgaccattcgcggtgagctgatcgcccagtacgccaagcttgaactggaaggccacgtggaaaacgccgagctgttcgccgagcacctgatcgtcgagcgcgacgtgcaggacccgagccgcgtgaacgtgctgttcccgcctgattacatcaacggtctgcgcgtgttcgcactgctcaaccagttccgtctgcagtacgacgacgtcgcctgatcggctcgtttgacactgtgatttcagcccacctcgcgtgggctttttatttgaagggagtaacaccatgggtcaactgattgcaggcacctgctacgtcaaggtcgacggtgcacaactgaccatcaatggcggctgcgaagccccgctgatggccgtcaaacgcgaaaccgtcgtgccgggtttctacaaggaaaccgacatcgcgccgtcgttcaaggtgaccgcgctgcacaccgccgacttcccgctgaagaagctgatcgaaggcaccgacatcaccgtcacctgcgaattcagcaacggcaaagtctacgtgctggccggtgcctacctggtcgaagagccagtctccaaaggcgatgacgccaccatcgaactgaaattcgaaggcatcaaggggacttggcaatgagcggcgccgtgaagcttcaagttgcgatcgaagctcacggcgagcccctgaccgaactcgtcctgcgccgtccgacggtgcaggaggtgcgagcgatcaaggcgctgccgtacaagatcgacaagagcgaagaggtcagcctcgacatggacgtggcggccaaatacatcgccgtgtgcgccggcattccgccgtcgtcggtcaaccagctggatctggctgacctcaacgcgctgagctgggccgttgcgagttttttcatgagtgcggcgtcggagccatcaccgacctgatttcggtcgcctatgacctggcctggttctggaaggttgaccccgaacagatgatggccaggccactggatgtgcttcgcgaatcgctggagcacgcgcaacggatcaatgcgatgcagcaggtgcagtgatggcagaagaaaccaaagcgaaagcgtcggtgctgcttaccggcatcgacgaactgtcacccaaactcggcgccctgcgagtgaaggtcgatgacttcaagaagaacctcgaacagaccggcctcggcaaactggacatcagcggtctgttcaagggtgggagcgtgattacgccgttcgtggacggcatcaaatccgccgcagcgtttcagggcaagttgaccgaagtcagcgagacggcgaaaaccgtcgatctgccggaaacaccgaaagccgccgcgcagaacatgaacgtgttcagcgcgtccatggaaagggtctccgctgcggtagacgccgcattggtgccggcggtgggcgccttggtggtcgggctggagccgatgctgacccaggtcggcagcctgctggccgacaacccgaaactggtcgaaggcctggcagcgggggcgattgcgttttccgccatgcaaaccgccgtcaccggtatgacccaggtgatggacgtcatgagcatggtgctcaagaccaacccgatcatgctgatcgccatgggcattgccgtggcggccggactgatcgtggccaactggacaccgatatccgcgttcttcaccggaatgtgggagggcgtgaaaaatgccggggccagtgcaatggcgacgttgcgctcggtactcgactggcgaccgctggaaacgctggcagcgctgtgggaaccggtcacgggtttcttctcgggtatctgggacaaggtcaaagcggtcacggcgccggtgatcgacttcttcaagtcggttttctcgtggtcgcccgcgggcctgatcctggaaaactgggggccgttgaccggtctgttttcggcgatctgggaattgctcaaggccttgagtgtgccggtgatgtcgttcctcaaggggctgttcgactggacgccgctgggcatgatcatcaacaactggggcgcaatcaccggtttcttcgcctcgatctgggtcgcgctgcaaccggcggcgcaagccatcaaggacttcttcggcagccttttcgattattccccgctgggcatgatcatcaacaactggagtgcgatcaccggcttcttcgcttcgatctgggcggcgctgcaaccggcggcgcaagccatcaaggacttcttcggcaccctgttcgactattccccattggggatgctcgtcaacaactggggcagcgtcgtgacctttttcgaaccggtctgggccgcgctgcaaacgtcggcacaaacgatcaaaagcttcttccagagcctgttcgaatggtcgccgctggagcagatcgcgcagtactggcagccgatcagcgaagtgttttcggcgctgtggggcgtggtgcaggcattggccgcgccggtgctggagttcctgcacaacatgttcgaatggacaccgttggggcagatcatcaagaactggggaccgatcaccgagtggttcggcgagctgtggcaaaagctgcaaaccgtcatcgcaccgatcaaggagctgttcgacggcggcttcgccgggctaatcgccagggtcaccggcaaggtcgaaaccttgacccaggcgcaacgtcagaccaatgccgaaggcaagggtgaactggcgccggccttctttggtgccagcccgaaacccgagggtggcagcgcgctgcagggcggttctttgccgcaatcctctggcgcactgatccagcaaagcgccgccaataaccgcacgcaactcgaaggcggcctgacggtccgcttcgaaaacgcgccggcgggcctgcgcaccgatcaaccgcaaaccaatcaaccggggctggcgctcagttcgcgcatcggctatcgctcgctatcggcaggaggttccaatgaactggcgtgaccgtttgttgccggcatcctttcgcggtgtcggcttctggatcgaccaggcgaaaaccccggtcggtcgcaagggacagttgcatgagtatccgcaacgggacctgccgtttttcgaggatctcggccagcaggccaagacccacgacctgacggcgttcatcatcggtgccgattgcctggagcagcgcgacaagctgctccaggccctggagcagggcagcggcgagctggtgcatccgtggctgggccgcttgcaggtcaaggtcggtgagtgcgacatgacccacacccgccaggacggcgggatggtgaccttcaccctgaagttctacccggaccggccgctgccgtttccgacggcgacggtcagcacgcaaaaagtcctgctgatcaaggctgacggtttgctcgggtcggcggtggcgcgctttgaacaggcgatgaccctgatcaaggccgcgcggatcggcatcgccaatctgcgcaacagcctcaccggcgtgtacgacgtgatcaaggagcagctcaagccgctgatcgcgcaatacaagcagatcaccgaactggtcagggccgtcaaggaactgcccaaggaagtggcggcggagttcaaaggattgctcggcgatatcaaggagctgaaggcattcgcgaaggagggttaccgtggcgtgattgccgacgtgtcccaacagatcgaagccatccgcaaggccgacgccccgaagatcaccaccggcaaggacaccacggctgcggcgcaggccctggccaatctggtgcaggacacccttatcgtcaaagcggcgcaatgggtagcctcgatgccggtggcctcgacgccggtgaaactgtcgtcgacgccgtcgctggatcagcagtcgaaacagccggtcagccgtcaggaagtgccggtcaccgacgatctgcaagcgttgcaaaaagagctgatcgaagcgctgcaaaaggcccaggacaaggccgatcccgcgcactaccaggccatcgccgatgtgaaggaagcgctgatcgcgcacctcaaggctgtggcttcgtccggtgtgcggctggtgagcaaaaccttccaggaaacctttccggcagtggtcgtggcttacaagcagtttggcgatgccacccgtgtgaccgaggtcattcagcgcaatggtctgtctcatccgagcttctcacccaacgaagtcaaggtttccagggagtgagtcatgaacgagactgacaaccgcgtgacgctgaccgtcggcgacatggaatacggcggctggaaaaacgtgcagatcaccgcggacctggagcgccagttccgcaccttcaaactcgatatcacctggcaatggccggggcagaccgtggatcagcggatcaaggccggcgacccgtgcgaagtgcggatcggcaaggatctggtgctcaccggttatgtgttcaaggccccgatcagctatgacgggcggcagatcagcctgagcatcgaaggcagttccaagacccaggatctggtggattgcgcagcgcgaaacaaccccggccaatggcaggatcagtcgctgctgagcatcgtccaggccctggccatggagtacgcgttgatggtggtcaacgaaattcccgagaccgcacgcctgagcaaacacacgatcgtaccgggtgaaacggcgtttcagtcgatcgaccgtctgctctcgctgtaccgggtgttttccaccgatgacgccgaaggccggctggtgctcgccaaacccggcagcgctggccgcgccagtgacgcgctggagttgggcaagaacattctttcggccaatgcgccgatggatttcagccaggtgttttccgagtaccgggtgatcggtcaacagaagggcaacgacaagaagagcggggcggcggtcagcgaagttgaatcgacggcgaccgacctgagcttcaagcgtcggcgcaccacgatcatcaacgaaggctcgcaactgacgttcgaactggctcagcaacgggcgcaatgggagagcgcgacgcgcatgggccgagcgctgaccactacctatcaggtacagggttggcgccagtccaatggcgatctgtggcgtcacaacacgttggtgcgggtcaaggatccggtgctcggattcgatgaagacatgctgatttccaaggtgacgtactcgctgtcggcgcagggctcggtgaccaccctgcaagtggcgccgccgcataccttcgacgcgaacccgactcccccgaaaaagacctgagcccgaccccgccctccaaggaaaaccctatgagcctactgacacgcctgctggcgcgcggcactgtcgtgctcgccagttcggcctccaagctgcaatcgctgcaaatgcgcctcaccgccggtgaagtgaacgacgacatggagcacttcgagccctacggctttaccagccatccgctggccggtgccgaaggcgtcgtcacgtttctcggcggcgaccgttcccatgccatcgcgctggtggtcgctgaccgccgttatcgcctgcaatcgctggcggccggcgaagtggcgatctacaccgacgaaggcgacaagatccacttcaggcgtgggcggatcatcgatatcgaaaccgccacgctgaatatccgcgccagtacggcggtgaactttgacacgccggtgatcaaccagaccggcaagatcgtttccaaaggtgatcagctggccggcggcatcagccagatcaaacacgtgcatggcggcgtgcagggcggcagcggccagaccggtgtgccggcgggaggtcagtgatgcttttcagtcaaaacctccacgccgcgctgacccgctcggtgctgatcagcctgttcacctggcgccgcgccgccgacgacgatgccctcgatgacgaggagcgttacggctggtggggcgacacctttcccaccgtggccgacgaccgcatcggttcgcggttgtggctgctgcgccgggtcaagctgacccgacagacccagatggacgccgagttctatgcccgcgaagccttgcagtggctgatcgacgacggccattgcagcgccatcgacatcatcagcgaacgcctcgacgcccagcgcctgaacctgcgtacggtcctgaccctggccgacggcgaacgcctggacatcaaccccgataacagttggcaggtgatctatgccgtttgaaaccccttcgctgccggtgctgatcaagcgcacccaaagcgacctggccggcgattcgctgcgccagtccgatgcgcaagtcctggcccgcaccgtcggtggtgccgcttacggtctgtatggctaccttgactggattgccgagcagatcctgcccgacaccgccgacgaatcgaccctggaacgcatcgccgcactgcgcctgaaccagccgcgcaaaccggcgcaaagcgccaccggcagcgtcagttttactgcaaccgcgggcgcggtgctggacgttgatacgctgctgcaatcgagcgatggccgtacctacaaagtcaccactgcgcgcaccaccgtcaatggcagcaacaccaccaccatcgcggcgctggatgccggcagcctcggcaatgctgacgccggactggcgttgactccggtgcagccgatcaccggcgtggtcggcaacagttttgtcgtgctggcgccgggcctcagtggcggcgtggcgcgggagagtctggagtcgctgcgttcgcgggtgatccgttcctatcgcgtcatcccccatggcggttcggccagcgactatgaaacctgggcgctggaagtgccgggcgtaactcgtgcctggtgccgaggcggcctgctcggcccgggcacggtgacggtgttcatcatgcgtgatgaagatccgcaaccggtgcccaacgacgagcaactggcggaagtccaggactacatcgaaccgctgcgaccggtgacggcggaagtgcatgtgcagcgaccgattcaagtgccggtggtgtaccgcttcaagagcgtcaacccggacaccaccgccgtgcgcgccgccgtcgaagcgcagttgcgcgacctgcacaaccgtgaagccgatctcggcgtgccgttgctgatcagccatatccgcgaagccatcagcagcgccggcggtgagtacgatcacaccttgaccgcgccggccgctgacgtgcctgccggtcaaagcgaactgctcaccttcggaggttgcgtatggggggcataagaaccgctgcgcaatatcaggcgcagcttcgcgcactgctgcccagcggcccggcgtgggacccggagcgggtgcccgaactcgatgaagtgctacaaggcgttgccgtcgaactggcgcgcctcgacgcccgcgccgccgatctgctcaacgaaatggacccggccggcgtcagcgaactggtgccggactgggaacaggtgatgaacctgcccgacccgtgcctcggcgccacaccgctgttcgacgaccgtcgcctcgccgtgcgccgccgcttgctggcggtcggtagccaggccgtcggctactacctggaaatcgccagaagccagggctaccccaacgccaccatcaccgaactcgaagccccgcgcatgggccgctcgcgcttcggcgcggcgcactggggcacctgggaagcgcagttcatgtggacgctcaacaccggcggccgcttgctgctcggccggcgtttcggcgcgagttactggggcgaacgcttcggcgtgaatccgggctcggcgcttgaatgcctgattcaccgggcggcgccggcgcataccaaggtgcacatcaactatgactagggaataacgcaatggattatccgaagagtgtgcccagtgccggtctggtgaatgggaaatttgtcgatgaaaacccgatgaccgggacgcccggatcgttgattccggcggactggggcaacggtgtcacgcaggaaattctcagcgtgatcaaggccggggatctgaccccggatgagaagaaatacgatcagttgttgcaggcgattcagacggtgacggccaagggctggaatcaggatctggcgctgccgctgtcggccttgccgctgccaaccgttgccactacggatgcgcggatgccgatcacgccggccgccgcctcgaccagtggcgggcgggtgtcggtgccggcaggtatctacgtcagcattggccaggaagtagtggcggggcagttgggacgttcgcggacgttcaccactcagacctggagcagcgccgatctgttgccgagttctggttactttctgcgggcgcaggtggtgagtggtgcactgacgttctacatgcagcgcgggacgatttacgacgtgacgcccgattccctgaagggcacggtcaacggtgctgccggcggtggtttccagagttcggtgctggacatgtgcctggcctgggtggttaccggtgcaccgggctcggtaccggtagtgcgtgcgatctataaccgggcacgcctgacctgggcgcagacgctcaacggcacgggggcagtgtttctgccactggatcctcatgcccgcgctgcgcgactggtggtggggaacccgacgccatcgtcgactgctgttacaacggttgcgtttccttcgactggatgggcgggtggcaactacagctacctttcgcccgtatccacaggcgtttccaataatgccggaggctggaatcctgccaccgcacaaccgtgcgtcatcttcaccaacaacatcgtcaatgacgtcacggtttcgacactgaccgccagtttcgatcacgccaatgtgcgctcgctctggcagtcctatcaggccgaacacaacctggcacaggccagcgccgacagcgatgagctgttgctgagcatgggcatcaagagccatccggtgaccgattacaacgccggtattccgatcaactttagcgaagctgtgaacgttcagctgtcgtgggagctcattcgatgatcgtcattcaggaactgcatcagatcgatggagagttgcgtcctgcgcagccgtccgccgcccatgactgggacggtgaacaatgggtcgtcaaccctgagaaagtcgcgctgctggaacaacaggaaactgaaagcctgtgtgcccgggtcgatgttgccgccgacagtgcacgcagcgtattggccggggatccgctcaaggcgttggagtatgcccaggcagccattgatgctcaggcctttcaggacgccggttatccgaagaaggaagtgccgctgtccgtggccgcgtgggtcgccaaaggccggtcggcgaaacaggcagccgagcagatcctcgacaaggctgctcaggtcagcgacagcctgttgaccctgcgcaccttgcgcctgaaggccaagacccagatccgtgggtacgccggcaaaagccagatggatcaggcgcgtgccgccacggacgaggtgttgctggccattcgtgatctgacggccatccagagccagtaaccgctatccgcctcacccaagcccacgtcagcgtgggctttttattttcaggaacagaagcgttggaaccgctgcgaaacccttcgcgccgccgcgtttcatttgtcatgacagaggaacgaacatcccatggattatccaaaaagcgtccccagcgtcggcctggtcgacggtcgcttcgtcgatgaaaacccggtggcgggaacgcccgggtcgttgattccggcggtgtggggtaacagcgttacacaagagattgtcaacgtgatttccggcgccgggatgaccgccgtcgaggccgataacggccagttgttccaggccattcagtcgattgtcggcaaggcaagtcctatgcgttcggtgatcacacggctggcagcgtccaaagcgctgaccgaacaagagcttggccttgtgctgatcgacagcagcccggcagccactacggtgaccttgccggcagccagtctcggtctgggcgtgcgtgacgttatcgttcgccgtgtcgacaacagtggcaatcgactggttgttcaggcttccggtacggaccgcattcgccttcatacacacctttcgtccaatggttacccctttctggtgctgatgggcaatggcgactggtggcatctgcgcagtgacgcagcgggtagctggtggcctgtcgggcgcttcgacaacacaccattgggccgaccggttttcgagaccaccactgtgctggggccgggcggttacggggcgcttaacggagcgttcctcgatcgggcgcaatggccctggctctgggattttgctcaggcgtccggcgtgctgaccaacgaagcggggcggtggggcagggaaggggcgtggaccagcggcgatggtgcgacgaactttcgtatcccggaagcgcgcggcgaatttctgcgcgtactcgatgaagcgagaggcgtagatgtcggtcgtgtcgcgggcagccttcaaaaccatgcgctgcagactcataaccattatctgcccaccagcacaggctcgttcgggcgtcccgctccctccattccggacaatctctggagtgtttcgtctgacgtcaacttttaccccaccaatggaacggtcgctacgacgtatccgaacccggcattcgactccgatacctacatcgggtcgatcggcaatttctcatctgaaacccgcccgcgaaacatcgcgtatcccggccgtatcaaactgatctgaggcacacatgttcaattatttgatagacgacagcggtgcgctgaccgggcctgtcgagtttccgctggtgccaggtatcggcgtacagctgcctggcaacgccgtgacgttgagtatcgaactctctgcggcaccgaatggatatgcctgggcctacgacaacggttctctgcagcaaaaactcgactttcgcggtgatgtttatcacaccgatacgggcattcgggaaacctggaccacgttgggtgacctgccggagggcttgaccacgcaaccatggccgggcggattccattcgtgggtcgataacgcctggcagctcgatgaagccgctcgactggcggatctcaaacggatcgctctgacccggcgcgacacgctgctgcgcgacgcggtcctgcgcatcgcccccctgcaatatgccgaagacatcggcgatgccagtcacgaagagcaactgcaactgctcgaatggaagctctactgcgtggaactgaatcgtatcgaaatgcagaccggtttcccggaacaaatcacctggccggcagcacccggcgcaaccgtaatcagctgacagaagcacagggaacagtgcaatggactatccaaaaagcatccccggcgtcggcctggtcgacggtggttttatcgatgaaaaccccattgccggcacgccaggatcgttgatccccgccgcctggggcaacagtgtcacgcaagaaattctcaacgccatcaaggcagccggactcaccccggacgagagcaaaaccaaccagctggccacagccatcggtgcgctggtcgacttcaccaaactgaagaacaccccgaccacgctggcgggctatggcatcaccgatgccgtggggcggttgctggcggttcggcagatcgagacggtcgggatcacggtttacaagccgaatccgagggcgaagcggattcgtgtgcgtctggtcggggcgggtggttcggggggcggatgtgcgcctgtaccccccacctatcaaagcttcggaggcggtggtggagcaggagcctatggcgaaagcctgtttgatgtgacggcggaaatgcaggctggtgttcctgtttcactgggtgccggcggtgccgcacgcaccgcgatgggtgtttcgggaggcggtgcgtccttcggcagttacatgagcgttgcgggtggcgcaggcgggcaaaccctgtcgatcgtgctgacgggaacttcgtccggttgcgtccagggtggtacgggtgggcaatcggtttctggcgggaatctcactgctgcgcgtggtcagccgggtggttatgccatgagcaacgccaactggggactgctgggaggcaccggtggtgcgagccagttcgacggaggtgctccattcacgggcgcgaacattaatgcgaattccggttctcgtggttcgggtggcggcggagcttgctccaatagcgcatccgtcgcgtatccgggtggagtgggcggcaacgccttctgtgaaatctgggagtacgagtaatggcccgttatgcacgtattgaaaacggtgtcgcggtcgaagtgatcgacaccggtgactacgcgatcgagcaactgtttgcgccggcgttcgtcgcggcgatggtgcaggtgcccgaaggtgctgatgttgaaatcggcgcgccgatgcctgagttgacgcccgctgtcgagcctctgcgcgaaccgccagttcctgaaatcgctcaggccgcaacggtcgagggcaacacgtcttcgacggctgagcgcgcctggcgccagtcggcgctggcggccacggaatggttggtcacacgccatcgcgacgagcaggaactgggacgcggcaccacgctcaaggcccagcattatctggaattgctcgagtaccgccaggcgctgcgcgactggcctgactcaatccattttccggcagtagttttgcgcccggcagcaccggagtggatggccgccgttcatggctgaggtcttgttttgatgttcttgaatagggagaagagtgatggattacccaaaaaacattcccagcgcagggttggtgaatggcaggtttgttgatgaaaaccctcttaccggaaccccgggttcgttgattccggcgagctggggaaatggcgttacgcaagagattcttgaagtcatcaaaggcgcagggtcggctgccgatgaaagtgataacactcagctcaaggcggcaatcgatacgctgatctcgaagaaacaaagcgacagtctggccagccaggaagaagctgaggcgggcgtcagcaacacgcggttgatgacgccgttacgagtgtttcaatccatcgcaaaaaaaatgcaacaggcgaccgagtcgctgatggggattgcaaaagttgcttctcaggcagaggtcaacgccggtgccagtgatacgtctatcgtgacccctaaaaaactcaggtttgggttcatggtgaggctgggggcatccggttatgtcgttttcccctcgtggatggggggggtgattatccagtggatcaccggaggcgcgagccaggcgggcaacaatggctacggggacctgaatctatggccgttggtctttcccaacgcactgtttcttgccgtcgcgacccatgaaggcacggcacccggaacgcagctgacctggaacatcaacgcgaccgtgagtcggcaggcaggcatcaatgttcgttgtcctgaatggccgtcaggctccattgctgctcgtgtcatcggaataggaaactgactatgtattacttttctccggctacttccggcttttatcactccgatctgcacggcgccaatatccccgctgatgcctttgaattgagcgaaggtgagtattgcgcgctggtctcgaacgctccaaaaggaaccgttcttagcctgactgccaacggacgcccggaacgggtgctactggctgaacaaactctcgatgctacagagcgggtctggcgagacaaggtattggatcgaactcaatggctggttcttcgcgatgcggaagaactggaagtcggcgagggaacaaccctgcgcggcgaagagttcaagcaactgctcgcctatcggcaggcgttgcgcgactggccaaatgatccggagtttccggatgcgcgttcgcgtccggtagagccggattggctggaaggcctgctgcgagcgaacaactgagcggattgcccgatggggcaaaaccggactaccaaggaaaatcattatggactaccccaaaagtgttccggggtcaggtttggtcgacggcagatttgtcgacgaagacgcgatcgccggcacccctggttcgttgatacctgcgagctggggcaacagcgttactcaagaaattctcggcgcgattaccgccgccggccttaagcctgacgagcagcagaccgatcaattggcgcaggcgatccgtcaattggcaaagcccgatccactgcaacaatttccggtgcaggtgtatcgccggaacgtcctgatcaatggcgggtttgatatctggcaacgcggtccaaccaaccccgggccaaatattggcggctatgtggctgatcgttttcgttgcgactggaatggcagtgcaggagtcgccatatctcagcagggttttgcacccggtcaaacggaagtcgccgacgagccgcagtttttcctgcggtggcaacaaacccaggcgggaaccggagccaccgtacacagaatctcccaagctattgagtcggtacggaccctggcaggcaaaaccgccaccgtaacattctgggcgcggtccgatgcggcacgacagctaagagtgtcggtcactcagaacttcggatccgcaggttcagactctgtggaaaaaacggtcgatgtctttcaattgggcacatcgtggaagaagtacagtgcgtcatttcgtctgcccggtattgccgggaaaatgctgggagccaacaacttcgtgaggcttgcgttcgacttgccattgaatgttttgcagaccgtggatctggcacaaatacaaatggaggaaggaccggtatccacacctttcgaatatcgcccagtggctgaagagttgatgctttgccagcgttacttcgagaagtcctttgccacttggttgccggtacgggcgaacaatggttctaacacctgcatttcaacgttcacgcaagtggcgcctgccaataacggtcagttcgcgatgacgacaggcatgttggtgcaaaagagggtgttacctaccgtcgtcatgtattgccctggcaataccagcaatcaggtatggaatcaggccgtggggccatgtaccggcagtattgtgcagggattgacggagcgtgccatttcgttttccaccgttaccccggtcggcagcttgcccggtcagaccttgcagatcgaatggactgccgacgccgaactttaggagaaaccatgagttatcaattgaccgccaacggcgttcttcgtctgagcgacctggcatatgttccacaggatcctgccaatagggattggctggaatatcaagcgtggctgttgtccggtggccaggtgttgccctcgaatgaagcaattgaggaatctgcaccgaacagcaccctgacaactctggcaaaaaaatggctggggggcgttggtcgccagccgtgattcaatcggcgcaatccagggaggatcaagcatt

SEQ ID NO: 3 - DNA, 35013 bp, Pseudomonas fluorescens Ps36
  source 1..35013: mol_type = genomic DNA
atgcaaaaacgcaacgtatcctccgtcttaagagcgctgctcgatcagtacgggatctcccccacggagctccaccgtcgcaccggcgtgcctcaatccactctctcgcggattctcagcgggaagatcgtcgatccttcggataaacacatctcgaagattgccgagtacttcgccgtgagtaccgatcagttgcgcgggcgcgcggatgttgcgccggtcgccggcggcgggcgcgaggagttgcattccgaactcaaggacataagcctgtgggacgatgacacgcccgtcgatgacgacgaggtgtcggtgcccttccttcgcgaggttgaattggctgctggatcaggaagattcgtcatcgaagagagcgaacgctctagcttgcgcttcggcaagcgcagcctgcgccataacggcgtgcagttcgaccaggccaaatgcgtgaccgtacggggcaacagcatgttgccggtgctgcgtgacggcgccaccgtcggtgtgaacgcgggcaagtgcgggatcggcgacatcatcgatggcgacctttacgcgatcaaccacaacggtcagttgcgggtgaaacagctctatcgcctgcccaccggtatccgcctgcgcagcttcaatcgcgacgagcatccggacgaggactacagcttccaggacatgcaggaagagcagatcgtcatcctcggtcacgtcttctggtggggcatgtacgcccggtaacgatccctctctcagataaaacccgcccacggcgggttttttttcgcctgtagaaaaccggacaacccttgattggcggggcttccatgcatccgcgcatttctcatgcataaataaatgcatttacgcattgactggatatgcatacatgcatattcttgccaccaagccgctcgacaaagcggctggcaacaacagctctttagttccacaagaacaggcagcgatgaaccggcctcaacggttcagagggttggcaactgacccgggtgtgcagcgtaaagcaccagaagcagttatccggcgggcagggaccgcggtcggaaaaacaatttgaacggactcgtaccgcgccagtagcgccgaaaagtcagcttccttcacgtacacaggattgaaggaaggcgaaggagcgcattactgaaaagcccggcgagatgccgggctttttggaatgcctgtcctgggcgccagcatcgaaatccattgtgcccgcaagtgcgggtgggcaatgcacatcgataaaccatctaacagacaactgaaaaaaggaaaaaacatgcgccgatatggacgtgttgatcaggatcgaattgtcgagttttttgaaaccgacggtgacatcacgcaaatgtttcacccaagcattatctgggcagaagtgaccgatcaccccgaagtgcaactgggctgggtcgccaccaaaaccgacggtgtctggacctttgccgcctatgtgccgccaccgccgaccgagcaggaactcatcgccaaggcgcagctgaacaaatggcaactgttgaacgtggccgccaactggctgctgctcaactccctgcagttcaaggtcgacaccggtgtggccacccctgacgaacaggctctgttgctggctcacaagatgtactccatcgctgtcagcgacatcgacaaacaatcgggttacccggcaaacattgtctggccggtggctccgtactgacagtgtttgaaagacagcactgacgactatcaaatcaaaggaagcaagaatgaatcgctacatactgatgaccacggcctattcctacaaccttgtcctcgacgtggtggataccgacgggccgatgcctgaggtgccggcagatgagccctattcgagttggcaagactataccggtaacactactgcagagccgggtatgaaaatggtatggaacgggctaccgagttttgttccgacaaccgcaactgagcgggaggccatgaatcagggacgcatccaaacgcggcttcaggaggcccagagctggttgatgttcaatcccgtgcaatacaaatcggacctggggactgcctctccagccgaggaggccgcattgcttgcctacaagcagtacttcgtggcggtcgccgaagtgaaaaatcaaaccacctttccgaagctcaactggccggtcgcaccgttctgatccagcgagcttcaaactcgacatcgagaacgcattactgaaaagcccggccaccgcgccgggctttttggaatgcctgcctcgagagaaaacgattgaacccgacacacaccactcatccatcacaccaggaggcgtgacatgacaaccgagcaacaagcgttggcggacatgccgatctggctggtcatcctgcttgccgtggcgggcggggtctccggcgaaatgtggcgcgccgacaaggacggcgcccgcggctggccactgctgcggcggctggccctgcgctccggcgcctgcatgatctgcggcgtctcggcgatcatgctgctgtacgccgccggcatgtcgatctgggccgccggcgcttttggctgcctgaccgcaatggccggcgccgacgtggccatcggtctgtatgaacgctgggccgccaagcgcatcggcgtctgcgaagttccgcccgccaatacgaataaggagcaatgaaaaaatacagcggtatttgaaaaggagttcatttcatgttgagcgattttcgttgtggaaaatgcaatcggttactcgcaaaagtagatccacttcatcaagtgcaaatcaaatgccctagatgcaggacgttgaattacgcgaaaacgggatgctttaaaaaatcgcctgtgagcgaaccagggcagcagtgactgctaataataaataatcgacttataggtgatatatatggctacattgccgcgttacccctttacaaccgacggcagttcgattctgttgccgctgcatgaaatgtctgctggacaatatcttcagtcgccagacaagcgttttaaattgattgttcaacccgatggcaatctggcgatttacgaaggagcaaatacagtttgggtggcgattgccggccaaccctatacaagctccgggaagcagatagacaactcaaaaatttacttttatctgatgtattacgcgttcctcaatgatccaacgcgtggccgtatgtggggcactgctaacagcacacctctcaattctgatatctgggcggcttacaatcgtgcctatctatctctgcagaatgatggaaaccttgtagtggtcgactcgatccccgtctggtcaagcaactctgccattcctatcagtccatctgtggagtccgtatatattccggcaggtacaacgcttgaggttgaccgtcggtatgttgtgggagggacgactctggtcttccagtcggatggaaatctggtggtttcaaacggaccacttggagtcctgtgggcgagctggacccagaacaaaggtgccactcgtgcagtcatgcaggaagatggaaattttgtgatctatggacaaaacaatacaccgctctggtttaccggaactgccggtcagccaggtgcaatggcgaaagttcaggcaaatggcagtttctctattgtcagtgaaaagccggtttgggctcgatttggtttcacgccaactattttgccaaaacgcgtattccagtgggacaacggaccatggaaaccgctaatcgaaattcctttgtggcgttttaaagattaattattttgaaatttgcctcccgcttggggggcattttcataatgcttccatccgatgttttatgcgtgcttcacgaagtttcaatttgaatttatcgttgtttagctgaaacccgatatttcgcctcgctgcatgttctgcggcgggactgcgcgtggacattcaaaaaggaggtcatgcatgcctgtaccgatccgacagccttcgcagctgttcacggcaatggcgacagccttgcgcaataacgccgacctgaacgtgcaggtcggtaatcacgatgacttcaccgcacccggcgacaaggcctgggtgctgatcgacatcgaacgcaatgcaccgggagagcgcgcggccaatgggcgcattgcccacgcattgacgctgtcccttcaggttattccggccatatccgccaccgcgtttgccgcgtgtgacctgattgccgccctgaaaaacctgatcaccgacaaccgctggggcctgcccggcgatcagtgcgatctgccgatgaatctcgacggtttgccgtcgctggcgattcgcgccgatcagcccaacaaggcctggaccctgacattcaaccagaccctctacctgggcccgaccttgatcgacgacccgctcggcacaccgaaattcgcccgcacctgggaagtcagcgacatcgacgaccccgaccaatacacctcgctggaggcctgaccgatgttcgacgcgttactgcgcatgcaactgggcccgatcattgagcgtcttgccgagatggaagcggagatcgaagacctgcaccgacgcgccgaaagcttttgccgcatcggcatttgtcaggaagtcgatgcggcgagcaatacctgcaaggtcagtcacggaggattgctcaccccggccatcaagttcttcaacccgagcgccggcgcgcagagcgagtcgcggattcccagcgtgggtgaacagtgtctgctgctcaactacggcagcggagagagtggcgcacaaagcgtggcgttgtttggcttgaacagtgaccgctttccacccgttgcgaccgtccccacgctgacgcgacgggtgcatgtcgatggcagtgaaagcggctacgacgacgccacgcacaccctgcactggcaaaacggtccggcagcgttcagcggttctcgtgaagcgcttgaactgagcatcggcccggcgcgactggcgatgacagcgcaagcgatcaacctgcaactgggcgccaccggcctgaccatcgacgcctcgggcgtgcacttcagcggcccgttggtggatcaccagggtcgcgtcatcagcccctgaatcaagagcctcccatgatcggaatcgatagagacaccggggccacggtcgacgattggctgcaattcgtgcagcgcgcgacacgagccctgaccacgccgctgggcacccggcaaaaaaggcccctttatggttcgttgatccccacgctgctggggcaaaacctcggcgatgacgttctgcttctggcccagagccacgccgcgcaggcgttctacaacccgcagaacggcatcggcgatttccagcccggcgtgatcgtcgccacccgacagggcgccggcctgctgctgcgtttcgccggcacctggaaaaaccgccaacagactttcgaggtcgtgacatgagcatgttgatccctggtcagaaccaactggccgaaccttcactgatcaaggtcgaggccttcgaggatctgctcgccgagttcaagaccttcgtccttgaatacgtcggtacccgttcgccggacagtgcggcaaaactcaagatcagcctggaaaacgaaagcgaactgctgacgatggcgctcgaagcgttttgcgttcgcctgcaaacccacgaacgcaaatacaacgcccgcatcaagcagatgctggcgtggtgggcgaccggcagcaaccttgatgcgcggctggctgacatgggcctggagcgacagttgctcgacccgggcgacccggcggcatttccgccggtgccggcgatttacgaaagcgacgatgacgcccggttgcgctactacctggcgccccatgcgccggcggcaggctcgcggatgcagtaccgccgcgaggtgttcaccctcggcgagcggccgtcggtgaaagtcgaatccaccgatgccggtgtcgtcgacgtcacctacacctttgccccggacggactcgccgcacaggtcaaggatggcaatggccgtcgcaccgcacccggtgaagtgcaggtgacagtgctgtcccgcgacgccgacggcacaccgtccgctgcattgctggatggcgtgcgccaacacttcgcccggcccgatgtctgcccggaaaccgacaaggtcacggtcaagggcgccgagattcagcgctacaagattcgcgtcgtggcgaagatcaattccggcccggattcgggcctgaccaaagttgctgccgagcaacatctgcaagcctacgccgacagttgccatcgcctggaaggccgggtcgccccgagctggatcgactacacgctgcacagcgccggcgccgtgcaactggagattcttgaaccgctgacaccgattgtgtgcagcgcgtttcaagcgccttactgcacggcggtcgaagtcgaggtgcagaccctatgacggaccagacaccgcgtccgaccctgctgccggccaacagctcggcactggaacgggcgctcgatatcggcttcggcaccttgcttgaccgcatcgtgccgccgtttcccgaattgatgaacccgagcgaaacaccggtcgcgttcctgccgtatctcgcagcggatcgcggtgtggccgaatggagcaccgacgcaccggaggcggaaaagcgcctgactgtcgaactggcctggcccaccgcgcgtcaggccggcactcgcaaggcactggaaaacgccgccaaggggttgcaactgaggccggaaattcgcgcctggtacgagcagacaccgccgggcgcgccttacagcttttccgtgcgggccttcaccgaacaaccctacagcgaagaaatcgacgcccgtctcgaccgacgcctggccgatgccaagagcgaacgggacgtgctgtcggtgtcggtcggcctcagcgcattcggcaaccacgtcatcggtgccgcgacgttctgcggtgagctgaccacggtttacccggtgttcctcgaagggctcgagacatccggcgagtccttcaaggccactggtctctacaccgtcgaaacatccactatttatcctcagggggcctgaatggctgactattacaccctgctcaccaacgcagggattgcctacgaaaccgcctgcaaggcagcgggcgtgccgatcaagctgacgcagatttctgtcggcgatggcggtggcgcggtctacaacccggccgcgaccgccactgcgctgaaacgcgaagtctggcgtggaccgcttaacgcgctgtttcaggacgagaaaaatccgagctggctgctcgccgaagtcaccatcccgccagacgtcggcggctggtatgtgcgcgaagccgggctatggaccgacaccggcattctctacgccatcgtcaaatacccggagtcgttcaaaccggtgctggccacgtccggctcgggcaaagagttctacatccgctcgattttcgaaaccagcaatgcttcgctagtgacgctgctgatcgacgacactgtggtcaaggccactcgtgcctgggtcatgagctacctcgccgaagaactcggcaaacttgatggcaaacaatcggtgcgcgtcgccgccaccgccagcgtggtgttgaacggtgcgcagcagatcgacggtgtggcggtgattgccggcgaccgcgtgttgctgccgaatcagactctggccaaggacaacggtctgtggatcgtggccaacggtgactgggttcgggcaaccgatgccaacgtcagcgccaaggtcacaccgggcctgacggtgatggtggaagagggcacgctcaacggcgattcgctgtggcacctgaccaccaacgcgccgatcaccctcggcaccactgcgctgacattcaagatgctcgcggggcgcaccgggattgctgccggcacttacaaaagtctgagcgtcgacgagtatggccgcgcaacagccggctcgaatcccgacacgctggccggcttcggcatcaaggactcctacaccaaggccgaagtcgaagcactgatcgccaaggcctcggcgttgccggtgggttcgattgttgccttccctgtcgatacaccgccgccgggttttctggagctggacaacagcgtcaaaagcagcgcgacttaccctgacttgagcgcctatctgggcggcaagttcaacaagggggatgagggtgtcgggaatttccggttgcctgaggcgcgtggggagtttttgcgcggttgggatcatgggcggggggtggatgcgggccgagagcttggtactgcgcagaccgaagcgttcaaggcacacaaccatcgatattttgatagcgtcgcagcaaccatggatccagcaggtggttggcagagtgggaccgttaacggtacccaggccggtgtttccccaggtgcatttatatcggttaccaatactggtgatgccggtcagatgctgaatgcacataccaccgtcaacaccggaggtactgaaacccgcccccgtaacatcgccgtcatgtggtgcatcaaggcctggaacgccccgatcaatcagggaaatatcgacgtagcggcactggtcaaggaagtctcccgtttgggatctgccgttccggtgggtgctgtcatggcgttcccgacggggatcgtgccgcccggttttcttgagctggatggcagtgtgcaaaacattgcgacttacccggatctggcggcttacctgggaacaacattcaacaagggcgatgaaggagttggtaactttcggttgccggaatctcgtggtgagttcctgcgtggctgggatcatggtcgtggtgtggatagcgggcgaaattttggcacgtatcagactgacgatttcaaggcgcacaatcatccgccggcaaataatcgtccgggcttcatgactaatgagtttccaacggttcaggcatatcacgcagccacttcggggggacctcaatcctactcgggtgaagggcaacagattgctacgacgggtaaccggggaggcacggaaacccgccctcgcaacctcgccgtcatgtggtgcatcaaggcctggaacgcgccgatcaatcagggaagcatcgatgtagctgcactggccaaggaagtctcgcagctgaaatcgtctgttccggtaggtgctgttctgtcgtttccaacgggtgtcgttcctgccggctatctggaactggatggcagtgtgcagagcattgcgacctatccggatctggcggcgtatctcggtacgacgttcaacaagggcgatgaaggtgccgggaatttccgcttgccggaatctcgcggtgaattcctgcgcggctgggatcatgggcgaggtattgatatcggtcgtagtgtcggcagttatcagtcgggtacgaaaactcagggcgatgacggcacggcgccggctgttcaaggtatcggcaactccaatctgattgatgctgatcctgctcctggcttcagtggcgatatttactacacctccaccaatgtcgtcgtgcagaacttttccaactcgttctggaaaacggttcgcccacgcaacctcgcggtcatgtggtgcatcaaggcctggaacgcaccggtcaatcagggaagcattgatgtcgcagcattggctgcagatgccaggtcggctcgactcaacggtgcagaagtcggcgccgcgcgtaatctgagagtgtcgctacccgctgctgcatcggttgcaacgcttacggccgaccaattgattgtcgagcaaccaggcgttggccagtacaagctatcgaacgtcaatctctctataaatctagccaccattggtgcgggcggaatggacttcggcgttgcaccagcaaacggcagtgttggcatttacgttatttacaaccctgagttgaaggttgcaaagctgctgggcgtcaacgcgacatcgacttctgttccggaaatttacactggcaccaacatgcccgtcggttatagcgccagtgcgctggtcagtgtgtggcaaaccgatgccaatcgattgatgaatgccggcattcaacatcagcgttcaatttccatcattcagacgatggtgctggaaaacggattatcgatgtcgtcgacaccgatctcgctggcctctgtcgttccgaagaatgcgaaaagtgtcggtggttacattcattacattggaagcgctgatttcccgggtggtggctctctggggctttcgccggatgtcaccgaagtggggctgaaagcatgcggcatcggtggaatcgtcgggttgggtgttctcagcccgttttcggatctggtcatgacgactccacagaccatctattaccgcctttatgcgtcggtttcccgagcaaacgatgtccacatctcccaatacactttctaaggagtcctctatgttgagagcctactcaaattcagggacggcctttcgttgtgtcgccccggactggccgctatctgacggtgaagtactgtttgaccatgaacccaccgtccaggaactggaggacgcatttgggttcgcgaacggcgagctggttgtaaagcgccaatgggaacagattgcagaagaacgattccgtagagagggttcgggcatcgtggtcgcgggtgtcgctatcgatacgtcccgtgacagtcagtcactgatcgccggtatggcagtttctgcgatgctcgatcctgagtaccactgtagctacaaggctatcgaaggatttatcgatattacctctcagcagatcctgcaaattgcgcaggctgtgcgttctcatgttcaggcttgcttcgatcgggaaaaaacgttgtacgaatctgctcaagcaggcacgtatagcagagaaatgctgaccgaaggatggccagattcctcgcctgaaacaccaccgaaaaaccttcaataaccccctgcaatccagggcgtttacttgctaaccaacacccgccagcccctccccacgaggggctttcccgtttatggagaaacgaaaaatggcaacccgccaaacctacaccgtgctcgttccattccccaccggcggtgggcactggtcgagcgtcggccaggaactcgatctgctcgacgtcgaggccagtgccctgcacagcgccggtcgactggagctgaaaacacctaccaccaaggccgtgaaggccgctgccaagaaggctgactgaatatggctgaggttctgaacttcgagcacaacggcattaccgtcaatgccaccgaatcccccgaggccatgggtggcctgggtgacaacgtcatcggtctggtcggcactgcgccgaaagccgatccgctgattccgcgcaacgcaccgtttcgcatcaacagcttcaccacccacgcgctgctcgatccgaccggcgcggaagagggcactctgtaccatgccgtttaccagatcctcaaagtggtcaaggtgccggtgtacgtggtgatcgtcgaggcgggcgcgaccccggccgacaccgtcaacgcagtgatcggcggcatcgagccagccaccggccgcaaactcggtctggcggcactgggcagcgtcccggaagacctgaccatcatcggcgcgccaggcttcaccggcaccaaagcggtggccagcgagttcgcctcgttcggcaagcgcatcaaggcccgtgtggtactggacggcaaggacgcttcggtcgccgaccaggtgacctacagccaggaactgggcggcgccgacctcggtttcgaccgttgcctggtggtgcacaacatgcccgccgtgtactcgaaagcggcgaagaaaaacgtcttcctcgcgccatccagtctggcgattgccgcgctggccaaggtcaagcaatgggaaagcccgggcaatcaggtgacctacgccgaagacgtgtcccgggtcgttgagtacaacatcctcgacacctccaccgaaggcgatctgctcaaccgctacggcgtcagctattacgcccgcaccgtgctgggcggcttctcgctgctgggcaaccgctcgatcaccggcaagttcatcagctacgtcggtctggaagacgccatcagccgcaagctggtgaaggccggccagaaggccatggccaagaacctgaccaagtcgttcatggatcaggaagtcaaacgcatcaacgactggctgcagaccctggtcgccgacgaaaccattcccggcggcagcgtctacctgcacccggaactcaacagcgtcgagaagtacaagaacggcacctggtacgtggtcatcgactacggccgctacgcgccgaacgaacacatggtttatcaactcaacgcccgcgatgaaatcatcgagcagttcctggaggacgttctctaatgtttaccaaccgtaatcgccaggccatcgcggccaccctgcaaggcctgccgctgtcggcgaccgtggaggaattcactccgccgaagatcgaattcgatgtagaagaaatgcgtggcggccgcttcatcgttgaagaaatggtcaagggcggcaaagcgctcaacgccaagttgaccctgcaaggcatgggcgccgaggtcatgcttgcactgggtgtgaagctgggcgacgacatcctgctgaacgtgcgtgaagccggtcaggaccaggacggtaacacctggttcacctaccacacggtcggcggcaagctgaaatccctggaggaaaccgcggtgaagatgggtgaaaaacccaagaccaacctggagctctcctgccgtacttacaaccgtctggaaaatggcgtgccggtgatcgacatcgacgtgcgcacccagaagttcgtactcaacggcgtcgacatcctcggtgatgcccgtcgtgcggtgctgatgccgtaagcctttcggcgcatcaagcacaccctgtgggcgcttatgcccacagggatcttcaagaacacccaaggaattcctttcatgtcgtggatgccacccaagcatgacctgttgtcgccgatcaccggtgacgacggctcgcagatcgaatcgatccagctcaagcccctgttctacgccgcccagaaagaagcgctggaacgcgccggcgatgacgaagacgatcagttcttcgaactggcgctgctggccaccgggttgtcggtcaaggaactcgaccagctcaaacgtccggactacgtgagcatcgcgcagtacgtacacgagatgtcgacccgtccggcgtcgtactttctcgaccaggtcgaagacgcggaaaagtccgacgatcccgaccaggtgcaactgctgcaaccgctcgccgtcaccggccgcaccgtgacctcgctgagcctggaaatgccggcgctgcgggccaccaaagtgatgaagaaactgaaaacggccaaggaacgcgccgagttcatcaccgcccattgcaccggcctgatgatccccgatctggccctgatgagcgtcccggactggacgcaattgcaggtgcgcatcgacgattttttaaaccagccggcggccttctttcagagcgcgacatcgaagtaatcctcgatatcgtgccgctcatttacccggtaagtgaggcggaaattctggagtgggacgccgaaaaggcgttgcgccgctacgacatagcgatcactcgccttggcgtgaaacaggagtagagcggcatggcacagagcaaatttgcgctcacatacgccaatgagagtggcaacgcagcagccgggttaaagctgcccgatggccttggcaaaccactgcaggacttgaacctgacaatggcgctggcgagcgcggatatccgcttgctgacccaggagcagatcaagcttcgagagctgttggccaatcagcaatcgctgttcaaggtgagtgctgcatccccggctgcaagcgccgaaccaaagtcaaaactcaaggccgagatcgagcagcgtccacctccaaagctcatgcaaccagccatggccaacgagacggcgcttgtcgaactcaatcagttgctcaaactgagcaatgatcagcttcaagcgcactcgcagagcactctggaactcgccagcgagaaacagatatccgccagtggtgcgaccaacgcggatctgttgcaagtgcagcttgccggagccagatccggcattgccgatggtgccaaaggtgaccagcgggcgaacgcactgaagtggttctcccatgatgccgcaatcaacgcatcggcattcaggatggacgtcaaggcggctggcgaaatgctcgccgcatggcgctcctcgctgaagctggatcagtatcaaagccaggatcttgcggatgcaacgacctacctcggcaatagtggtctggatgccaaggccgcggacatcggttcggtggtgcaacgttccggtgagagtgcgattgccgccggattgactcccgaacaggtcgctgcattggcggcggcgcttctcaatagtggtgcggacaaggagggcgccagcgccgcgctgaaaggcatcacctcgatgctggccaaaggcggtgcggtatcgactgagcagcgaacagccttgactcagttagggcttgatcctcaatcgctgtctgagggtatgaagaaggatgcgcctgctgtcatcaactcggttcttgctgcacttaacaagcagcctgtgcaagagcgggcggcactgacgaagacgctgttcggcgaaaacgacaccagagttctcgaactgctgaagaagccggacgatgtaaaaaacgccttctcgctggtagccgacaagcacaagtacgcaacaacggagcttggcgcgggtgaaggcgctgcggcgaagtccgcagaggcgttcggcaatacttcgcagggtcgctggaatgcgctggacgcaagtctgacccggttgaccacatcattcggcacggcgcttgcgcccctggctgacggtgccgccgtcgtgctcaccgccctggtcaacggtgttagcgcagcggcggaaacgttcccggcactcacggcaggactggctctgctcgccgtggcagccatgccgttcgtggggggggcgttgaagtccggcgtggcctcggtgctcgacgtggtttccacgaaactattgcgcctggcatcgacgcgactgccgccggatattgccgatgtgataggcggtgatgacaacgatgacgacggtcgaaaacgcagaaagaaggggcgcggatcgcgccgacgccccccttctgctgcacggtcgtccggcaccgcttccataacccgcaagagcagtcgcttgagtggtgtgacggccagaatcgcacccatgttcgacgatgcgctcacccgattcagaatggttggcgatgttgtcaaaagcgccatgccgagccggctgagcggggctggcgcgaaagtcatgtcgttggcagagggcttgggagccaggctcatgccctcggttgtcaaggcattgcctgtcatcaaggttggcgcgcctctggccattgctcatgctgcctatacagggttgaaaggttggcgcgaaggtgacgacaaagcggtaaagggcgcggccggcgaactggccggaacggcgattggcgctacgatcggtacgttcattgcgcccggcatcggaacctttattggtggcacgctgggtggaatagccgggtccattctgggtcaaaaactggcgacgccacctgaagacaaattggcaccgccggcacaggtcgccaaagacgtatccattgcgcaaacgcaaatgcaagcgtcaaacccgcaatacacttacgcaccttcagttcatgtcagcggcagcgaactggttagttccgagaaagtcggcacgatgctttcgcaggtgctggagtcgcacttcaattctcaatttgtcccgggtgtggctaccaatgccctcgccacccgccgtgacgcagccctgaccgatggagtcgcctgatgaaacaacaaatggcactgggcagtttcatcttcggactgtcccgggattttgcgtacagcacgctgtcgcgaaaatccgagggtggctggaccgagctgcagatcctcaacagcaaacccagatcccatcagacaggacagaagcctgaaaccctgaccatctccggaacctcgatgtacgccgtggcgatggagcggctcgatgagctgcgtgcgctgcaagcgttgagagtaccgctgccgttgattgacggcatcggtcgtaactggggtttgtggcggattaacagcatcgacgaaaaccagagcgaggtcatcgatgacggaaccgcgatggtgatcaagtgggtcatcggattgtcggagttcaacaatgcgtaaggtacgaagcgtggccggcgattcggtgaatctgttgctgtaccgcgaaaccggtcgcagcgatgacagcgccgaagaagccctgtggacactcaatccgaccctggccgagcacggtccgattctgtcggccggtgtctgggtgacactgccggaactcgatagcaaaccggccgcgatcaaaccggttctggcctgggattaaggaggcagcatggcacagggatttacgccggcgatcgaaatctacggcgccaacaaggacctgctgaaccagcgcctgatcagttgggaacacatcgatgctgccgggatggagtccgatcaactgacgctggtgctcgacctggaaggccttgaaggcttgccaaccctgggcggaatcatcggcctgcgggtggggtatctggagaccgggctggtcgaaaaaggccagttccgggtgactcgattgacaccgacgctgttcccgctgcgtctgacgctggtcgcgaccgccgcacctttcagcggcaaggacgaaaccggattcaaggaacgacgcacggccagtcatggccccacgacgcttggcgggctgtttcgcaaactggtcgagccgcacggtttctcgccgcgcgtcgatcccgaactggcgctgatcaggattgctcatgtcgaccagtcaaatgaaaccgacatgggcttcatcacgcgactggcgaagaagtacgacgcggtggccaaaccgttcaacgacctctacgtactggcgaaaccggcgcagctcaaaaatctgtcgggtcaggtgataccgaatgtgaggctgtcggtgacccacaacaatcggccgggcgaacacgccttcatcagcgctacgctggaagagaccgcccgcacccagaatgaaggttgcaaagtctgctgttgggacgccaatgccggcaaacaggtggaggtgaaaaccggctcggcgccctacaaggtcgttcgtcagaaacaggccagtgtggaagaagccaaagccatcggcgaagccgaagtgcgcaagatgctgcgcgagaaatacaagctgaaggtcacctgcccgggcgatccgctgctggttgccgagggcctgctggtgctcgatgacacctggccggacttcatgcgcggtcgctggtcgatcgagaaggtgacagccagcggcaagcccgaagaaagctatcgctgcctgatcgaagcaaacggccgggatcccgaggcaaaagccaaggactgatcccccgatctcaccaccacactcctcacggtggtcactcccaaaacctggaacgctccccatgaagatctccccgatcctcacgcagctgcgtgcgcaatgcccaagccttgccggccatatcgcgacaggtgtcgacctggcgctgctgcaaggcaacccgaatctgccgaccccgtcggctcatgttttaccgctggccgatctggccagcgccagcaccgcacagaattccgccagtcagccgatccgcgaccgcttcgaaatcatcctggcacttgatgccacggacgccacaaaagcgctggatctgttgcacgacctgcgcgccgaagtgtggcgtgcgctggtggggttcaagcccggttccgactacagcgccatcgtttatgacggcggcgaaacggtctcgatcaacagcagccgcgcgttctaccggctgcgcttttttgccgagttccagctgggccgcaatctgccaagtcagcctgcggagagttggcacgaacgtgaactggacggtttgtcgtcctttaccggggtcaccgtgcgggtcgatgcgatcgacccggccgaccccaacctgaaacacccgggccctgacgggcgcgtggaaatgactttctctggagacgtaaccccatgagcaaccgcatcaccgtagtgccggccactggccgtgccgtgccggacccggaagcaggcgacctgctgccactggaaggccgtgaagtgctggacagcgcctggtggcgccggcgtctggccgacggcgatatcaccctcaaaaccgcaacagctaaacaaaagggagccaaataatggcgatcggattcagcaacattcctgcggacattcgtgtaccgctgttctatgccgaaatggacaactcggccgccaatagcgcgtcctcgtccatgcgccgcctgatcgtggcacaggtcaacgacaacatcgccccgagcgaagtcggcaaactggtgctggtctccagcgtggcactggccaaaagcattggcggccagggctcgatgctcgcctcgatgtacgagaccttccgcaaggccgacccgatcggtgagatctggtgcctgccgctgcacaacgctaccggcgccatcgccaaaggcgtgctgaccctgaccggcaccgcgactcaggctggcgtgctcaacctgtatgtcggcggtgtccgtgtgcaggccaccgtggtcaacggtgccacggctgcccaggcggccaccgccctggcacagaaaatcaacgccaccgccgatctgccggtgagcgctgtggccgctgaaggcgtggtcaccctgaatgccaaatggaccggcgagagcggcaacgacatcagcctgcaattcaatcgcctgggcaagagcaacggcgaagaaaccccggccggcctgaccactgccgtcaccgccatgaccggcggcgtcggtgtaccggatcaagtggcggccgttgccgcactgggtgatgaaccgttcgaattcatcgcgctgccatggtccgatctggcgaccctcaacacctggcaagcggtgatggacgacagcaccggtcgctggtcctgggccaagcaactgttcggtcacgtctacagcgccaagcgcggcaccgtcggcactctggtggcggccggtcaggcgcgcaacgaccagcacatgaccattcaggcgctggagcctggcgttccgcaaccggtgtgggtacaagccgctgcactggctgcacgtacttcggtgttcatctccgccgacgccagccgtccgacccagagcggcagcctgccaggcgtcgatccggcgccggccagcgagcgcttcaccctgaccgagcgtcagtcgctgctcaactacggcatcgccaccgcgtactacgaaggcggctacgtgcgcatccagcgctcgatcaccacctatcagaagaacgcttacggccaggccgacaactcgtacctggacagcgaaaccatgcaccagtcggcgttcatcgtgcgtcgtctgcaaagcgtgatcaccagcaaatacggtcgccacaaactggcctccgacggcacccgtttcggcgccggtcagccgatcgttaccccggcgaccattcgcggtgagctgatcgcccagtacgccaagcttgaactggaaggccacgtggaaaacgccgagctgttcgccgagcacctgatcgtcgagcgcgacgtgcaggacccgagccgcgtgaacgtgctgttcccgcctgattacatcaacggtctgcgcgtgttcgcactgctcaaccagttccgtctgcagtacgacgacgtcgcctgatcggctcgtttgacactgtgatttcagcccacctcgcgtgggctttttatttgaagggagtaacaccatgggtcaactgattgcaggcacctgctacgtcaaggtcgacggtgcacaactgaccatcaatggcggctgcgaagccccgctgatggccgtcaaacgcgaaaccgtcgtgccgggtttctacaaggaaaccgacatcgcgccgtcgttcaaggtgaccgcgctgcacaccgccgacttcccgctgaagaagctgatcgaaggcaccgacatcaccgtcacctgcgaattcagcaacggcaaagtctacgtgctggccggtgcctacctggtcgaagagccagtctccaaaggcgatgacgccaccatcgaactgaaattcgaaggcatcaaggggacttggcaatgagcggcgccgtgaagcttcaagttgcgatcgaagctcacggcgagcccctgaccgaactcgtcctgcgccgtccgacggtgcaggaggtgcgagcgatcaaggcgctgccgtacaagatcgacaagagcgaagaggtcagcctcgacatggacgtggcggccaaatacatcgccgtgtgcgccggcattccgccgtcgtcggtcaaccagctggatctggctgacctcaacgcgctgagctgggccgttgcgagttttttcatgagtgcggcgtcggagccatcaccgacctgatttcggtcgcctatgacctggcctggttctggaaggttgaccccgaacagatgatggccaggccactggatgtgcttcgcgaatcgctggagcacgcgcaacggatcaatgcgatgcagcaggtgcagtgatggcagaagaaaccaaagcgaaagcgtcggtgctgcttaccggcatcgacgaactgtcacccaaactcggcgccctgcgagtgaaggtcgatgacttcaagaagaacctcgaacagaccggcctcggcaaactggacatcagcggtctgttcaagggtgggagcgtgattacgccgttcgtggacggcatcaaatccgccgcagcgtttcagggcaagttgaccgaagtcagcgagacggcgaaaaccgtcgatctgccggaaacaccgaaagccgccgcgcagaacatgaacgtgttcagcgcgtccatggaaagggtctccgctgcggtagacgccgcattggtgccggcggtgggcgccttggtggtcgggctggagccgatgctgacccaggtcggcagcctgctggccgacaacccgaaactggtcgaaggcctggcagcgggggcgattgcgttttccgccatgcaaaccgccgtcaccggtatgacccaggtgatggacgtcatgagcatggtgctcaagaccaacccgatcatgctgatcgccatgggcattgccgtggcggccggactgatcgtggccaactggacaccgatatccgcgttcttcaccggaatgtgggagggcgtgaaaaatgccggggccagtgcaatggcgacgttgcgctcggtactcgactggcgaccgctggaaacgctggcagcgctgtgggaaccggtcacgggtttcttctcgggtatctgggacaaggtcaaagcggtcacggcgccggtgatcgacttcttcaagtcggttttctcgtggtcgcccgcgggcctgatcctggaaaactgggggccgttgaccggtctgttttcggcgatctgggaattgctcaaggccttgagtgtgccggtgatgtcgttcctcaaggggctgttcgactggacgccgctgggcatgatcatcaacaactggggcgcaatcaccggtttcttcgcctcgatctgggtcgcgctgcaaccggcggcgcaagccatcaaggacttcttcggcagccttttcgattattccccgctgggcatgatcatcaacaactggagtgcgatcaccggcttcttcgcttcgatctgggcggcgctgcaaccggcggcgcaagccatcaaggacttcttcggcaccctgttcgactattccccattggggatgctcgtcaacaactggggcagcgtcgtgacctttttcgaaccggtctgggccgcgctgcaaacgtcggcacaaacgatcaaaagcttcttccagagcctgttcgaatggtcgccgctggagcagatcgcgcagtactggcagccgatcagcgaagtgttttcggcgctgtggggcgtggtgcaggcattggccgcgccggtgctggagttcctgcacaacatgttcgaatggacaccgttggggcagatcatcaagaactggggaccgatcaccgagtggttcggcgagctgtggcaaaagctgcaaaccgtcatcgcaccgatcaaggagctgttcgacggcggcttcgccgggctaatcgccagggtcaccggcaaggtcgaaaccttgacccaggcgcaacgtcagaccaatgccgaaggcaagggtgaactggcgccggccttctttggtgccagcccgaaacccgagggtggcagcgcgctgcagggcggttctttgccgcaatcctctggcgcactgatccagcaaagcgccgccaataaccgcacgcaactcgaaggcggcctgacggtccgcttcgaaaacgcgccggcgggcctgcgcaccgatcaaccgcaaaccaatcaaccggggctggcgctcagttcgcgcatcggctatcgctcgctatcggcaggaggttccaatgaactggcgtgaccgtttgttgccggcatcctttcgcggtgtcggcttctggatcgaccaggcgaaaaccccggtcggtcgcaagggacagttgcatgagtatccgcaacgggacctgccgtttttcgaggatctcggccagcaggccaagacccacgacctgacggcgttcatcatcggtgccgattgcctggagcagcgcgacaagctgctccaggccctggagcagggcagcggcgagctggtgcatccgtggctgggccgcttgcaggtcaaggtcggtgagtgcgacatgacccacacccgccaggacggcgggatggtgaccttcaccctgaagttctacccggaccggccgctgccgtttccgacggcgacggtcagcacgcaaaaagtcctgctgatcaaggctgacggtttgctcgggtcggcggtggcgcgctttgaacaggcgatgaccctgatcaaggccgcgcggatcggcatcgccaatctgcgcaacagcctcaccggcgtgtacgacgtgatcaaggagcagctcaagccgctgatcgcgcaatacaagcagatcaccgaactggtcagggccgtcaaggaactgcccaaggaagtggcggcggagttcaaaggattgctcggcgatatcaaggagctgaaggcattcgcgaaggagggttaccgtggcgtgattgccgacgtgtcccaacagatcgaagccatccgcaaggccgacgccccgaagatcaccaccggcaaggacaccacggctgcggcgcaggccctggccaatctggtgcaggacacccttatcgtcaaagcggcgcaatgggtagcctcgatgccggtggcctcgacgccggtgaaactgtcgtcgacgccgtcgctggatcagcagtcgaaacagccggtcagccgtcaggaagtgccggtcaccgacgatctgcaagcgttgcaaaaagagctgatcgaagcgctgcaaaaggcccaggacaaggccgatcccgcgcactaccaggccatcgccgatgtgaaggaagcgctgatcgcgcacctcaaggctgtggcttcgtccggtgtgcggctggtgagcaaaaccttccaggaaacctttccggcagtggtcgtggcttacaagcagtttggcgatgccacccgtgtgaccgaggtcattcagcgcaatggtctgtctcatccgagcttctcacccaacgaagtcaaggtttccagggagtgagtcatgaacgagactgacaaccgcgtgacgctgaccgtcggcgacatggaatacggcggctggaaaaacgtgcagatcaccgcggacctggagcgccagttccgcaccttcaaactcgatatcacctggcaatggccggggcagaccgtggatcagcggatcaaggccggcgacccgtgcgaagtgcggatcggcaaggatctggtgctcaccggttatgtgttcaaggccccgatcagctatgacgggcggcagatcagcctgagcatcgaaggcagttccaagacccaggatctggtggattgcgcagcgcgaaacaaccccggccaatggcaggatcagtcgctgctgagcatcgtccaggccctggccatggagtacgcgttgatggtggtcaacgaaattcccgagaccgcacgcctgagcaaacacacgatcgtaccgggtgaaacggcgtttcagtcgatcgaccgtctgctctcgctgtaccgggtgttttccaccgatgacgccgaaggccggctggtgctcgccaaacccggcagcgctggccgcgccagtgacgcgctggagttgggcaagaacattctttcggccaatgcgccgatggatttcagccaggtgttttccgagtaccgggtgatcggtcaacagaagggcaacgacaagaagagcggggcggcggtcagcgaagttgaatcgacggcgaccgacctgagcttcaagcgtcggcgcaccacgatcatcaacgaaggctcgcaactgacgttcgaactggctcagcaacgggcgcaatgggagagcgcgacgcgcatgggccgagcgctgaccactacctatcaggtacagggttggcgccagtccaatggcgatctgtggcgtcacaacacgttggtgcgggtcaaggatccggtgctcggattcgatgaagacatgctgatttccaaggtgacgtactcgctgtcggcgcagggctcggtgaccaccctgcaagtggcgccgccgcataccttcgacgcgaacccgactcccccgaaaaagacctgagcccgaccccgccctccaaggaaaaccctatgagcctactgacacgcctgctggcgcgcggcactgtcgtgctcgccagttcggcctccaagctgcaatcgctgcaaatgcgcctcaccgccggtgaagtgaacgacgacatggagcacttcgagccctacggctttaccagccatccgctggccggtgccgaaggcgtcgtcacgtttctcggcggcgaccgttcccatgccatcgcgctggtggtcgctgaccgccgttatcgcctgcaatcgctggcggccggcgaagtggcgatctacaccgacgaaggcgacaagatccacttcaggcgtgggcggatcatcgatatcgaaaccgccacgctgaatatccgcgccagtacggcggtgaactttgacacgccggtgatcaaccagaccggcaagatcgtttccaaaggtgatcagctggccggcggcatcagccagatcaaacacgtgcatggcggcgtgcagggcggcagcggccagaccggtgtgccggcgggaggtcagtgatgcttttcagtcaaaacctccacgccgcgctgacccgctcggtgctgatcagcctgttcacctggcgccgcgccgccgacgacgatgccctcgatgacgaggagcgttacggctggtggggcgacacctttcccaccgtggccgacgaccgcatcggttcgcggttgtggctgctgcgccgggtcaagctgacccgacagacccagatggacgccgagttctatgcccgcgaagccttgcagtggctgatcgacgacggccattgcagcgccatcgacatcatcagcgaacgcctcgacgcccagcgcctgaacctgcgtacggtcctgaccctggccgacggcgaacgcctggacatcaaccccgataacagttggcaggtgatctatgccgtttgaaaccccttcgctgccggtgctgatcaagcgcacccaaagcgacctggccggcgattcgctgcgccagtccgatgcgcaagtcctggcccgcaccgtcggtggtgccgcttacggtctgtatggctaccttgactggattgccgagcagatcctgcccgacaccgccgacgaatcgaccctggaacgcatcgccgcactgcgcctgaaccagccgcgcaaaccggcgcaaagcgccaccggcagcgtcagttttactgcaaccgcgggcgcggtgctggacgttgatacgctgctgcaatcgagcgatggccgtacctacaaagtcaccactgcgcgcaccaccgtcaatggcagcaacaccaccaccatcgcggcgctggatgccggcagcctcggcaatgctgacgccggactggcgttgactccggtgcagccgatcaccggcgtggtcggcaacagttttgtcgtgctggcgccgggcctcagtggcggcgtggcgcgggagagtctggagtcgctgcgttcgcgggtgatccgttcctatcgcgtcatcccccatggcggttcggccagcgactatgaaacctgggcgctggaagtgccgggcgtaactcgtgcctggtgccgaggcggcctgctcggcccgggcacggtgacggtgttcatcatgcgtgatgaagatccgcaaccggtgcccaacgacgagcaactggcggaagtccaggactacatcgaaccgctgcgaccggtgacggcggaagtgcatgtgcagcgaccgattcaagtgccggtggtgtaccgcttcaagagcgtcaacccggacaccaccgccgtgcgcgccgccgtcgaagcgcagttgcgcgacctgcacaaccgtgaagccgatctcggcgtgccgttgctgatcagccatatccgcgaagccatcagcagcgccggcggtgagtacgatcacaccttgaccgcgccggccgctgacgtgcctgccggtcaaagcgaactgctcaccttcggaggttgcgtatggggggcataagaaccgctgcgcaatatcaggcgcagcttcgcgcactgctgcccagcggcccggcgtgggacccggagcgggtgcccgaactcgatgaagtgctacaaggcgttgccgtcgaactggcgcgcctcgacgcccgcgccgccgatctgctcaacgaaatggacccggccggcgtcagcgaactggtgccggactgggaacaggtgatgaacctgcccgacccgtgcctcggcgccacaccgctgttcgacgaccgtcgcctcgccgtgcgccgccgcttgctggcggtcggtagccaggccgtcggctactacctggaaatcgccagaagccagggctaccccaacgccaccatcaccgaactcgaagccccgcgcatgggccgctcgcgcttcggcgcggcgcactggggcacctgggaagcgcagttcatgtggacgctcaacaccggcggccgcttgctgctcggccggcgtttcggcgcgagttactggggcgaacgcttcggcgtgaatccgggctcggcgcttgaatgcctgattcaccgggcggcgccggcgcataccaaggtgcacatcaactatgactagggaataacgcaatggattatccgaagagtgtgcccagtgccggtctggtgaatgggaaatttgtcgatgaaaacccgatgaccgggacgcccggatcgttgattccggcggactggggcaacggtgtcacgcaggaaattctcagcgtgatcaaggccggggatctgaccccggatgagaagaaatacgatcagttgttgcaggcgattcagacggtgacggccaagggctggaatcaggatctggcgctgccgctgtcggccttgccgctgccaaccgttgccactacggatgcgcggatgccgatcacgccggccgccgcctcgaccagtggcgggcgggtgtcggtgccggcaggtatctacgtcagcattggccaggaagtagtggcggggcagttgggacgttcgcggacgttcaccactcagacctggagcagcgccgatctgttgccgagttctggttactttctgcgggcgcaggtggtgagtggtgcactgacgttctacatgcagcgcgggacgatttacgacgtgacgcccgattccctgaagggcacggtcaacggtgctgccggcggtggtttccagagttcggtgctggacatgtgcctggcctgggtggttaccggtgcaccgggctcggtaccggtagtgcgtgcgatctataaccgggcacgcctgacctgggcgcagacgctcaacggcacgggggcagtgtttctgccactggatcctcatgcccgcgctgcgcgactggtggtggggaacccgacgccatcgtcgactgctgttacaacggttgcgtttccttcgactggatgggcgggtggcaactacagctacctttcgcccgtatccacaggcgtttccaataatgccggaggctggaatcctgccaccgcacaaccgtgcgtcatcttcaccaacaacatcgtcaatgacgtcacggtttcgacactgaccgccagtttcgatcacgccaatgtgcgctcgctctggcagtcctatcaggccgaacacaacctggcacaggccagcgccgacagcgatgagctgttgctgagcatgggcatcaagagccatccggtgaccgattacaacgccggtattccgatcaactttagcgaagctgtgaacgttcagctgtcgtgggagctcattcgatgatcgtcattcaggaactgcatcagatcgatggagagttgcgtcctgcgcagccgtccgccgcccatgactgggacggtgaacaatgggtcgtcaaccctgagaaagtcgcgctgctggaacaacaggaaactgaaagcctgtgtgcccgggtcgatgttgccgccgacagtgcacgcagcgtattggccggggatccgctcaaggcgttggagtatgcccaggcagccattgatgctcaggcctttcaggacgccggttatccgaagaaggaagtgccgctgtccgtggccgcgtgggtcgccaaaggccggtcggcgaaacaggcagccgagcagatcctcgacaaggctgctcaggtcagcgacagcctgttgaccctgcgcaccttgcgcctgaaggccaagacccagatccgtgggtacgccggcaaaagccagatggatcaggcgcgtgccgccacggacgaggtgttgctggccattcgtgatctgacggccatccagagccagtaaccgctatccgcctcacccaagcccacgtcagcgtgggctttttattttcaggaacagaagcgttggaaccgctgcgaaacccttcgcgccgccgcgtttcatttgtcatgacagaggaacgaacatcccatggattatccaaaaagcgtccccagcgtcggcctggtcgacggtcgcttcgtcgatgaaaacccggtggcgggaacgcccgggtcgttgattccggcggtgtggggtaacagcgttacacaagagattgtcaacgtgatttccggcgccgggatgaccgccgtcgaggccgataacggccagttgttccaggccattcagtcgattgtcggcaaggcaagtcctatgcgttcggtgatcacacggctggcagcgtccaaagcgctgaccgaacaagagcttggccttgtgctgatcgacagcagcccggcagccactacggtgaccttgccggcagccagtctcggtctgggcgtgcgtgacgttatcgttcgccgtgtcgacaacagtggcaatcgactggttgttcaggcttccggtacggaccgcattcgccttcatacacacctttcgtccaatggttacccctttctggtgctgatgggcaatggcgactggtggcatctgcgcagtgacgcagcgggtagctggtggcctgtcgggcgcttcgacaacacaccattgggccgaccggttttcgagaccaccactgtgctggggccgggcggttacggggcgcttaacggagcgttcctcgatcgggcgcaatggccctggctctgggattttgctcaggcgtccggcgtgctgaccaacgaagcggggcggtggggcagggaaggggcgtggaccagcggcgatggtgcgacgaactttcgtatcccggaagcgcgcggcgaatttctgcgcgtactcgatgaagcgagaggcgtagatgtcggtcgtgtcgcgggcagccttcaaaaccatgcgctgcagactcataaccattatctgcccaccagcacaggctcgttcgggcgtcccgctccctccattccggacaatctctggagtgtttcgtctgacgtcaacttttaccccaccaatggaacggtcgctacgacgtatccgaacccggcattcgactccgatacctacatcgggtcgatcggcaatttctcatctgaaacccgcccgcgaaacatcgcgtatcccggccgtatcaaactgatctgaggcacacatgttcaattatttgatagacgacagcggtgcgctgaccgggcctgtcgagtttccgctggtgccaggtatcggcgtacagctgcctggcaacgccgtgacgttgagtatcgaactctctgcggcaccgaatggatatgcctgggcctacgacaacggttctctgcagcaaaaactcgactttcgcggtgatgtttatcacaccgatacgggcattcgggaaacctggaccacgttgggtgacctgccggagggcttgaccacgcaaccatggccgggcggattccattcgtgggtcgataacgcctggcagctcgatgaagccgctcgactggcggatctcaaacggatcgctctgacccggcgcgacacgctgctgcgcgacgcggtcctgcgcatcgcccccctgcaatatgccgaagacatcggcgatgccagtcacgaagagcaactgcaactgctcgaatggaagctctactgcgtggaactgaatcgtatcgaaatgcagaccggtttcccggaacaaatcacctggccggcagcacccggcgcaaccgtaatcagctgacagaagcacagggaacagtgcaatggactatccaaaaagcatccccggcgtcggcctggtcgacggtggttttatcgatgaaaaccccattgccggcacgccaggatcgttgatccccgccgcctggggcaacagtgtcacgcaagaaattctcaacgccatcaaggcagccggactcaccccggacgagagcaaaaccaaccagctggccacagccatcggtgcgctggtcgacttcaccaaactgaagaacaccccgaccacgctggcgggctatggcatcaccgatgccgtggggcggttgctggcggttcggcagatcgagacggtcgggatcacggtttacaagccgaatccgagggcgaagcggattcgtgtgcgtctggtcggggcgggtggttcggggggcggatgtgcgcctgtaccccccacctatcaaagcttcggaggcggtggtggagcaggagcctatggcgaaagcctgtttgatgtgacggcggaaatgcaggctggtgttcctgtttcactgggtgccggcggtgccgcacgcaccgcgatgggtgtttcgggaggcggtgcgtccttcggcagttacatgagcgttgcgggtggcgcaggcgggcaaaccctgtcgatcgtgctgacgggaacttcgtccggttgcgtccagggtggtacgggtgggcaatcggtttctggcgggaatctcactgctgcgcgtggtcagccgggtggttatgccatgagcaacgccaactggggactgctgggaggcaccggtggtgcgagccagttcgacggaggtgctccattcacgggcgcgaacattaatgcgaattccggttctcgtggttcgggtggcggcggagcttgctccaatagcgcatccgtcgcgtatccgggtggagtgggcggcaacgccttctgtgaaatctgggagtacgagtaatggcccgttatgcacgtattgaaaacggtgtcgcggtcgaagtgatcgacaccggtgactacgcgatcgagcaactgtttgcgccggcgttcgtcgcggcgatggtgcaggtgcccgaaggtgctgatgttgaaatcggcgcgccgatgcctgagttgacgcccgctgtcgagcctctgcgcgaaccgccagttcctgaaatcgctcaggccgcaacggtcgagggcaacacgtcttcgacggctgagcgcgcctggcgccagtcggcgctggcggccacggaatggttggtcacacgccatcgcgacgagcaggaactgggacgcggcaccacgctcaaggcccagcattatctggaattgctcgagtaccgccaggcgctgcgcgactggcctgactcaatccattttccggcagtagttttgcgcccggcagcaccggagtggatggccgccgttcatggctgaggtcttgttttgatgttcttgaatagggagaagagtgatggattacccaaaaaacattcccagcgcagggttggtgaatggcaggtttgttgatgaaaaccctcttaccggaaccccgggttcgttgattccggcgagctggggaaatggcgttacgcaagagattcttgaagtcatcaaaggcgcagggtcggctgccgatgaaagtgataacactcagctcaaggcggcaatcgatacgctgatctcgaagaaacaaagcgacagtctggccagccaggaagaagctgaggcgggcgtcagcaacacgcggttgatgacgccgttacgagtgtttcaatccatcgcaaaaaaaatgcaacaggcgaccgagtcgctgatggggattgcaaaagttgcttctcaggcagaggtcaacgccggtgccagtgatacgtctatcgtgacccctaaaaaactcaggtttgggttcatggtgaggctgggggcatccggttatgtcgttttcccctcgtggatggggggggtgattatccagtggatcaccggaggcgcgagccaggcgggcaacaatggctacggggacctgaatctatggccgttggtctttcccaacgcactgtttcttgccgtcgcgacccatgaaggcacggcacccggaacgcagctgacctggaacatcaacgcgaccgtgagtcggcaggcaggcatcaatgttcgttgtcctgaatggccgtcaggctccattgctgctcgtgtcatcggaataggaaactgactatgtattacttttctccggctacttccggcttttatcactccgatctgcacggcgccaatatccccgctgatgcctttgaattgagcgaaggtgagtattgcgcgctggtctcgaacgctccaaaaggaaccgttcttagcctgactgccaacggacgcccggaacgggtgctactggctgaacaaactctcgatgctacagagcgggtctggcgagacaaggtattggatcgaactcaatggctggttcttcgcgatgcggaagaactggaagtcggcgagggaacaaccctgcgcggcgaagagttcaagcaactgctcgcctatcggcaggcgttgcgcgactggccaaatgatccggagtttccggatgcgcgttcgcgtccggtagagccggattggctggaaggcctgctgcgagcgaacaactgagcggattgcccgatggggcaaaaccggactaccaaggaaaatcattatggactaccccaaaagtgttccggggtcaggtttggtcgacggcagatttgtcgacgaagacgcgatcgccggcacccctggttcgttgatacctgcgagctggggcaacagcgttactcaagaaattctcggcgcgattaccgccgccggccttaagcctgacgagcagcagaccgatcaattggcgcaggcgatccgtcaattggcaaagcccgatccactgcaacaatttccggtgcaggtgtatcgccggaacgtcctgatcaatggcgggtttgatatctggcaacgcggtccaaccaaccccgggccaaatattggcggctatgtggctgatcgttttcgttgcgactggaatggcagtgcaggagtcgccatatctcagcagggttttgcacccggtcaaacggaagtcgccgacgagccgcagtttttcctgcggtggcaacaaacccaggcgggaaccggagccaccgtacacagaatctcccaagctattgagtcggtacggaccctggcaggcaaaaccgccaccgtaacattctgggcgcggtccgatgcggcacgacagctaagagtgtcggtcactcagaacttcggatccgcaggttcagactctgtggaaaaaacggtcgatgtctttcaattgggcacatcgtggaagaagtacagtgcgtcatttcgtctgcccggtattgccgggaaaatgctgggagccaacaacttcgtgaggcttgcgttcgacttgccattgaatgttttgcagaccgtggatctggcacaaatacaaatggaggaaggaccggtatccacacctttcgaatatcgcccagtggctgaagagttgatgctttgccagcgttacttcgagaagtcctttgccacttggttgccggtacgggcgaacaatggttctaacacctgcatttcaacgttcacgcaagtggcgcctgccaataacggtcagttcgcgatgacgacaggcatgttggtgcaaaagagggtgttacctaccgtcgtcatgtattgccctggcaataccagcaatcaggtatggaatcaggccgtggggccatgtaccggcagtattgtgcagggattgacggagcgtgccatttcgttttccaccgttaccccggtcggcagcttgcccggtcagaccttgcagatcgaatggactgccgacgccgaactttaggagaaaccatgagttatcaattgaccgccaacggcgttcttcgtctgagcgacctggcatatgttccacaggatcctgccaatagggattggctggaatatcaagcgtggctgttgtccggtggccaggtgttgccctcgaatgaagcaattgaggaatctgcaccgaacagcaccctgacaactctggcaaaaaaatggctggggggcgttggtcgccagccgtgattcaatcggcgcaatccagggaggatcaagcatt

SEQ ID NO: 4 - DNA, 1064 bp, Pseudomonas fluorescens Ps36
  source 1..1064: mol_type = genomic DNA
atgcaaatcactgaaaacaacctcagcaacatcatgcccaacgcccgctcccaagcgggcgtttttgtttcaccgctcaacgacgccatggcgcgtcatcgcatcgatacgcccaagcgcgtcgctgcgtttctcgcccaggtcggccatgagtccgggcaactgcgctacgtgcgcgaactgggcaacaaccaatacctgagcaaatacgacaccggcacgctggccctgcgcctgggcaatacgccggaagccgatggcgacgggcaaaagtatcgcggtcgcgggctgatccagatcaccggccgcaccaactatcgccagtgcagcctcggactgttcggcgatgagcgtctgttatcgttgcccgaattgctcgagcaaccacagtgggcggcggagtccgccgcgtggttctgggagcagaacggtttgaacgaactggcggaccgcgatcagttcaacaccatcacccgtcgaatcaacggcgggttgaacggtttgcaggatcgcctggatctctgggctcgggcgagggcggtgctatgcccatctcctggcgtataaccggtgttgtattgctggtcctgggggctgccgcgctggcctggcaattccaggactggcgctacggccgccaattggccgagcaggcccgacagcatgccgaaaccctcaaccaactgactcaggctgctgcctcggcgcagcaggccgagcaggacaagcgtctggccctggagcaacggctcgcggccagtgaacaaacccactatcgagcactcagcgatgcccaacgtgatcaggatcgcctgcgcgatcgccttgccactgctgatctgcgcctgtcagtcctcatcgacgcaggcgacgctgcccaaggctgcggcgtgccagccgcctccggcaccggcggcgtggatcatgcaaccgtacgcgcccgacttgacccggcgcatgctcaacgaattgtcgccatcaccggcgaaggcgatcgcggactgattgccctgcaggcctgtcaggcctatatcagagcgctggcgcctgcacattttgaatga

SEQ ID NO: 5 - DNA, 36077 bp, Pseudomonas fluorescens Ps36
  source 1..36077: mol_type = genomic DNA
atgcaaaaacgcaacgtatcctccgtcttaagagcgctgctcgatcagtacgggatctcccccacggagctccaccgtcgcaccggcgtgcctcaatccactctctcgcggattctcagcgggaagatcgtcgatccttcggataaacacatctcgaagattgccgagtacttcgccgtgagtaccgatcagttgcgcgggcgcgcggatgttgcgccggtcgccggcggcgggcgcgaggagttgcattccgaactcaaggacataagcctgtgggacgatgacacgcccgtcgatgacgacgaggtgtcggtgcccttccttcgcgaggttgaattggctgctggatcaggaagattcgtcatcgaagagagcgaacgctctagcttgcgcttcggcaagcgcagcctgcgccataacggcgtgcagttcgaccaggccaaatgcgtgaccgtacggggcaacagcatgttgccggtgctgcgtgacggcgccaccgtcggtgtgaacgcgggcaagtgcgggatcggcgacatcatcgatggcgacctttacgcgatcaaccacaacggtcagttgcgggtgaaacagctctatcgcctgcccaccggtatccgcctgcgcagcttcaatcgcgacgagcatccggacgaggactacagcttccaggacatgcaggaagagcagatcgtcatcctcggtcacgtcttctggtggggcatgtacgcccggtaacgatccctctctcagataaaacccgcccacggcgggttttttttcgcctgtagaaaaccggacaacccttgattggcggggcttccatgcatccgcgcatttctcatgcataaataaatgcatttacgcattgactggatatgcatacatgcatattcttgccaccaagccgctcgacaaagcggctggcaacaacagctctttagttccacaagaacaggcagcgatgaaccggcctcaacggttcagagggttggcaactgacccgggtgtgcagcgtaaagcaccagaagcagttatccggcgggcagggaccgcggtcggaaaaacaatttgaacggactcgtaccgcgccagtagcgccgaaaagtcagcttccttcacgtacacaggattgaaggaaggcgaaggagcgcattactgaaaagcccggcgagatgccgggctttttggaatgcctgtcctgggcgccagcatcgaaatccattgtgcccgcaagtgcgggtgggcaatgcacatcgataaaccatctaacagacaactgaaaaaaggaaaaaacatgcgccgatatggacgtgttgatcaggatcgaattgtcgagttttttgaaaccgacggtgacatcacgcaaatgtttcacccaagcattatctgggcagaagtgaccgatcaccccgaagtgcaactgggctgggtcgccaccaaaaccgacggtgtctggacctttgccgcctatgtgccgccaccgccgaccgagcaggaactcatcgccaaggcgcagctgaacaaatggcaactgttgaacgtggccgccaactggctgctgctcaactccctgcagttcaaggtcgacaccggtgtggccacccctgacgaacaggctctgttgctggctcacaagatgtactccatcgctgtcagcgacatcgacaaacaatcgggttacccggcaaacattgtctggccggtggctccgtactgacagtgtttgaaagacagcactgacgactatcaaatcaaaggaagcaagaatgaatcgctacatactgatgaccacggcctattcctacaaccttgtcctcgacgtggtggataccgacgggccgatgcctgaggtgccggcagatgagccctattcgagttggcaagactataccggtaacactactgcagagccgggtatgaaaatggtatggaacgggctaccgagttttgttccgacaaccgcaactgagcgggaggccatgaatcagggacgcatccaaacgcggcttcaggaggcccagagctggttgatgttcaatcccgtgcaatacaaatcggacctggggactgcctctccagccgaggaggccgcattgcttgcctacaagcagtacttcgtggcggtcgccgaagtgaaaaatcaaaccacctttccgaagctcaactggccggtcgcaccgttctgatccagcgagcttcaaactcgacatcgagaacgcattactgaaaagcccggccaccgcgccgggctttttggaatgcctgcctcgagagaaaacgattgaacccgacacacaccactcatccatcacaccaggaggcgtgacatgacaaccgagcaacaagcgttggcggacatgccgatctggctggtcatcctgcttgccgtggcgggcggggtctccggcgaaatgtggcgcgccgacaaggacggcgcccgcggctggccactgctgcggcggctggccctgcgctccggcgcctgcatgatctgcggcgtctcggcgatcatgctgctgtacgccgccggcatgtcgatctgggccgccggcgcttttggctgcctgaccgcaatggccggcgccgacgtggccatcggtctgtatgaacgctgggccgccaagcgcatcggcgtctgcgaagttccgcccgccaatacgaataaggagcaatgaaaaaatacagcggtatttgaaaaggagttcatttcatgttgagcgattttcgttgtggaaaatgcaatcggttactcgcaaaagtagatccacttcatcaagtgcaaatcaaatgccctagatgcaggacgttgaattacgcgaaaacgggatgctttaaaaaatcgcctgtgagcgaaccagggcagcagtgactgctaataataaataatcgacttataggtgatatatatggctacattgccgcgttacccctttacaaccgacggcagttcgattctgttgccgctgcatgaaatgtctgctggacaatatcttcagtcgccagacaagcgttttaaattgattgttcaacccgatggcaatctggcgatttacgaaggagcaaatacagtttgggtggcgattgccggccaaccctatacaagctccgggaagcagatagacaactcaaaaatttacttttatctgatgtattacgcgttcctcaatgatccaacgcgtggccgtatgtggggcactgctaacagcacacctctcaattctgatatctgggcggcttacaatcgtgcctatctatctctgcagaatgatggaaaccttgtagtggtcgactcgatccccgtctggtcaagcaactctgccattcctatcagtccatctgtggagtccgtatatattccggcaggtacaacgcttgaggttgaccgtcggtatgttgtgggagggacgactctggtcttccagtcggatggaaatctggtggtttcaaacggaccacttggagtcctgtgggcgagctggacccagaacaaaggtgccactcgtgcagtcatgcaggaagatggaaattttgtgatctatggacaaaacaatacaccgctctggtttaccggaactgccggtcagccaggtgcaatggcgaaagttcaggcaaatggcagtttctctattgtcagtgaaaagccggtttgggctcgatttggtttcacgccaactattttgccaaaacgcgtattccagtgggacaacggaccatggaaaccgctaatcgaaattcctttgtggcgttttaaagattaattattttgaaatttgcctcccgcttggggggcattttcataatgcttccatccgatgttttatgcgtgcttcacgaagtttcaatttgaatttatcgttgtttagctgaaacccgatatttcgcctcgctgcatgttctgcggcgggactgcgcgtggacattcaaaaaggaggtcatgcatgcctgtaccgatccgacagccttcgcagctgttcacggcaatggcgacagccttgcgcaataacgccgacctgaacgtgcaggtcggtaatcacgatgacttcaccgcacccggcgacaaggcctgggtgctgatcgacatcgaacgcaatgcaccgggagagcgcgcggccaatgggcgcattgcccacgcattgacgctgtcccttcaggttattccggccatatccgccaccgcgtttgccgcgtgtgacctgattgccgccctgaaaaacctgatcaccgacaaccgctggggcctgcccggcgatcagtgcgatctgccgatgaatctcgacggtttgccgtcgctggcgattcgcgccgatcagcccaacaaggcctggaccctgacattcaaccagaccctctacctgggcccgaccttgatcgacgacccgctcggcacaccgaaattcgcccgcacctgggaagtcagcgacatcgacgaccccgaccaatacacctcgctggaggcctgaccgatgttcgacgcgttactgcgcatgcaactgggcccgatcattgagcgtcttgccgagatggaagcggagatcgaagacctgcaccgacgcgccgaaagcttttgccgcatcggcatttgtcaggaagtcgatgcggcgagcaatacctgcaaggtcagtcacggaggattgctcaccccggccatcaagttcttcaacccgagcgccggcgcgcagagcgagtcgcggattcccagcgtgggtgaacagtgtctgctgctcaactacggcagcggagagagtggcgcacaaagcgtggcgttgtttggcttgaacagtgaccgctttccacccgttgcgaccgtccccacgctgacgcgacgggtgcatgtcgatggcagtgaaagcggctacgacgacgccacgcacaccctgcactggcaaaacggtccggcagcgttcagcggttctcgtgaagcgcttgaactgagcatcggcccggcgcgactggcgatgacagcgcaagcgatcaacctgcaactgggcgccaccggcctgaccatcgacgcctcgggcgtgcacttcagcggcccgttggtggatcaccagggtcgcgtcatcagcccctgaatcaagagcctcccatgatcggaatcgatagagacaccggggccacggtcgacgattggctgcaattcgtgcagcgcgcgacacgagccctgaccacgccgctgggcacccggcaaaaaaggcccctttatggttcgttgatccccacgctgctggggcaaaacctcggcgatgacgttctgcttctggcccagagccacgccgcgcaggcgttctacaacccgcagaacggcatcggcgatttccagcccggcgtgatcgtcgccacccgacagggcgccggcctgctgctgcgtttcgccggcacctggaaaaaccgccaacagactttcgaggtcgtgacatgagcatgttgatccctggtcagaaccaactggccgaaccttcactgatcaaggtcgaggccttcgaggatctgctcgccgagttcaagaccttcgtccttgaatacgtcggtacccgttcgccggacagtgcggcaaaactcaagatcagcctggaaaacgaaagcgaactgctgacgatggcgctcgaagcgttttgcgttcgcctgcaaacccacgaacgcaaatacaacgcccgcatcaagcagatgctggcgtggtgggcgaccggcagcaaccttgatgcgcggctggctgacatgggcctggagcgacagttgctcgacccgggcgacccggcggcatttccgccggtgccggcgatttacgaaagcgacgatgacgcccggttgcgctactacctggcgccccatgcgccggcggcaggctcgcggatgcagtaccgccgcgaggtgttcaccctcggcgagcggccgtcggtgaaagtcgaatccaccgatgccggtgtcgtcgacgtcacctacacctttgccccggacggactcgccgcacaggtcaaggatggcaatggccgtcgcaccgcacccggtgaagtgcaggtgacagtgctgtcccgcgacgccgacggcacaccgtccgctgcattgctggatggcgtgcgccaacacttcgcccggcccgatgtctgcccggaaaccgacaaggtcacggtcaagggcgccgagattcagcgctacaagattcgcgtcgtggcgaagatcaattccggcccggattcgggcctgaccaaagttgctgccgagcaacatctgcaagcctacgccgacagttgccatcgcctggaaggccgggtcgccccgagctggatcgactacacgctgcacagcgccggcgccgtgcaactggagattcttgaaccgctgacaccgattgtgtgcagcgcgtttcaagcgccttactgcacggcggtcgaagtcgaggtgcagaccctatgacggaccagacaccgcgtccgaccctgctgccggccaacagctcggcactggaacgggcgctcgatatcggcttcggcaccttgcttgaccgcatcgtgccgccgtttcccgaattgatgaacccgagcgaaacaccggtcgcgttcctgccgtatctcgcagcggatcgcggtgtggccgaatggagcaccgacgcaccggaggcggaaaagcgcctgactgtcgaactggcctggcccaccgcgcgtcaggccggcactcgcaaggcactggaaaacgccgccaaggggttgcaactgaggccggaaattcgcgcctggtacgagcagacaccgccgggcgcgccttacagcttttccgtgcgggccttcaccgaacaaccctacagcgaagaaatcgacgcccgtctcgaccgacgcctggccgatgccaagagcgaacgggacgtgctgtcggtgtcggtcggcctcagcgcattcggcaaccacgtcatcggtgccgcgacgttctgcggtgagctgaccacggtttacccggtgttcctcgaagggctcgagacatccggcgagtccttcaaggccactggtctctacaccgtcgaaacatccactatttatcctcagggggcctgaatggctgactattacaccctgctcaccaacgcagggattgcctacgaaaccgcctgcaaggcagcgggcgtgccgatcaagctgacgcagatttctgtcggcgatggcggtggcgcggtctacaacccggccgcgaccgccactgcgctgaaacgcgaagtctggcgtggaccgcttaacgcgctgtttcaggacgagaaaaatccgagctggctgctcgccgaagtcaccatcccgccagacgtcggcggctggtatgtgcgcgaagccgggctatggaccgacaccggcattctctacgccatcgtcaaatacccggagtcgttcaaaccggtgctggccacgtccggctcgggcaaagagttctacatccgctcgattttcgaaaccagcaatgcttcgctagtgacgctgctgatcgacgacactgtggtcaaggccactcgtgcctgggtcatgagctacctcgccgaagaactcggcaaacttgatggcaaacaatcggtgcgcgtcgccgccaccgccagcgtggtgttgaacggtgcgcagcagatcgacggtgtggcggtgattgccggcgaccgcgtgttgctgccgaatcagactctggccaaggacaacggtctgtggatcgtggccaacggtgactgggttcgggcaaccgatgccaacgtcagcgccaaggtcacaccgggcctgacggtgatggtggaagagggcacgctcaacggcgattcgctgtggcacctgaccaccaacgcgccgatcaccctcggcaccactgcgctgacattcaagatgctcgcggggcgcaccgggattgctgccggcacttacaaaagtctgagcgtcgacgagtatggccgcgcaacagccggctcgaatcccgacacgctggccggcttcggcatcaaggactcctacaccaaggccgaagtcgaagcactgatcgccaaggcctcggcgttgccggtgggttcgattgttgccttccctgtcgatacaccgccgccgggttttctggagctggacaacagcgtcaaaagcagcgcgacttaccctgacttgagcgcctatctgggcggcaagttcaacaagggggatgagggtgtcgggaatttccggttgcctgaggcgcgtggggagtttttgcgcggttgggatcatgggcggggggtggatgcgggccgagagcttggtactgcgcagaccgaagcgttcaaggcacacaaccatcgatattttgatagcgtcgcagcaaccatggatccagcaggtggttggcagagtgggaccgttaacggtacccaggccggtgtttccccaggtgcatttatatcggttaccaatactggtgatgccggtcagatgctgaatgcacataccaccgtcaacaccggaggtactgaaacccgcccccgtaacatcgccgtcatgtggtgcatcaaggcctggaacgccccgatcaatcagggaaatatcgacgtagcggcactggtcaaggaagtctcccgtttgggatctgccgttccggtgggtgctgtcatggcgttcccgacggggatcgtgccgcccggttttcttgagctggatggcagtgtgcaaaacattgcgacttacccggatctggcggcttacctgggaacaacattcaacaagggcgatgaaggagttggtaactttcggttgccggaatctcgtggtgagttcctgcgtggctgggatcatggtcgtggtgtggatagcgggcgaaattttggcacgtatcagactgacgatttcaaggcgcacaatcatccgccggcaaataatcgtccgggcttcatgactaatgagtttccaacggttcaggcatatcacgcagccacttcggggggacctcaatcctactcgggtgaagggcaacagattgctacgacgggtaaccggggaggcacggaaacccgccctcgcaacctcgccgtcatgtggtgcatcaaggcctggaacgcgccgatcaatcagggaagcatcgatgtagctgcactggccaaggaagtctcgcagctgaaatcgtctgttccggtaggtgctgttctgtcgtttccaacgggtgtcgttcctgccggctatctggaactggatggcagtgtgcagagcattgcgacctatccggatctggcggcgtatctcggtacgacgttcaacaagggcgatgaaggtgccgggaatttccgcttgccggaatctcgcggtgaattcctgcgcggctgggatcatgggcgaggtattgatatcggtcgtagtgtcggcagttatcagtcgggtacgaaaactcagggcgatgacggcacggcgccggctgttcaaggtatcggcaactccaatctgattgatgctgatcctgctcctggcttcagtggcgatatttactacacctccaccaatgtcgtcgtgcagaacttttccaactcgttctggaaaacggttcgcccacgcaacctcgcggtcatgtggtgcatcaaggcctggaacgcaccggtcaatcagggaagcattgatgtcgcagcattggctgcagatgccaggtcggctcgactcaacggtgcagaagtcggcgccgcgcgtaatctgagagtgtcgctacccgctgctgcatcggttgcaacgcttacggccgaccaattgattgtcgagcaaccaggcgttggccagtacaagctatcgaacgtcaatctctctataaatctagccaccattggtgcgggcggaatggacttcggcgttgcaccagcaaacggcagtgttggcatttacgttatttacaaccctgagttgaaggttgcaaagctgctgggcgtcaacgcgacatcgacttctgttccggaaatttacactggcaccaacatgcccgtcggttatagcgccagtgcgctggtcagtgtgtggcaaaccgatgccaatcgattgatgaatgccggcattcaacatcagcgttcaatttccatcattcagacgatggtgctggaaaacggattatcgatgtcgtcgacaccgatctcgctggcctctgtcgttccgaagaatgcgaaaagtgtcggtggttacattcattacattggaagcgctgatttcccgggtggtggctctctggggctttcgccggatgtcaccgaagtggggctgaaagcatgcggcatcggtggaatcgtcgggttgggtgttctcagcccgttttcggatctggtcatgacgactccacagaccatctattaccgcctttatgcgtcggtttcccgagcaaacgatgtccacatctcccaatacactttctaaggagtcctctatgttgagagcctactcaaattcagggacggcctttcgttgtgtcgccccggactggccgctatctgacggtgaagtactgtttgaccatgaacccaccgtccaggaactggaggacgcatttgggttcgcgaacggcgagctggttgtaaagcgccaatgggaacagattgcagaagaacgattccgtagagagggttcgggcatcgtggtcgcgggtgtcgctatcgatacgtcccgtgacagtcagtcactgatcgccggtatggcagtttctgcgatgctcgatcctgagtaccactgtagctacaaggctatcgaaggatttatcgatattacctctcagcagatcctgcaaattgcgcaggctgtgcgttctcatgttcaggcttgcttcgatcgggaaaaaacgttgtacgaatctgctcaagcaggcacgtatagcagagaaatgctgaccgaaggatggccagattcctcgcctgaaacaccaccgaaaaaccttcaataaccccctgcaatccagggcgtttacttgctaaccaacacccgccagcccctccccacgaggggctttcccgtttatggagaaacgaaaaatggcaacccgccaaacctacaccgtgctcgttccattccccaccggcggtgggcactggtcgagcgtcggccaggaactcgatctgctcgacgtcgaggccagtgccctgcacagcgccggtcgactggagctgaaaacacctaccaccaaggccgtgaaggccgctgccaagaaggctgactgaatatggctgaggttctgaacttcgagcacaacggcattaccgtcaatgccaccgaatcccccgaggccatgggtggcctgggtgacaacgtcatcggtctggtcggcactgcgccgaaagccgatccgctgattccgcgcaacgcaccgtttcgcatcaacagcttcaccacccacgcgctgctcgatccgaccggcgcggaagagggcactctgtaccatgccgtttaccagatcctcaaagtggtcaaggtgccggtgtacgtggtgatcgtcgaggcgggcgcgaccccggccgacaccgtcaacgcagtgatcggcggcatcgagccagccaccggccgcaaactcggtctggcggcactgggcagcgtcccggaagacctgaccatcatcggcgcgccaggcttcaccggcaccaaagcggtggccagcgagttcgcctcgttcggcaagcgcatcaaggcccgtgtggtactggacggcaaggacgcttcggtcgccgaccaggtgacctacagccaggaactgggcggcgccgacctcggtttcgaccgttgcctggtggtgcacaacatgcccgccgtgtactcgaaagcggcgaagaaaaacgtcttcctcgcgccatccagtctggcgattgccgcgctggccaaggtcaagcaatgggaaagcccgggcaatcaggtgacctacgccgaagacgtgtcccgggtcgttgagtacaacatcctcgacacctccaccgaaggcgatctgctcaaccgctacggcgtcagctattacgcccgcaccgtgctgggcggcttctcgctgctgggcaaccgctcgatcaccggcaagttcatcagctacgtcggtctggaagacgccatcagccgcaagctggtgaaggccggccagaaggccatggccaagaacctgaccaagtcgttcatggatcaggaagtcaaacgcatcaacgactggctgcagaccctggtcgccgacgaaaccattcccggcggcagcgtctacctgcacccggaactcaacagcgtcgagaagtacaagaacggcacctggtacgtggtcatcgactacggccgctacgcgccgaacgaacacatggtttatcaactcaacgcccgcgatgaaatcatcgagcagttcctggaggacgttctctaatgtttaccaaccgtaatcgccaggccatcgcggccaccctgcaaggcctgccgctgtcggcgaccgtggaggaattcactccgccgaagatcgaattcgatgtagaagaaatgcgtggcggccgcttcatcgttgaagaaatggtcaagggcggcaaagcgctcaacgccaagttgaccctgcaaggcatgggcgccgaggtcatgcttgcactgggtgtgaagctgggcgacgacatcctgctgaacgtgcgtgaagccggtcaggaccaggacggtaacacctggttcacctaccacacggtcggcggcaagctgaaatccctggaggaaaccgcggtgaagatgggtgaaaaacccaagaccaacctggagctctcctgccgtacttacaaccgtctggaaaatggcgtgccggtgatcgacatcgacgtgcgcacccagaagttcgtactcaacggcgtcgacatcctcggtgatgcccgtcgtgcggtgctgatgccgtaagcctttcggcgcatcaagcacaccctgtgggcgcttatgcccacagggatcttcaagaacacccaaggaattcctttcatgtcgtggatgccacccaagcatgacctgttgtcgccgatcaccggtgacgacggctcgcagatcgaatcgatccagctcaagcccctgttctacgccgcccagaaagaagcgctggaacgcgccggcgatgacgaagacgatcagttcttcgaactggcgctgctggccaccgggttgtcggtcaaggaactcgaccagctcaaacgtccggactacgtgagcatcgcgcagtacgtacacgagatgtcgacccgtccggcgtcgtactttctcgaccaggtcgaagacgcggaaaagtccgacgatcccgaccaggtgcaactgctgcaaccgctcgccgtcaccggccgcaccgtgacctcgctgagcctggaaatgccggcgctgcgggccaccaaagtgatgaagaaactgaaaacggccaaggaacgcgccgagttcatcaccgcccattgcaccggcctgatgatccccgatctggccctgatgagcgtcccggactggacgcaattgcaggtgcgcatcgacgattttttaaaccagccggcggccttctttcagagcgcgacatcgaagtaatcctcgatatcgtgccgctcatttacccggtaagtgaggcggaaattctggagtgggacgccgaaaaggcgttgcgccgctacgacatagcgatcactcgccttggcgtgaaacaggagtagagcggcatggcacagagcaaatttgcgctcacatacgccaatgagagtggcaacgcagcagccgggttaaagctgcccgatggccttggcaaaccactgcaggacttgaacctgacaatggcgctggcgagcgcggatatccgcttgctgacccaggagcagatcaagcttcgagagctgttggccaatcagcaatcgctgttcaaggtgagtgctgcatccccggctgcaagcgccgaaccaaagtcaaaactcaaggccgagatcgagcagcgtccacctccaaagctcatgcaaccagccatggccaacgagacggcgcttgtcgaactcaatcagttgctcaaactgagcaatgatcagcttcaagcgcactcgcagagcactctggaactcgccagcgagaaacagatatccgccagtggtgcgaccaacgcggatctgttgcaagtgcagcttgccggagccagatccggcattgccgatggtgccaaaggtgaccagcgggcgaacgcactgaagtggttctcccatgatgccgcaatcaacgcatcggcattcaggatggacgtcaaggcggctggcgaaatgctcgccgcatggcgctcctcgctgaagctggatcagtatcaaagccaggatcttgcggatgcaacgacctacctcggcaatagtggtctggatgccaaggccgcggacatcggttcggtggtgcaacgttccggtgagagtgcgattgccgccggattgactcccgaacaggtcgctgcattggcggcggcgcttctcaatagtggtgcggacaaggagggcgccagcgccgcgctgaaaggcatcacctcgatgctggccaaaggcggtgcggtatcgactgagcagcgaacagccttgactcagttagggcttgatcctcaatcgctgtctgagggtatgaagaaggatgcgcctgctgtcatcaactcggttcttgctgcacttaacaagcagcctgtgcaagagcgggcggcactgacgaagacgctgttcggcgaaaacgacaccagagttctcgaactgctgaagaagccggacgatgtaaaaaacgccttctcgctggtagccgacaagcacaagtacgcaacaacggagcttggcgcgggtgaaggcgctgcggcgaagtccgcagaggcgttcggcaatacttcgcagggtcgctggaatgcgctggacgcaagtctgacccggttgaccacatcattcggcacggcgcttgcgcccctggctgacggtgccgccgtcgtgctcaccgccctggtcaacggtgttagcgcagcggcggaaacgttcccggcactcacggcaggactggctctgctcgccgtggcagccatgccgttcgtggggggggcgttgaagtccggcgtggcctcggtgctcgacgtggtttccacgaaactattgcgcctggcatcgacgcgactgccgccggatattgccgatgtgataggcggtgatgacaacgatgacgacggtcgaaaacgcagaaagaaggggcgcggatcgcgccgacgccccccttctgctgcacggtcgtccggcaccgcttccataacccgcaagagcagtcgcttgagtggtgtgacggccagaatcgcacccatgttcgacgatgcgctcacccgattcagaatggttggcgatgttgtcaaaagcgccatgccgagccggctgagcggggctggcgcgaaagtcatgtcgttggcagagggcttgggagccaggctcatgccctcggttgtcaaggcattgcctgtcatcaaggttggcgcgcctctggccattgctcatgctgcctatacagggttgaaaggttggcgcgaaggtgacgacaaagcggtaaagggcgcggccggcgaactggccggaacggcgattggcgctacgatcggtacgttcattgcgcccggcatcggaacctttattggtggcacgctgggtggaatagccgggtccattctgggtcaaaaactggcgacgccacctgaagacaaattggcaccgccggcacaggtcgccaaagacgtatccattgcgcaaacgcaaatgcaagcgtcaaacccgcaatacacttacgcaccttcagttcatgtcagcggcagcgaactggttagttccgagaaagtcggcacgatgctttcgcaggtgctggagtcgcacttcaattctcaatttgtcccgggtgtggctaccaatgccctcgccacccgccgtgacgcagccctgaccgatggagtcgcctgatgaaacaacaaatggcactgggcagtttcatcttcggactgtcccgggattttgcgtacagcacgctgtcgcgaaaatccgagggtggctggaccgagctgcagatcctcaacagcaaacccagatcccatcagacaggacagaagcctgaaaccctgaccatctccggaacctcgatgtacgccgtggcgatggagcggctcgatgagctgcgtgcgctgcaagcgttgagagtaccgctgccgttgattgacggcatcggtcgtaactggggtttgtggcggattaacagcatcgacgaaaaccagagcgaggtcatcgatgacggaaccgcgatggtgatcaagtgggtcatcggattgtcggagttcaacaatgcgtaaggtacgaagcgtggccggcgattcggtgaatctgttgctgtaccgcgaaaccggtcgcagcgatgacagcgccgaagaagccctgtggacactcaatccgaccctggccgagcacggtccgattctgtcggccggtgtctgggtgacactgccggaactcgatagcaaaccggccgcgatcaaaccggttctggcctgggattaaggaggcagcatggcacagggatttacgccggcgatcgaaatctacggcgccaacaaggacctgctgaaccagcgcctgatcagttgggaacacatcgatgctgccgggatggagtccgatcaactgacgctggtgctcgacctggaaggccttgaaggcttgccaaccctgggcggaatcatcggcctgcgggtggggtatctggagaccgggctggtcgaaaaaggccagttccgggtgactcgattgacaccgacgctgttcccgctgcgtctgacgctggtcgcgaccgccgcacctttcagcggcaaggacgaaaccggattcaaggaacgacgcacggccagtcatggccccacgacgcttggcgggctgtttcgcaaactggtcgagccgcacggtttctcgccgcgcgtcgatcccgaactggcgctgatcaggattgctcatgtcgaccagtcaaatgaaaccgacatgggcttcatcacgcgactggcgaagaagtacgacgcggtggccaaaccgttcaacgacctctacgtactggcgaaaccggcgcagctcaaaaatctgtcgggtcaggtgataccgaatgtgaggctgtcggtgacccacaacaatcggccgggcgaacacgccttcatcagcgctacgctggaagagaccgcccgcacccagaatgaaggttgcaaagtctgctgttgggacgccaatgccggcaaacaggtggaggtgaaaaccggctcggcgccctacaaggtcgttcgtcagaaacaggccagtgtggaagaagccaaagccatcggcgaagccgaagtgcgcaagatgctgcgcgagaaatacaagctgaaggtcacctgcccgggcgatccgctgctggttgccgagggcctgctggtgctcgatgacacctggccggacttcatgcgcggtcgctggtcgatcgagaaggtgacagccagcggcaagcccgaagaaagctatcgctgcctgatcgaagcaaacggccgggatcccgaggcaaaagccaaggactgatcccccgatctcaccaccacactcctcacggtggtcactcccaaaacctggaacgctccccatgaagatctccccgatcctcacgcagctgcgtgcgcaatgcccaagccttgccggccatatcgcgacaggtgtcgacctggcgctgctgcaaggcaacccgaatctgccgaccccgtcggctcatgttttaccgctggccgatctggccagcgccagcaccgcacagaattccgccagtcagccgatccgcgaccgcttcgaaatcatcctggcacttgatgccacggacgccacaaaagcgctggatctgttgcacgacctgcgcgccgaagtgtggcgtgcgctggtggggttcaagcccggttccgactacagcgccatcgtttatgacggcggcgaaacggtctcgatcaacagcagccgcgcgttctaccggctgcgcttttttgccgagttccagctgggccgcaatctgccaagtcagcctgcggagagttggcacgaacgtgaactggacggtttgtcgtcctttaccggggtcaccgtgcgggtcgatgcgatcgacccggccgaccccaacctgaaacacccgggccctgacgggcgcgtggaaatgactttctctggagacgtaaccccatgagcaaccgcatcaccgtagtgccggccactggccgtgccgtgccggacccggaagcaggcgacctgctgccactggaaggccgtgaagtgctggacagcgcctggtggcgccggcgtctggccgacggcgatatcaccctcaaaaccgcaacagctaaacaaaagggagccaaataatggcgatcggattcagcaacattcctgcggacattcgtgtaccgctgttctatgccgaaatggacaactcggccgccaatagcgcgtcctcgtccatgcgccgcctgatcgtggcacaggtcaacgacaacatcgccccgagcgaagtcggcaaactggtgctggtctccagcgtggcactggccaaaagcattggcggccagggctcgatgctcgcctcgatgtacgagaccttccgcaaggccgacccgatcggtgagatctggtgcctgccgctgcacaacgctaccggcgccatcgccaaaggcgtgctgaccctgaccggcaccgcgactcaggctggcgtgctcaacctgtatgtcggcggtgtccgtgtgcaggccaccgtggtcaacggtgccacggctgcccaggcggccaccgccctggcacagaaaatcaacgccaccgccgatctgccggtgagcgctgtggccgctgaaggcgtggtcaccctgaatgccaaatggaccggcgagagcggcaacgacatcagcctgcaattcaatcgcctgggcaagagcaacggcgaagaaaccccggccggcctgaccactgccgtcaccgccatgaccggcggcgtcggtgtaccggatcaagtggcggccgttgccgcactgggtgatgaaccgttcgaattcatcgcgctgccatggtccgatctggcgaccctcaacacctggcaagcggtgatggacgacagcaccggtcgctggtcctgggccaagcaactgttcggtcacgtctacagcgccaagcgcggcaccgtcggcactctggtggcggccggtcaggcgcgcaacgaccagcacatgaccattcaggcgctggagcctggcgttccgcaaccggtgtgggtacaagccgctgcactggctgcacgtacttcggtgttcatctccgccgacgccagccgtccgacccagagcggcagcctgccaggcgtcgatccggcgccggccagcgagcgcttcaccctgaccgagcgtcagtcgctgctcaactacggcatcgccaccgcgtactacgaaggcggctacgtgcgcatccagcgctcgatcaccacctatcagaagaacgcttacggccaggccgacaactcgtacctggacagcgaaaccatgcaccagtcggcgttcatcgtgcgtcgtctgcaaagcgtgatcaccagcaaatacggtcgccacaaactggcctccgacggcacccgtttcggcgccggtcagccgatcgttaccccggcgaccattcgcggtgagctgatcgcccagtacgccaagcttgaactggaaggccacgtggaaaacgccgagctgttcgccgagcacctgatcgtcgagcgcgacgtgcaggacccgagccgcgtgaacgtgctgttcccgcctgattacatcaacggtctgcgcgtgttcgcactgctcaaccagttccgtctgcagtacgacgacgtcgcctgatcggctcgtttgacactgtgatttcagcccacctcgcgtgggctttttatttgaagggagtaacaccatgggtcaactgattgcaggcacctgctacgtcaaggtcgacggtgcacaactgaccatcaatggcggctgcgaagccccgctgatggccgtcaaacgcgaaaccgtcgtgccgggtttctacaaggaaaccgacatcgcgccgtcgttcaaggtgaccgcgctgcacaccgccgacttcccgctgaagaagctgatcgaaggcaccgacatcaccgtcacctgcgaattcagcaacggcaaagtctacgtgctggccggtgcctacctggtcgaagagccagtctccaaaggcgatgacgccaccatcgaactgaaattcgaaggcatcaaggggacttggcaatgagcggcgccgtgaagcttcaagttgcgatcgaagctcacggcgagcccctgaccgaactcgtcctgcgccgtccgacggtgcaggaggtgcgagcgatcaaggcgctgccgtacaagatcgacaagagcgaagaggtcagcctcgacatggacgtggcggccaaatacatcgccgtgtgcgccggcattccgccgtcgtcggtcaaccagctggatctggctgacctcaacgcgctgagctgggccgttgcgagttttttcatgagtgcggcgtcggagccatcaccgacctgatttcggtcgcctatgacctggcctggttctggaaggttgaccccgaacagatgatggccaggccactggatgtgcttcgcgaatcgctggagcacgcgcaacggatcaatgcgatgcagcaggtgcagtgatggcagaagaaaccaaagcgaaagcgtcggtgctgcttaccggcatcgacgaactgtcacccaaactcggcgccctgcgagtgaaggtcgatgacttcaagaagaacctcgaacagaccggcctcggcaaactggacatcagcggtctgttcaagggtgggagcgtgattacgccgttcgtggacggcatcaaatccgccgcagcgtttcagggcaagttgaccgaagtcagcgagacggcgaaaaccgtcgatctgccggaaacaccgaaagccgccgcgcagaacatgaacgtgttcagcgcgtccatggaaagggtctccgctgcggtagacgccgcattggtgccggcggtgggcgccttggtggtcgggctggagccgatgctgacccaggtcggcagcctgctggccgacaacccgaaactggtcgaaggcctggcagcgggggcgattgcgttttccgccatgcaaaccgccgtcaccggtatgacccaggtgatggacgtcatgagcatggtgctcaagaccaacccgatcatgctgatcgccatgggcattgccgtggcggccggactgatcgtggccaactggacaccgatatccgcgttcttcaccggaatgtgggagggcgtgaaaaatgccggggccagtgcaatggcgacgttgcgctcggtactcgactggcgaccgctggaaacgctggcagcgctgtgggaaccggtcacgggtttcttctcgggtatctgggacaaggtcaaagcggtcacggcgccggtgatcgacttcttcaagtcggttttctcgtggtcgcccgcgggcctgatcctggaaaactgggggccgttgaccggtctgttttcggcgatctgggaattgctcaaggccttgagtgtgccggtgatgtcgttcctcaaggggctgttcgactggacgccgctgggcatgatcatcaacaactggggcgcaatcaccggtttcttcgcctcgatctgggtcgcgctgcaaccggcggcgcaagccatcaaggacttcttcggcagccttttcgattattccccgctgggcatgatcatcaacaactggagtgcgatcaccggcttcttcgcttcgatctgggcggcgctgcaaccggcggcgcaagccatcaaggacttcttcggcaccctgttcgactattccccattggggatgctcgtcaacaactggggcagcgtcgtgacctttttcgaaccggtctgggccgcgctgcaaacgtcggcacaaacgatcaaaagcttcttccagagcctgttcgaatggtcgccgctggagcagatcgcgcagtactggcagccgatcagcgaagtgttttcggcgctgtggggcgtggtgcaggcattggccgcgccggtgctggagttcctgcacaacatgttcgaatggacaccgttggggcagatcatcaagaactggggaccgatcaccgagtggttcggcgagctgtggcaaaagctgcaaaccgtcatcgcaccgatcaaggagctgttcgacggcggcttcgccgggctaatcgccagggtcaccggcaaggtcgaaaccttgacccaggcgcaacgtcagaccaatgccgaaggcaagggtgaactggcgccggccttctttggtgccagcccgaaacccgagggtggcagcgcgctgcagggcggttctttgccgcaatcctctggcgcactgatccagcaaagcgccgccaataaccgcacgcaactcgaaggcggcctgacggtccgcttcgaaaacgcgccggcgggcctgcgcaccgatcaaccgcaaaccaatcaaccggggctggcgctcagttcgcgcatcggctatcgctcgctatcggcaggaggttccaatgaactggcgtgaccgtttgttgccggcatcctttcgcggtgtcggcttctggatcgaccaggcgaaaaccccggtcggtcgcaagggacagttgcatgagtatccgcaacgggacctgccgtttttcgaggatctcggccagcaggccaagacccacgacctgacggcgttcatcatcggtgccgattgcctggagcagcgcgacaagctgctccaggccctggagcagggcagcggcgagctggtgcatccgtggctgggccgcttgcaggtcaaggtcggtgagtgcgacatgacccacacccgccaggacggcgggatggtgaccttcaccctgaagttctacccggaccggccgctgccgtttccgacggcgacggtcagcacgcaaaaagtcctgctgatcaaggctgacggtttgctcgggtcggcggtggcgcgctttgaacaggcgatgaccctgatcaaggccgcgcggatcggcatcgccaatctgcgcaacagcctcaccggcgtgtacgacgtgatcaaggagcagctcaagccgctgatcgcgcaatacaagcagatcaccgaactggtcagggccgtcaaggaactgcccaaggaagtggcggcggagttcaaaggattgctcggcgatatcaaggagctgaaggcattcgcgaaggagggttaccgtggcgtgattgccgacgtgtcccaacagatcgaagccatccgcaaggccgacgccccgaagatcaccaccggcaaggacaccacggctgcggcgcaggccctggccaatctggtgcaggacacccttatcgtcaaagcggcgcaatgggtagcctcgatgccggtggcctcgacgccggtgaaactgtcgtcgacgccgtcgctggatcagcagtcgaaacagccggtcagccgtcaggaagtgccggtcaccgacgatctgcaagcgttgcaaaaagagctgatcgaagcgctgcaaaaggcccaggacaaggccgatcccgcgcactaccaggccatcgccgatgtgaaggaagcgctgatcgcgcacctcaaggctgtggcttcgtccggtgtgcggctggtgagcaaaaccttccaggaaacctttccggcagtggtcgtggcttacaagcagtttggcgatgccacccgtgtgaccgaggtcattcagcgcaatggtctgtctcatccgagcttctcacccaacgaagtcaaggtttccagggagtgagtcatgaacgagactgacaaccgcgtgacgctgaccgtcggcgacatggaatacggcggctggaaaaacgtgcagatcaccgcggacctggagcgccagttccgcaccttcaaactcgatatcacctggcaatggccggggcagaccgtggatcagcggatcaaggccggcgacccgtgcgaagtgcggatcggcaaggatctggtgctcaccggttatgtgttcaaggccccgatcagctatgacgggcggcagatcagcctgagcatcgaaggcagttccaagacccaggatctggtggattgcgcagcgcgaaacaaccccggccaatggcaggatcagtcgctgctgagcatcgtccaggccctggccatggagtacgcgttgatggtggtcaacgaaattcccgagaccgcacgcctgagcaaacacacgatcgtaccgggtgaaacggcgtttcagtcgatcgaccgtctgctctcgctgtaccgggtgttttccaccgatgacgccgaaggccggctggtgctcgccaaacccggcagcgctggccgcgccagtgacgcgctggagttgggcaagaacattctttcggccaatgcgccgatggatttcagccaggtgttttccgagtaccgggtgatcggtcaacagaagggcaacgacaagaagagcggggcggcggtcagcgaagttgaatcgacggcgaccgacctgagcttcaagcgtcggcgcaccacgatcatcaacgaaggctcgcaactgacgttcgaactggctcagcaacgggcgcaatgggagagcgcgacgcgcatgggccgagcgctgaccactacctatcaggtacagggttggcgccagtccaatggcgatctgtggcgtcacaacacgttggtgcgggtcaaggatccggtgctcggattcgatgaagacatgctgatttccaaggtgacgtactcgctgtcggcgcagggctcggtgaccaccctgcaagtggcgccgccgcataccttcgacgcgaacccgactcccccgaaaaagacctgagcccgaccccgccctccaaggaaaaccctatgagcctactgacacgcctgctggcgcgcggcactgtcgtgctcgccagttcggcctccaagctgcaatcgctgcaaatgcgcctcaccgccggtgaagtgaacgacgacatggagcacttcgagccctacggctttaccagccatccgctggccggtgccgaaggcgtcgtcacgtttctcggcggcgaccgttcccatgccatcgcgctggtggtcgctgaccgccgttatcgcctgcaatcgctggcggccggcgaagtggcgatctacaccgacgaaggcgacaagatccacttcaggcgtgggcggatcatcgatatcgaaaccgccacgctgaatatccgcgccagtacggcggtgaactttgacacgccggtgatcaaccagaccggcaagatcgtttccaaaggtgatcagctggccggcggcatcagccagatcaaacacgtgcatggcggcgtgcagggcggcagcggccagaccggtgtgccggcgggaggtcagtgatgcttttcagtcaaaacctccacgccgcgctgacccgctcggtgctgatcagcctgttcacctggcgccgcgccgccgacgacgatgccctcgatgacgaggagcgttacggctggtggggcgacacctttcccaccgtggccgacgaccgcatcggttcgcggttgtggctgctgcgccgggtcaagctgacccgacagacccagatggacgccgagttctatgcccgcgaagccttgcagtggctgatcgacgacggccattgcagcgccatcgacatcatcagcgaacgcctcgacgcccagcgcctgaacctgcgtacggtcctgaccctggccgacggcgaacgcctggacatcaaccccgataacagttggcaggtgatctatgccgtttgaaaccccttcgctgccggtgctgatcaagcgcacccaaagcgacctggccggcgattcgctgcgccagtccgatgcgcaagtcctggcccgcaccgtcggtggtgccgcttacggtctgtatggctaccttgactggattgccgagcagatcctgcccgacaccgccgacgaatcgaccctggaacgcatcgccgcactgcgcctgaaccagccgcgcaaaccggcgcaaagcgccaccggcagcgtcagttttactgcaaccgcgggcgcggtgctggacgttgatacgctgctgcaatcgagcgatggccgtacctacaaagtcaccactgcgcgcaccaccgtcaatggcagcaacaccaccaccatcgcggcgctggatgccggcagcctcggcaatgctgacgccggactggcgttgactccggtgcagccgatcaccggcgtggtcggcaacagttttgtcgtgctggcgccgggcctcagtggcggcgtggcgcgggagagtctggagtcgctgcgttcgcgggtgatccgttcctatcgcgtcatcccccatggcggttcggccagcgactatgaaacctgggcgctggaagtgccgggcgtaactcgtgcctggtgccgaggcggcctgctcggcccgggcacggtgacggtgttcatcatgcgtgatgaagatccgcaaccggtgcccaacgacgagcaactggcggaagtccaggactacatcgaaccgctgcgaccggtgacggcggaagtgcatgtgcagcgaccgattcaagtgccggtggtgtaccgcttcaagagcgtcaacccggacaccaccgccgtgcgcgccgccgtcgaagcgcagttgcgcgacctgcacaaccgtgaagccgatctcggcgtgccgttgctgatcagccatatccgcgaagccatcagcagcgccggcggtgagtacgatcacaccttgaccgcgccggccgctgacgtgcctgccggtcaaagcgaactgctcaccttcggaggttgcgtatggggggcataagaaccgctgcgcaatatcaggcgcagcttcgcgcactgctgcccagcggcccggcgtgggacccggagcgggtgcccgaactcgatgaagtgctacaaggcgttgccgtcgaactggcgcgcctcgacgcccgcgccgccgatctgctcaacgaaatggacccggccggcgtcagcgaactggtgccggactgggaacaggtgatgaacctgcccgacccgtgcctcggcgccacaccgctgttcgacgaccgtcgcctcgccgtgcgccgccgcttgctggcggtcggtagccaggccgtcggctactacctggaaatcgccagaagccagggctaccccaacgccaccatcaccgaactcgaagccccgcgcatgggccgctcgcgcttcggcgcggcgcactggggcacctgggaagcgcagttcatgtggacgctcaacaccggcggccgcttgctgctcggccggcgtttcggcgcgagttactggggcgaacgcttcggcgtgaatccgggctcggcgcttgaatgcctgattcaccgggcggcgccggcgcataccaaggtgcacatcaactatgactagggaataacgcaatggattatccgaagagtgtgcccagtgccggtctggtgaatgggaaatttgtcgatgaaaacccgatgaccgggacgcccggatcgttgattccggcggactggggcaacggtgtcacgcaggaaattctcagcgtgatcaaggccggggatctgaccccggatgagaagaaatacgatcagttgttgcaggcgattcagacggtgacggccaagggctggaatcaggatctggcgctgccgctgtcggccttgccgctgccaaccgttgccactacggatgcgcggatgccgatcacgccggccgccgcctcgaccagtggcgggcgggtgtcggtgccggcaggtatctacgtcagcattggccaggaagtagtggcggggcagttgggacgttcgcggacgttcaccactcagacctggagcagcgccgatctgttgccgagttctggttactttctgcgggcgcaggtggtgagtggtgcactgacgttctacatgcagcgcgggacgatttacgacgtgacgcccgattccctgaagggcacggtcaacggtgctgccggcggtggtttccagagttcggtgctggacatgtgcctggcctgggtggttaccggtgcaccgggctcggtaccggtagtgcgtgcgatctataaccgggcacgcctgacctgggcgcagacgctcaacggcacgggggcagtgtttctgccactggatcctcatgcccgcgctgcgcgactggtggtggggaacccgacgccatcgtcgactgctgttacaacggttgcgtttccttcgactggatgggcgggtggcaactacagctacctttcgcccgtatccacaggcgtttccaataatgccggaggctggaatcctgccaccgcacaaccgtgcgtcatcttcaccaacaacatcgtcaatgacgtcacggtttcgacactgaccgccagtttcgatcacgccaatgtgcgctcgctctggcagtcctatcaggccgaacacaacctggcacaggccagcgccgacagcgatgagctgttgctgagcatgggcatcaagagccatccggtgaccgattacaacgccggtattccgatcaactttagcgaagctgtgaacgttcagctgtcgtgggagctcattcgatgatcgtcattcaggaactgcatcagatcgatggagagttgcgtcctgcgcagccgtccgccgcccatgactgggacggtgaacaatgggtcgtcaaccctgagaaagtcgcgctgctggaacaacaggaaactgaaagcctgtgtgcccgggtcgatgttgccgccgacagtgcacgcagcgtattggccggggatccgctcaaggcgttggagtatgcccaggcagccattgatgctcaggcctttcaggacgccggttatccgaagaaggaagtgccgctgtccgtggccgcgtgggtcgccaaaggccggtcggcgaaacaggcagccgagcagatcctcgacaaggctgctcaggtcagcgacagcctgttgaccctgcgcaccttgcgcctgaaggccaagacccagatccgtgggtacgccggcaaaagccagatggatcaggcgcgtgccgccacggacgaggtgttgctggccattcgtgatctgacggccatccagagccagtaaccgctatccgcctcacccaagcccacgtcagcgtgggctttttattttcaggaacagaagcgttggaaccgctgcgaaacccttcgcgccgccgcgtttcatttgtcatgacagaggaacgaacatcccatggattatccaaaaagcgtccccagcgtcggcctggtcgacggtcgcttcgtcgatgaaaacccggtggcgggaacgcccgggtcgttgattccggcggtgtggggtaacagcgttacacaagagattgtcaacgtgatttccggcgccgggatgaccgccgtcgaggccgataacggccagttgttccaggccattcagtcgattgtcggcaaggcaagtcctatgcgttcggtgatcacacggctggcagcgtccaaagcgctgaccgaacaagagcttggccttgtgctgatcgacagcagcccggcagccactacggtgaccttgccggcagccagtctcggtctgggcgtgcgtgacgttatcgttcgccgtgtcgacaacagtggcaatcgactggttgttcaggcttccggtacggaccgcattcgccttcatacacacctttcgtccaatggttacccctttctggtgctgatgggcaatggcgactggtggcatctgcgcagtgacgcagcgggtagctggtggcctgtcgggcgcttcgacaacacaccattgggccgaccggttttcgagaccaccactgtgctggggccgggcggttacggggcgcttaacggagcgttcctcgatcgggcgcaatggccctggctctgggattttgctcaggcgtccggcgtgctgaccaacgaagcggggcggtggggcagggaaggggcgtggaccagcggcgatggtgcgacgaactttcgtatcccggaagcgcgcggcgaatttctgcgcgtactcgatgaagcgagaggcgtagatgtcggtcgtgtcgcgggcagccttcaaaaccatgcgctgcagactcataaccattatctgcccaccagcacaggctcgttcgggcgtcccgctccctccattccggacaatctctggagtgtttcgtctgacgtcaacttttaccccaccaatggaacggtcgctacgacgtatccgaacccggcattcgactccgatacctacatcgggtcgatcggcaatttctcatctgaaacccgcccgcgaaacatcgcgtatcccggccgtatcaaactgatctgaggcacacatgttcaattatttgatagacgacagcggtgcgctgaccgggcctgtcgagtttccgctggtgccaggtatcggcgtacagctgcctggcaacgccgtgacgttgagtatcgaactctctgcggcaccgaatggatatgcctgggcctacgacaacggttctctgcagcaaaaactcgactttcgcggtgatgtttatcacaccgatacgggcattcgggaaacctggaccacgttgggtgacctgccggagggcttgaccacgcaaccatggccgggcggattccattcgtgggtcgataacgcctggcagctcgatgaagccgctcgactggcggatctcaaacggatcgctctgacccggcgcgacacgctgctgcgcgacgcggtcctgcgcatcgcccccctgcaatatgccgaagacatcggcgatgccagtcacgaagagcaactgcaactgctcgaatggaagctctactgcgtggaactgaatcgtatcgaaatgcagaccggtttcccggaacaaatcacctggccggcagcacccggcgcaaccgtaatcagctgacagaagcacagggaacagtgcaatggactatccaaaaagcatccccggcgtcggcctggtcgacggtggttttatcgatgaaaaccccattgccggcacgccaggatcgttgatccccgccgcctggggcaacagtgtcacgcaagaaattctcaacgccatcaaggcagccggactcaccccggacgagagcaaaaccaaccagctggccacagccatcggtgcgctggtcgacttcaccaaactgaagaacaccccgaccacgctggcgggctatggcatcaccgatgccgtggggcggttgctggcggttcggcagatcgagacggtcgggatcacggtttacaagccgaatccgagggcgaagcggattcgtgtgcgtctggtcggggcgggtggttcggggggcggatgtgcgcctgtaccccccacctatcaaagcttcggaggcggtggtggagcaggagcctatggcgaaagcctgtttgatgtgacggcggaaatgcaggctggtgttcctgtttcactgggtgccggcggtgccgcacgcaccgcgatgggtgtttcgggaggcggtgcgtccttcggcagttacatgagcgttgcgggtggcgcaggcgggcaaaccctgtcgatcgtgctgacgggaacttcgtccggttgcgtccagggtggtacgggtgggcaatcggtttctggcgggaatctcactgctgcgcgtggtcagccgggtggttatgccatgagcaacgccaactggggactgctgggaggcaccggtggtgcgagccagttcgacggaggtgctccattcacgggcgcgaacattaatgcgaattccggttctcgtggttcgggtggcggcggagcttgctccaatagcgcatccgtcgcgtatccgggtggagtgggcggcaacgccttctgtgaaatctgggagtacgagtaatggcccgttatgcacgtattgaaaacggtgtcgcggtcgaagtgatcgacaccggtgactacgcgatcgagcaactgtttgcgccggcgttcgtcgcggcgatggtgcaggtgcccgaaggtgctgatgttgaaatcggcgcgccgatgcctgagttgacgcccgctgtcgagcctctgcgcgaaccgccagttcctgaaatcgctcaggccgcaacggtcgagggcaacacgtcttcgacggctgagcgcgcctggcgccagtcggcgctggcggccacggaatggttggtcacacgccatcgcgacgagcaggaactgggacgcggcaccacgctcaaggcccagcattatctggaattgctcgagtaccgccaggcgctgcgcgactggcctgactcaatccattttccggcagtagttttgcgcccggcagcaccggagtggatggccgccgttcatggctgaggtcttgttttgatgttcttgaatagggagaagagtgatggattacccaaaaaacattcccagcgcagggttggtgaatggcaggtttgttgatgaaaaccctcttaccggaaccccgggttcgttgattccggcgagctggggaaatggcgttacgcaagagattcttgaagtcatcaaaggcgcagggtcggctgccgatgaaagtgataacactcagctcaaggcggcaatcgatacgctgatctcgaagaaacaaagcgacagtctggccagccaggaagaagctgaggcgggcgtcagcaacacgcggttgatgacgccgttacgagtgtttcaatccatcgcaaaaaaaatgcaacaggcgaccgagtcgctgatggggattgcaaaagttgcttctcaggcagaggtcaacgccggtgccagtgatacgtctatcgtgacccctaaaaaactcaggtttgggttcatggtgaggctgggggcatccggttatgtcgttttcccctcgtggatggggggggtgattatccagtggatcaccggaggcgcgagccaggcgggcaacaatggctacggggacctgaatctatggccgttggtctttcccaacgcactgtttcttgccgtcgcgacccatgaaggcacggcacccggaacgcagctgacctggaacatcaacgcgaccgtgagtcggcaggcaggcatcaatgttcgttgtcctgaatggccgtcaggctccattgctgctcgtgtcatcggaataggaaactgactatgtattacttttctccggctacttccggcttttatcactccgatctgcacggcgccaatatccccgctgatgcctttgaattgagcgaaggtgagtattgcgcgctggtctcgaacgctccaaaaggaaccgttcttagcctgactgccaacggacgcccggaacgggtgctactggctgaacaaactctcgatgctacagagcgggtctggcgagacaaggtattggatcgaactcaatggctggttcttcgcgatgcggaagaactggaagtcggcgagggaacaaccctgcgcggcgaagagttcaagcaactgctcgcctatcggcaggcgttgcgcgactggccaaatgatccggagtttccggatgcgcgttcgcgtccggtagagccggattggctggaaggcctgctgcgagcgaacaactgagcggattgcccgatggggcaaaaccggactaccaaggaaaatcattatggactaccccaaaagtgttccggggtcaggtttggtcgacggcagatttgtcgacgaagacgcgatcgccggcacccctggttcgttgatacctgcgagctggggcaacagcgttactcaagaaattctcggcgcgattaccgccgccggccttaagcctgacgagcagcagaccgatcaattggcgcaggcgatccgtcaattggcaaagcccgatccactgcaacaatttccggtgcaggtgtatcgccggaacgtcctgatcaatggcgggtttgatatctggcaacgcggtccaaccaaccccgggccaaatattggcggctatgtggctgatcgttttcgttgcgactggaatggcagtgcaggagtcgccatatctcagcagggttttgcacccggtcaaacggaagtcgccgacgagccgcagtttttcctgcggtggcaacaaacccaggcgggaaccggagccaccgtacacagaatctcccaagctattgagtcggtacggaccctggcaggcaaaaccgccaccgtaacattctgggcgcggtccgatgcggcacgacagctaagagtgtcggtcactcagaacttcggatccgcaggttcagactctgtggaaaaaacggtcgatgtctttcaattgggcacatcgtggaagaagtacagtgcgtcatttcgtctgcccggtattgccgggaaaatgctgggagccaacaacttcgtgaggcttgcgttcgacttgccattgaatgttttgcagaccgtggatctggcacaaatacaaatggaggaaggaccggtatccacacctttcgaatatcgcccagtggctgaagagttgatgctttgccagcgttacttcgagaagtcctttgccacttggttgccggtacgggcgaacaatggttctaacacctgcatttcaacgttcacgcaagtggcgcctgccaataacggtcagttcgcgatgacgacaggcatgttggtgcaaaagagggtgttacctaccgtcgtcatgtattgccctggcaataccagcaatcaggtatggaatcaggccgtggggccatgtaccggcagtattgtgcagggattgacggagcgtgccatttcgttttccaccgttaccccggtcggcagcttgcccggtcagaccttgcagatcgaatggactgccgacgccgaactttaggagaaaccatgagttatcaattgaccgccaacggcgttcttcgtctgagcgacctggcatatgttccacaggatcctgccaatagggattggctggaatatcaagcgtggctgttgtccggtggccaggtgttgccctcgaatgaagcaattgaggaatctgcaccgaacagcaccctgacaactctggcaaaaaaatggctggggggcgttggtcgccagccgtgattcaatcggcgcaatccagggaggatcaagcattatgcaaatcactgaaaacaacctcagcaacatcatgcccaacgcccgctcccaagcgggcgtttttgtttcaccgctcaacgacgccatggcgcgtcatcgcatcgatacgcccaagcgcgtcgctgcgtttctcgcccaggtcggccatgagtccgggcaactgcgctacgtgcgcgaactgggcaacaaccaatacctgagcaaatacgacaccggcacgctggccctgcgcctgggcaatacgccggaagccgatggcgacgggcaaaagtatcgcggtcgcgggctgatccagatcaccggccgcaccaactatcgccagtgcagcctcggactgttcggcgatgagcgtctgttatcgttgcccgaattgctcgagcaaccacagtgggcggcggagtccgccgcgtggttctgggagcagaacggtttgaacgaactggcggaccgcgatcagttcaacaccatcacccgtcgaatcaacggcgggttgaacggtttgcaggatcgcctggatctctgggctcgggcgagggcggtgctatgcccatctcctggcgtataaccggtgttgtattgctggtcctgggggctgccgcgctggcctggcaattccaggactggcgctacggccgccaattggccgagcaggcccgacagcatgccgaaaccctcaaccaactgactcaggctgctgcctcggcgcagcaggccgagcaggacaagcgtctggccctggagcaacggctcgcggccagtgaacaaacccactatcgagcactcagcgatgcccaacgtgatcaggatcgcctgcgcgatcgccttgccactgctgatctgcgcctgtcagtcctcatcgacgcaggcgacgctgcccaaggctgcggcgtgccagccgcctccggcaccggcggcgtggatcatgcaaccgtacgcgcccgacttgacccggcgcatgctcaacgaattgtcgccatcaccggcgaaggcgatcgcggactgattgccctgcaggcctgtcaggcctatatcagagcgctggcgcctgcacattttgaatga

SEQ ID NO: 6 - protein, 244 aa, Pseudomonas fluorescens Ps36
MQKRNVSSVLRALLDQYGISPTELHRRTGVPQSTLSRILSGKIVDPSDKHISKIAEYFAVSTDQLRGRADVAPVAGGGREELHSELKDISLWDDDTPVDDDEVSVPFLREVELAAGSGRFVIEESERSSLRFGKRSLRHNGVQFDQAKCVTVRGNSMLPVLRDGATVGVNAGKCGIGDIIDGDLYAINHNGQLRVKQLYRLPTGIRLRSFNRDEHPDEDYSFQDMQEEQIVILGHVFWWGMYAR

SEQ ID NO: 7 - protein, 140 aa, Pseudomonas fluorescens Ps36
MRRYGRVDQDRIVEFFETDGDITQMFHPSIIWAEVTDHPEVQLGWVATKTDGVWTFAAYVPPPPTEQELIAKAQLNKWQLLNVAANWLLLNSLQFKVDTGVATPDEQALLLAHKMYSIAVSDIDKQSGYPANIVWPVAPY

SEQ ID NO: 8 - protein, 139 aa, Pseudomonas fluorescens Ps36
MNRYILMTTAYSYNLVLDVVDTDGPMPEVPADEPYSSWQDYTGNTTAEPGMKMVWNGLPSFVPTTATEREAMNQGRIQTRLQEAQSWLMFNPVQYKSDLGTASPAEEAALLAYKQYFVAVAEVKNQTTFPKLNWPVAPF

SEQ ID NO: 9 - protein, 115 aa, Pseudomonas fluorescens Ps36
MTTEQQALADMPIWLVILLAVAGGVSGEMWRADKDGARGWPLLRRLALRSGACMICGVSAIMLLYAAGMSIWAAGAFGCLTAMAGADVAIGLYERWAAKRIGVCEVPPANTNKEQ

SEQ ID NO: 10 - protein, 283 aa, Pseudomonas fluorescens Ps36
MATLPRYPFTTDGSSILLPLHEMSAGQYLQSPDKRFKLIVQPDGNLAIYEGANTVWVAIAGQPYTSSGKQIDNSKIYFYLMYYAFLNDPTRGRMWGTANSTPLNSDIWAAYNRAYLSLQNDGNLVVVDSIPVWSSNSAIPISPSVESVYIPAGTTLEVDRRYVVGGTTLVFQSDGNLVVSNGPLGVLWASWTQNKGATRAVMQEDGNFVIYGQNNTPLWFTGTAGQPGAMAKVQANGSFSIVSEKPVWARFGFTPTILPKRVFQWDNGPWKPLIEIPLWRFKD

SEQ ID NO: 11 - protein, 173 aa, Pseudomonas fluorescens Ps36
MPVPIRQPSQLFTAMATALRNNADLNVQVGNHDDFTAPGDKAWVLIDIERNAPGERAANGRIAHALTLSLQVIPAISATAFAACDLIAALKNLITDNRWGLPGDQCDLPMNLDGLPSLAIRADQPNKAWTLTFNQTLYLGPTLIDDPLGTPKFARTWEVSDIDDPDQYTSLEA

SEQ ID NO: 12 - protein, 202 aa, Pseudomonas fluorescens Ps36
MFDALLRMQLGPIIERLAEMEAEIEDLHRRAESFCRIGICQEVDAASNTCKVSHGGLLTPAIKFFNPSAGAQSESRIPSVGEQCLLLNYGSGESGAQSVALFGLNSDRFPPVATVPTLTRRVHVDGSESGYDDATHTLHWQNGPAAFSGSREALELSIGPARLAMTAQAINLQLGATGLTIDASGVHFSGPLVDHQGRVISP

SEQ ID NO: 13 - protein, 110 aa, Pseudomonas fluorescens Ps36
MIGIDRDTGATVDDWLQFVQRATRALTTPLGTRQKRPLYGSLIPTLLGQNLGDDVLLLAQSHAAQAFYNPQNGIGDFQPGVIVATRQGAGLLLRFAGTWKNRQQTFEVVT

SEQ ID NO: 14 - protein, 331 aa, Pseudomonas fluorescens Ps36
MSMLIPGQNQLAEPSLIKVEAFEDLLAEFKTFVLEYVGTRSPDSAAKLKISLENESELLTMALEAFCVRLQTHERKYNARIKQMLAWWATGSNLDARLADMGLERQLLDPGDPAAFPPVPAIYESDDDARLRYYLAPHAPAAGSRMQYRREVFTLGERPSVKVESTDAGVVDVTYTFAPDGLAAQVKDGNGRRTAPGEVQVTVLSRDADGTPSAALLDGVRQHFARPDVCPETDKVTVKGAEIQRYKIRVVAKINSGPDSGLTKVAAEQHLQAYADSCHRLEGRVAPSWIDYTLHSAGAVQLEILEPLTPIVCSAFQAPYCTAVEVEVQTL

SEQ ID NO: 15 - protein, 211 aa, Pseudomonas fluorescens Ps36
MTDQTPRPTLLPANSSALERALDIGFGTLLDRIVPPFPELMNPSETPVAFLPYLAADRGVAEWSTDAPEAEKRLTVELAWPTARQAGTRKALENAAKGLQLRPEIRAWYEQTPPGAPYSFSVRAFTEQPYSEEIDARLDRRLADAKSERDVLSVSVGLSAFGNHVIGAATFCGELTTVYPVFLEGLETSGESFKATGLYTVETSTIYPQGA

SEQ ID NO: 16 - protein, 1104 aa, Pseudomonas fluorescens Ps36
MADYYTLLTNAGIAYETACKAAGVPIKLTQISVGDGGGAVYNPAATATALKREVWRGPLNALFQDEKNPSWLLAEVTIPPDVGGWYVREAGLWTDTGILYAIVKYPESFKPVLATSGSGKEFYIRSIFETSNASLVTLLIDDTVVKATRAWVMSYLAEELGKLDGKQSVRVAATASVVLNGAQQIDGVAVIAGDRVLLPNQTLAKDNGLWIVANGDWVRATDANVSAKVTPGLTVMVEEGTLNGDSLWHLTTNAPITLGTTALTFKMLAGRTGIAAGTYKSLSVDEYGRATAGSNPDTLAGFGIKDSYTKAEVEALIAKASALPVGSIVAFPVDTPPPGFLELDNSVKSSATYPDLSAYLGGKFNKGDEGVGNFRLPEARGEFLRGWDHGRGVDAGRELGTAQTEAFKAHNHRYFDSVAATMDPAGGWQSGTVNGTQAGVSPGAFISVTNTGDAGQMLNAHTTVNTGGTETRPRNIAVMWCIKAWNAPINQGNIDVAALVKEVSRLGSAVPVGAVMAFPTGIVPPGFLELDGSVQNIATYPDLAAYLGTTFNKGDEGVGNFRLPESRGEFLRGWDHGRGVDSGRNFGTYQTDDFKAHNHPPANNRPGFMTNEFPTVQAYHAATSGGPQSYSGEGQQIATTGNRGGTETRPRNLAVMWCIKAWNAPINQGSIDVAALAKEVSQLKSSVPVGAVLSFPTGVVPAGYLELDGSVQSIATYPDLAAYLGTTFNKGDEGAGNFRLPESRGEFLRGWDHGRGIDIGRSVGSYQSGTKTQGDDGTAPAVQGIGNSNLIDADPAPGFSGDIYYTSTNVVVQNFSNSFWKTVRPRNLAVMWCIKAWNAPVNQGSIDVAALAADARSARLNGAEVGAARNLRVSLPAAASVATLTADQLIVEQPGVGQYKLSNVNLSINLATIGAGGMDFGVAPANGSVGIYVIYNPELKVAKLLGVNATSTSVPEIYTGTNMPVGYSASALVSVWQTDANRLMNAGIQHQRSISIIQTMVLENGLSMSSTPISLASVVPKNAKSVGGYIHYIGSADFPGGGSLGLSPDVTEVGLKACGIGGIVGLGVLSPFSDLVMTTPQTIYYRLYASVSRANDVHISQYTF

SEQ ID NO: 17 - protein, 169 aa, Pseudomonas fluorescens Ps36
MLRAYSNSGTAFRCVAPDWPLSDGEVLFDHEPTVQELEDAFGFANGELVVKRQWEQIAEERFRREGSGIVVAGVAIDTSRDSQSLIAGMAVSAMLDPEYHCSYKAIEGFIDITSQQILQIAQAVRSHVQACFDREKTLYESAQAGTYSREMLTEGWPDSSPETPPKNLQ

SEQ ID NO: 18 - protein, 61 aa, Pseudomonas fluorescens Ps36
MATRQTYTVLVPFPTGGGHWSSVGQELDLLDVEASALHSAGRLELKTPTTKAVKAAAKKAD

SEQ ID NO: 19 - protein, 388 aa, Pseudomonas fluorescens Ps36
MAEVLNFEHNGITVNATESPEAMGGLGDNVIGLVGTAPKADPLIPRNAPFRINSFTTHALLDPTGAEEGTLYHAVYQILKVVKVPVYVVIVEAGATPADTVNAVIGGIEPATGRKLGLAALGSVPEDLTIIGAPGFTGTKAVASEFASFGKRIKARVVLDGKDASVADQVTYSQELGGADLGFDRCLVVHNMPAVYSKAAKKNVFLAPSSLAIAALAKVKQWESPGNQVTYAEDVSRVVEYNILDTSTEGDLLNRYGVSYYARTVLGGFSLLGNRSITGKFISYVGLEDAISRKLVKAGQKAMAKNLTKSFMDQEVKRINDWLQTLVADETIPGGSVYLHPELNSVEKYKNGTWYVVIDYGRYAPNEHMVYQLNARDEIIEQFLEDVL

SEQ ID NO: 20 - protein, 168 aa, Pseudomonas fluorescens Ps36
MFTNRNRQAIAATLQGLPLSATVEEFTPPKIEFDVEEMRGGRFIVEEMVKGGKALNAKLTLQGMGAEVMLALGVKLGDDILLNVREAGQDQDGNTWFTYHTVGGKLKSLEETAVKMGEKPKTNLELSCRTYNRLENGVPVIDIDVRTQKFVLNGVDILGDARRAVLMP

SEQ ID NO: 21 - protein, 193 aa, Pseudomonas fluorescens Ps36
MSWMPPKHDLLSPITGDDGSQIESIQLKPLFYAAQKEALERAGDDEDDQFFELALLATGLSVKELDQLKRPDYVSIAQYVHEMSTRPASYFLDQVEDAEKSDDPDQVQLLQPLAVTGRTVTSLSLEMPALRATKVMKKLKTAKERAEFITAHCTGLMIPDLALMSVPDWTQLQVRIDDFLNQPAAFFQSATSK

SEQ ID NO: 22 - protein, 757 aa, Pseudomonas fluorescens Ps36
MAQSKFALTYANESGNAAAGLKLPDGLGKPLQDLNLTMALASADIRLLTQEQIKLRELLANQQSLFKVSAASPAASAEPKSKLKAEIEQRPPPKLMQPAMANETALVELNQLLKLSNDQLQAHSQSTLELASEKQISASGATNADLLQVQLAGARSGIADGAKGDQRANALKWFSHDAAINASAFRMDVKAAGEMLAAWRSSLKLDQYQSQDLADATTYLGNSGLDAKAADIGSVVQRSGESAIAAGLTPEQVAALAAALLNSGADKEGASAALKGITSMLAKGGAVSTEQRTALTQLGLDPQSLSEGMKKDAPAVINSVLAALNKQPVQERAALTKTLFGENDTRVLELLKKPDDVKNAFSLVADKHKYATTELGAGEGAAAKSAEAFGNTSQGRWNALDASLTRLTTSFGTALAPLADGAAVVLTALVNGVSAAAETFPALTAGLALLAVAAMPFVGGALKSGVASVLDVVSTKLLRLASTRLPPDIADVIGGDDNDDDGRKRRKKGRGSRRRPPSAARSSGTASITRKSSRLSGVTARIAPMFDDALTRFRMVGDVVKSAMPSRLSGAGAKVMSLAEGLGARLMPSVVKALPVIKVGAPLAIAHAAYTGLKGWREGDDKAVKGAAGELAGTAIGATIGTFIAPGIGTFIGGTLGGIAGSILGQKLATPPEDKLAPPAQVAKDVSIAQTQMQASNPQYTYAPSVHVSGSELVSSEKVGTMLSQVLESHFNSQFVPGVATNALATRRDAALTDGVA

SEQ ID NO: 23 - protein, 127 aa, Pseudomonas fluorescens Ps36
MKQQMALGSFIFGLSRDFAYSTLSRKSEGGWTELQILNSKPRSHQTGQKPETLTISGTSMYAVAMERLDELRALQALRVPLPLIDGIGRNWGLWRINSIDENQSEVIDDGTAMVIKWVIGLSEFNNA

SEQ ID NO: 24 - protein, 70 aa, Pseudomonas fluorescens Ps36
MRKVRSVAGDSVNLLLYRETGRSDDSAEEALWTLNPTLAEHGPILSAGVWVTLPELDSKPAAIKPVLAWD

SEQ ID NO: 25 - protein, 342 aa, Pseudomonas fluorescens Ps36
MAQGFTPAIEIYGANKDLLNQRLISWEHIDAAGMESDQLTLVLDLEGLEGLPTLGGIIGLRVGYLETGLVEKGQFRVTRLTPTLFPLRLTLVATAAPFSGKDETGFKERRTASHGPTTLGGLFRKLVEPHGFSPRVDPELALIRIAHVDQSNETDMGFITRLAKKYDAVAKPFNDLYVLAKPAQLKNLSGQVIPNVRLSVTHNNRPGEHAFISATLEETARTQNEGCKVCCWDANAGKQVEVKTGSAPYKVVRQKQASVEEAKAIGEAEVRKMLREKYKLKVTCPGDPLLVAEGLLVLDDTWPDFMRGRWSIEKVTASGKPEESYRCLIEANGRDPEAKAKD

SEQ ID NO: 26 - protein, 194 aa, Pseudomonas fluorescens Ps36
MKISPILTQLRAQCPSLAGHIATGVDLALLQGNPNLPTPSAHVLPLADLASASTAQNSASQPIRDRFEIILALDATDATKALDLLHDLRAEVWRALVGFKPGSDYSAIVYDGGETVSINSSRAFYRLRFFAEFQLGRNLPSQPAESWHERELDGLSSFTGVTVRVDAIDPADPNLKHPGPDGRVEMTFSGDVTP

SEQ ID NO: 27 - protein, 59 aa, Pseudomonas fluorescens Ps36
MSNRITVVPATGRAVPDPEAGDLLPLEGREVLDSAWWRRRLADGDITLKTATAKQKGAK

SEQ ID NO: 28 - protein, 498 aa, Pseudomonas fluorescens Ps36
MAIGFSNIPADIRVPLFYAEMDNSAANSASSSMRRLIVAQVNDNIAPSEVGKLVLVSSVALAKSIGGQGSMLASMYETFRKADPIGEIWCLPLHNATGAIAKGVLTLTGTATQAGVLNLYVGGVRVQATVVNGATAAQAATALAQKINATADLPVSAVAAEGVVTLNAKWTGESGNDISLQFNRLGKSNGEETPAGLTTAVTAMTGGVGVPDQVAAVAALGDEPFEFIALPWSDLATLNTWQAVMDDSTGRWSWAKQLFGHVYSAKRGTVGTLVAAGQARNDQHMTIQALEPGVPQPVWVQAAALAARTSVFISADASRPTQSGSLPGVDPAPASERFTLTERQSLLNYGIATAYYEGGYVRIQRSITTYQKNAYGQADNSYLDSETMHQSAFIVRRLQSVITSKYGRHKLASDGTRFGAGQPIVTPATIRGELIAQYAKLELEGHVENAELFAEHLIVERDVQDPSRVNVLFPPDYINGLRVFALLNQFRLQYDDVA

SEQ ID NO: 29 - protein, 115 aa, Pseudomonas fluorescens Ps36
MGQLIAGTCYVKVDGAQLTINGGCEAPLMAVKRETVVPGFYKETDIAPSFKVTALHTADFPLKKLIEGTDITVTCEFSNGKVYVLAGAYLVEEPVSKGDDATIELKFEGIKGTWQ

SEQ ID NO: 30 - protein, 98 aa, Pseudomonas fluorescens Ps36
MSGAVKLQVAIEAHGEPLTELVLRRPTVQEVRAIKALPYKIDKSEEVSLDMDVAAKYIAVCAGIPPSSVNQLDLADLNALSWAVASFFMSAASEPSPT

SEQ ID NO: 31 - protein, 631 aa, Pseudomonas fluorescens Ps36
MAEETKAKASVLLTGIDELSPKLGALRVKVDDFKKNLEQTGLGKLDISGLFKGGSVITPFVDGIKSAAAFQGKLTEVSETAKTVDLPETPKAAAQNMNVFSASMERVSAAVDAALVPAVGALVVGLEPMLTQVGSLLADNPKLVEGLAAGAIAFSAMQTAVTGMTQVMDVMSMVLKTNPIMLIAMGIAVAAGLIVANWTPISAFFTGMWEGVKNAGASAMATLRSVLDWRPLETLAALWEPVTGFFSGIWDKVKAVTAPVIDFFKSVFSWSPAGLILENWGPLTGLFSAIWELLKALSVPVMSFLKGLFDWTPLGMIINNWGAITGFFASIWVALQPAAQAIKDFFGSLFDYSPLGMIINNWSAITGFFASIWAALQPAAQAIKDFFGTLFDYSPLGMLVNNWGSVVTFFEPVWAALQTSAQTIKSFFQSLFEWSPLEQIAQYWQPISEVFSALWGVVQALAAPVLEFLHNMFEWTPLGQIIKNWGPITEWFGELWQKLQTVIAPIKELFDGGFAGLIARVTGKVETLTQAQRQTNAEGKGELAPAFFGASPKPEGGSALQGGSLPQSSGALIQQSAANNRTQLEGGLTVRFENAPAGLRTDQPQTNQPGLALSSRIGYRSLSAGGSNELA

SEQ ID NO: 32 - protein, 411 aa, Pseudomonas fluorescens Ps36
MNWRDRLLPASFRGVGFWIDQAKTPVGRKGQLHEYPQRDLPFFEDLGQQAKTHDLTAFIIGADCLEQRDKLLQALEQGSGELVHPWLGRLQVKVGECDMTHTRQDGGMVTFTLKFYPDRPLPFPTATVSTQKVLLIKADGLLGSAVARFEQAMTLIKAARIGIANLRNSLTGVYDVIKEQLKPLIAQYKQITELVRAVKELPKEVAAEFKGLLGDIKELKAFAKEGYRGVIADVSQQIEAIRKADAPKITTGKDTTAAAQALANLVQDTLIVKAAQWVASMPVASTPVKLSSTPSLDQQSKQPVSRQEVPVTDDLQALQKELIEALQKAQDKADPAHYQAIADVKEALIAHLKAVASSGVRLVSKTFQETFPAVVVAYKQFGDATRVTEVIQRNGLSHPSFSPNEVKVSRE

SEQ ID NO: 33 - protein, 347 aa, Pseudomonas fluorescens Ps36
MNETDNRVTLTVGDMEYGGWKNVQITADLERQFRTFKLDITWQWPGQTVDQRIKAGDPCEVRIGKDLVLTGYVFKAPISYDGRQISLSIEGSSKTQDLVDCAARNNPGQWQDQSLLSIVQALAMEYALMVVNEIPETARLSKHTIVPGETAFQSIDRLLSLYRVFSTDDAEGRLVLAKPGSAGRASDALELGKNILSANAPMDFSQVFSEYRVIGQQKGNDKKSGAAVSEVESTATDLSFKRRRTTIINEGSQLTFELAQQRAQWESATRMGRALTTTYQVQGWRQSNGDLWRHNTLVRVKDPVLGFDEDMLISKVTYSLSAQGSVTTLQVAPPHTFDANPTPPKKT

SEQ ID NO: 34 - protein, 169 aa, Pseudomonas fluorescens Ps36
MSLLTRLLARGTVVLASSASKLQSLQMRLTAGEVNDDMEHFEPYGFTSHPLAGAEGVVTFLGGDRSHAIALVVADRRYRLQSLAAGEVAIYTDEGDKIHFRRGRIIDIETATLNIRASTAVNFDTPVINQTGKIVSKGDQLAGGISQIKHVHGGVQGGSGQTGVPAGGQ

SEQ ID NO: 35 - protein, 132 aa, Pseudomonas fluorescens Ps36
MLFSQNLHAALTRSVLISLFTWRRAADDDALDDEERYGWWGDTFPTVADDRIGSRLWLLRRVKLTRQTQMDAEFYAREALQWLIDDGHCSAIDIISERLDAQRLNLRTVLTLADGERLDINPDNSWQVIYAV

SEQ ID NO: 36 - protein, 348 aa, Pseudomonas fluorescens Ps36
MPFETPSLPVLIKRTQSDLAGDSLRQSDAQVLARTVGGAAYGLYGYLDWIAEQILPDTADESTLERIAALRLNQPRKPAQSATGSVSFTATAGAVLDVDTLLQSSDGRTYKVTTARTTVNGSNTTTIAALDAGSLGNADAGLALTPVQPITGVVGNSFVVLAPGLSGGVARESLESLRSRVIRSYRVIPHGGSASDYETWALEVPGVTRAWCRGGLLGPGTVTVFIMRDEDPQPVPNDEQLAEVQDYIEPLRPVTAEVHVQRPIQVPVVYRFKSVNPDTTAVRAAVEAQLRDLHNREADLGVPLLISHIREAISSAGGEYDHTLTAPAADVPAGQSELLTFGGCVWGA

SEQ ID NO: 37 - protein, 199 aa, Pseudomonas fluorescens Ps36
MGGIRTAAQYQAQLRALLPSGPAWDPERVPELDEVLQGVAVELARLDARAADLLNEMDPAGVSELVPDWEQVMNLPDPCLGATPLFDDRRLAVRRRLLAVGSQAVGYYLEIARSQGYPNATITELEAPRMGRSRFGAAHWGTWEAQFMWTLNTGGRLLLGRRFGASYWGERFGVNPGSALECLIHRAAPAHTKVHINYD

SEQ ID NO: 38 - protein, 385 aa, Pseudomonas fluorescens Ps36
MDYPKSVPSAGLVNGKFVDENPMTGTPGSLIPADWGNGVTQEILSVIKAGDLTPDEKKYDQLLQAIQTVTAKGWNQDLALPLSALPLPTVATTDARMPITPAAASTSGGRVSVPAGIYVSIGQEVVAGQLGRSRTFTTQTWSSADLLPSSGYFLRAQVVSGALTFYMQRGTIYDVTPDSLKGTVNGAAGGGFQSSVLDMCLAWVVTGAPGSVPVVRAIYNRARLTWAQTLNGTGAVFLPLDPHARAARLVVGNPTPSSTAVTTVAFPSTGWAGGNYSYLSPVSTGVSNNAGGWNPATAQPCVIFTNNIVNDVTVSTLTASFDHANVRSLWQSYQAEHNLAQASADSDELLLSMGIKSHPVTDYNAGIPINFSEAVNVQLSWELIR

SEQ ID NO: 39 - protein, 171 aa, Pseudomonas fluorescens Ps36
MIVIQELHQIDGELRPAQPSAAHDWDGEQWVVNPEKVALLEQQETESLCARVDVAADSARSVLAGDPLKALEYAQAAIDAQAFQDAGYPKKEVPLSVAAWVAKGRSAKQAAEQILDKAAQVSDSLLTLRTLRLKAKTQIRGYAGKSQMDQARAATDEVLLAIRDLTAIQSQ

SEQ ID NO: 40 - protein, 365 aa, Pseudomonas fluorescens Ps36
MDYPKSVPSVGLVDGRFVDENPVAGTPGSLIPAVWGNSVTQEIVNVISGAGMTAVEADNGQLFQAIQSIVGKASPMRSVITRLAASKALTEQELGLVLIDSSPAATTVTLPAASLGLGVRDVIVRRVDNSGNRLVVQASGTDRIRLHTHLSSNGYPFLVLMGNGDWWHLRSDAAGSWWPVGRFDNTPLGRPVFETTTVLGPGGYGALNGAFLDRAQWPWLWDFAQASGVLTNEAGRWGREGAWTSGDGATNFRIPEARGEFLRVLDEARGVDVGRVAGSLQNHALQTHNHYLPTSTGSFGRPAPSIPDNLWSVSSDVNFYPTNGTVATTYPNPAFDSDTYIGSIGNFSSETRPRNIAYPGRIKLI

SEQ ID NO: 41 - protein, 188 aa, Pseudomonas fluorescens Ps36
MFNYLIDDSGALTGPVEFPLVPGIGVQLPGNAVTLSIELSAAPNGYAWAYDNGSLQQKLDFRGDVYHTDTGIRETWTTLGDLPEGLTTQPWPGGFHSWVDNAWQLDEAARLADLKRIALTRRDTLLRDAVLRIAPLQYAEDIGDASHEEQLQLLEWKLYCVELNRIEMQTGFPEQITWPAAPGATVIS

SEQ ID NO: 42 - protein, 308 aa, Pseudomonas fluorescens Ps36
MDYPKSIPGVGLVDGGFIDENPIAGTPGSLIPAAWGNSVTQEILNAIKAAGLTPDESKTNQLATAIGALVDFTKLKNTPTTLAGYGITDAVGRLLAVRQIETVGITVYKPNPRAKRIRVRLVGAGGSGGGCAPVPPTYQSFGGGGGAGAYGESLFDVTAEMQAGVPVSLGAGGAARTAMGVSGGGASFGSYMSVAGGAGGQTLSIVLTGTSSGCVQGGTGGQSVSGGNLTAARGQPGGYAMSNANWGLLGGTGGASQFDGGAPFTGANINANSGSRGSGGGGACSNSASVAYPGGVGGNAFCEIWEYE

SEQ ID NO: 43 - protein, 155 aa, Pseudomonas fluorescens Ps36
MARYARIENGVAVEVIDTGDYAIEQLFAPAFVAAMVQVPEGADVEIGAPMPELTPAVEPLREPPVPEIAQAATVEGNTSSTAERAWRQSALAATEWLVTRHRDEQELGRGTTLKAQHYLELLEYRQALRDWPDSIHFPAVVLRPAAPEWMAAVHG

SEQ ID NO: 44 - protein, 246 aa, Pseudomonas fluorescens Ps36
MDYPKNIPSAGLVNGRFVDENPLTGTPGSLIPASWGNGVTQEILEVIKGAGSAADESDNTQLKAAIDTLISKKQSDSLASQEEAEAGVSNTRLMTPLRVFQSIAKKMQQATESLMGIAKVASQAEVNAGASDTSIVTPKKLRFGFMVRLGASGYVVFPSWMGGVIIQWITGGASQAGNNGYGDLNLWPLVFPNALFLAVATHEGTAPGTQLTWNINATVSRQAGINVRCPEWPSGSIAARVIGIGN

SEQ ID NO: 45 - protein, 143 aa, Pseudomonas fluorescens Ps36
MYYFSPATSGFYHSDLHGANIPADAFELSEGEYCALVSNAPKGTVLSLTANGRPERVLLAEQTLDATERVWRDKVLDRTQWLVLRDAEELEVGEGTTLRGEEFKQLLAYRQALRDWPNDPEFPDARSRPVEPDWLEGLLRANN

SEQ ID NO: 46 - protein, 399 aa, Pseudomonas fluorescens Ps36
MDYPKSVPGSGLVDGRFVDEDAIAGTPGSLIPASWGNSVTQEILGAITAAGLKPDEQQTDQLAQAIRQLAKPDPLQQFPVQVYRRNVLINGGFDIWQRGPTNPGPNIGGYVADRFRCDWNGSAGVAISQQGFAPGQTEVADEPQFFLRWQQTQAGTGATVHRISQAIESVRTLAGKTATVTFWARSDAARQLRVSVTQNFGSAGSDSVEKTVDVFQLGTSWKKYSASFRLPGIAGKMLGANNFVRLAFDLPLNVLQTVDLAQIQMEEGPVSTPFEYRPVAEELMLCQRYFEKSFATWLPVRANNGSNTCISTFTQVAPANNGQFAMTTGMLVQKRVLPTVVMYCPGNTSNQVWNQAVGPCTGSIVQGLTERAISFSTVTPVGSLPGQTLQIEWTADAEL

SEQ ID NO: 47 - protein, 72 aa, Pseudomonas fluorescens Ps36
MSYQLTANGVLRLSDLAYVPQDPANRDWLEYQAWLLSGGQVLPSNEAIEESAPNSTLTTLAKKWLGGVGRQP

SEQ ID NO: 48 - protein, 188 aa, Pseudomonas fluorescens Ps36
MQITENNLSNIMPNARSQAGVFVSPLNDAMARHRIDTPKRVAAFLAQVGHESGQLRYVRELGNNQYLSKYDTGTLALRLGNTPEADGDGQKYRGRGLIQITGRTNYRQCSLGLFGDERLLSLPELLEQPQWAAESAAWFWEQNGLNELADRDQFNTITRRINGGLNGLQDRLDLWARARAVLCPSPGV

SEQ ID NO: 49 - protein, 172 aa, Pseudomonas fluorescens Ps36
MPISWRITGVVLLVLGAAALAWQFQDWRYGRQLAEQARQHAETLNQLTQAAASAQQAEQDKRLALEQRLAASEQTHYRALSDAQRDQDRLRDRLATADLRLSVLIDAGDAAQGCGVPAASGTGGVDHATVRARLDPAHAQRIVAITGEGDRGLIALQACQAYIRALAPAHFE

SEQ ID NO: 50 - DNA, 20 bp, Synthetic construct
  source 1..20: mol_type = other DNA
agagtttgatcctggctcag

SEQ ID NO: 51 - DNA, 19 bp, Synthetic construct
  source 1..19: mol_type = other DNA
ggttaccttgttacgactt

SEQ ID NO: 52 - DNA, 1532 bp, Pseudomonas fluorescens Ps36
  source 1..1532: mol_type = genomic DNA
tgaagagtttgatcatggctcagattgaacgctggcggcaggcctaacacatgcaagtcgagcggatgaagggagcttgctcctggattcagcggcggacgggtgagtaatgcctaggaatctgcctggtagtgggggacaacgtttcgaaaggaacgctaataccgcatacgtcctacgggagaaagcaggggaccttcgggccttgcgctatcagatgagcctaggtcggattagctagttggtgaggtaatggctcaccaaggcgacgatccgtaactggtctgagaggatgatcagtcacactggaactgagacacggtccagactcctacgggaggcagcagtggggaatattggacaatgggcgaaagcctgatccagccatgccgcgtgtgtgaagaaggtcttcggattgtaaagcactttaagttgggaggaagggttgtagattaatactctgcaattttgacgttaccgacagaataagcaccggctaactctgtgccagcagccgcggtaatacagagggtgcaagcgttaatcggaattactgggcgtaaagcgcgcgtaggtggttcgttaagttggatgtgaaatccccgggctcaacctgggaactgcatccaaaactggcgagctagagtatggtagagggtggtggaatttcctgtgtagcggtgaaatgcgtagatataggaaggaacaccagtggcgaaggcgaccacctggactgatactgacactgaggtgcgaaagcgtggggagcaaacaggattagataccctggtagtccacgccgtaaacgatgtcaactagccgttgggagccttgagctcttagtggcgcagctaacgcattaagttgaccgcctggggagtacggccgcaaggttaaaactcaaatgaattgacgggggcccgcacaagcggtggagcatgtggtttaattcgaagcaacgcgaagaaccttaccaggccttgacatccaatgaactttccagagatggattggtgccttcgggaacattgagacaggtgctgcatggctgtcgtcagctcgtgtcgtgagatgttgggttaagtcccgtaacgagcgcaacccttgtccttagttaccagcacgttatggtgggcactctaaggagactgccggtgacaaaccggaggaaggtggggatgacgtcaagtcatcatggcccttacggcctgggctacacacgtgctacaatggtcggtacaaagggttgccaagccgcgaggtggagctaatcccataaaaccgatcgtagtccggatcgcagtctgcaactcgactgcgtgaagtcggaatcgctagtaatcgcgaatcagaatgtcgcggtgaatacgttcccgggccttgtacacaccgcccgtcacaccatgggagtgggttgcaccagaagtagctagtctaaccttcgggaggacggttaccacggtgtgattcatgactggggtgaagtcgtaacaaggtagccgtaggggaacctgcggctggatcacctcctt

SEQ ID NO: 53 - DNA, 1399 bp, Pseudomonas koreensis Ps4
  source 1..1399: mol_type = genomic DNA
aagtcgagcggatgaaaggagcttgctcctggattcagcggcggacgggtgagtaatgcctaggaatctgcctggtagtgggggacaacgtttcgaaaggaacgctaataccgcatacgtcctacgggagaaagcaggggaccttcgggccttgcgctatcagatgagcctaggtcggattagctagttggtgaggtaatggctcaccaaggcgacgatccgtaactggtctgagaggatgatcagtcacactggaactgagacacggtccagactcctacgggaggcagcagtggggaatattggacaatgggcgaaagcctgatccagccatgccgcgtgtgtgaagaaggtcttcggattgtaaagcactttaagttgggaggaagggttgtagattaatactctgcaattttgacgttaccgacagaataagcaccggctaactctgtgccagcagccgcggtaatacagagggtgcaagcgttaatcggaattactgggcgtaaagcgcgcgtaggtggtttgttaagttggatgtgaaatccccgggctcaacctgggaactgcatccaaaactggcaagctagagtatggtagagggtggtggaatttcctgtgtagcggtgaaatgcgtagatataggaaggaacaccagtggcgaaggcgaccacctggactgatactgacactgaggtgcgaaagcgtggggagcaaacaggattagataccctggtagtccacgccgtaaacgatgtcaactagccgttgggagccttgagctcttagtggcgcagctaacgcattaagttgaccgcctggggagtacggccgcaaggttaaaactcaaatgaattgacgggggcccgcacaagcggtggagcatgtggtttaattcgaagcaacgcgaagaaccttaccaggccttgacatccaatgaactttccagagatggattggtgccttcgggaacattgagacaggtgctgcatggctgtcgtcagctcgtgtcgtgagatgttgggttaagtcccgtaacgagcgcaacccttgtccttagttaccagcacgtaatggtgggcactctaaggagactgccggtgacaaaccggaggaaggtggggatgacgtcaagtcatcatggcccttacggcctgggctacacacgtgctacaatggtcggtacagagggttgccaagccgcgaggtggagctaatcccacaaaaccgatcgtagtccggatcgcagtctgcaactcgactgcgtgaagtcggaatcgctagtaatcgcgaatcagaatgtcgcggtgaatacgttcccgggccttgtacacaccgcccgtcacaccatgggagtgggttgcaccagaagtagctagtctaaccttcgggaggacgg

SEQ ID NO: 54 - DNA, 1401 bp, Pseudomonas koreensis Ps7
  source 1..1401: mol_type = genomic DNA
tgcaagtcgagcggatgaaaggagcttgctcctggattcagcggcggacgggtgagtaatgcctaggaatctgcctggtagtgggggacaacgtttcgaaaggaacgctaataccgcatacgtcctacgggagaaagcaggggaccttcgggccttgcgctatcagatgagcctaggtcggattagctagttggtgaggtaatggctcaccaaggcgacgatccgtaactggtctgagaggatgatcagtcacactggaactgagacacggtccagactcctacgggaggcagcagtggggaatattggacaatgggcgaaagcctgatccagccatgccgcgtgtgtgaagaaggtcttcggattgtaaagcactttaagttgggaggaagggttgtagattaatactctgcaattttgacgttaccgacagaataagcaccggctaactctgtgccagcagccgcggtaatacagagggtgcaagcgttaatcggaattactgggcgtaaagcgcgcgtaggtggtttgttaagttggatgtgaaatccccgggctcaacctgggaactgcatccaaaactggcaagctagagtatggtagagggtggtggaatttcctgtgtagcggtgaaatgcgtagatataggaaggaacaccagtggcgaaggcgaccacctggactgatactgacactgaggtgcgaaagcgtggggagcaaacaggattagataccctggtagtccacgccgtaaacgatgtcaactagccgttgggagccttgagctcttagtggcgcagctaacgcattaagttgaccgcctggggagtacggccgcaaggttaaaactcaaatgaattgacgggggcccgcacaagcggtggagcatgtggtttaattcgaagcaacgcgaagaaccttaccaggccttgacatccaatgaactttccagagatggattggtgccttcgggaacattgagacaggtgctgcatggctgtcgtcagctcgtgtcgtgagatgttgggttaagtcccgtaacgagcgcaacccttgtccttagttaccagcacgtaatggtgggcactctaaggagactgccggtgacaaaccggaggaaggtggggatgacgtcaagtcatcatggcccttacggcctgggctacacacgtgctacaatggtcggtacagagggttgccaagccgcgaggtggagctaatcccacaaaaccgatcgtagtccggatcgcagtctgcaactcgactgcgtgaagtcggaatcgctagtaatcgcgaatcagaatgtcgcggtgaatacgttcccgggccttgtacacaccgcccgtcacaccatgggagtgggttgcaccagaagtagctagtctaaccttcgggaggacg

SEQ ID NO: 55 - DNA, 1379 bp, Pseudomonas chlororaphis Ps6
  source 1..1379: mol_type = genomic DNA
caagtcgagcggtagagaggtgcttgcacctcttgagagcggcggacgggtgagtaatgcctaggaatctgcctggtagtgggggataacgttcggaaacggacgctaataccgcatacgtcctacgggagaaagcaggggaccttcgggccttgcgctatcagatgagcctaggtcggattagctagttggtgaggtaatggctcaccaaggcgacgatccgtaactggtctgagaggatgatcagtcacactggaactgagacacggtccagactcctagcgggaggcagccagtggggaatattggacaatgggcgaaaaccctgatcccagccatgccgcgggtgtggaaagaaggtcttcggattgtaaaaccactttaagttgggaggaagggtacttaccttaatacgtgagtattttgacgttaccgacagaataagcaccggctaactctgtgccagcagccgcggtaatacagagggtgcaagcgttaatcggaattactgggcgtaaagcgcgcgtaggtggttcgttaagttgaatgtgaaatccccgggctcaacctgggaactgcatccaaaactggcgagctagagtatggtagagggtgggtggaatttcctgtgtagcggtgaaatgcgtagatataaggaaggaacaccagtggcgaaggcgaccacctggactgatactgacactgaggtgcgaaagcgtggggagcaaacaggattagataccctggtagtccacgccgtaaacgatgtcaactagccgttgggagccttgagctcttagtggcgcagctaacgcattaagttgaccgcctggggagtacggccgcaaggttaaaactcaaatgaattgacgggggcccgcacaagcggtggagcatgtggtttaattcgaagcaacgcgaagaaccttaccaggccttgacatccaatgaactttccagagatggattggtgccttcgggaacattgagacaggtgctgcatggctgtcgtcagctcgtgtcgtgagatgttggggttaagtcccgtaacgagcgcaacccttgtccttagttaccagcacgtaaaggtgggcactctaaggagactgccggtgacaaaccggagaaagggggggggaagaagtcaaatcatcaaagggcccttacggccggggcaacacacgggctacaaagggtcggaaaaaaggtgtcgccaagccgccgaggtggagctaatcccacaaaaccaatcgtagtccggagcgcactctgcaactcgaccgcgtgaagtcggaaaccctagtaatcccgaatcagaatgtcgcggtgaatacgttcccgggccttgtacacaccgcccgtcacaccatgggagtggg